European Patent Application EP 4 481 027 A1, published December 25, 2024. Title: CLEANING COMPOSITIONS CONTAINING ENZYMES. Applicant: Procter & Gamble. The sequence listing filed with the application follows.

SEQUENCE LISTING (190 sequences)

SEQ ID NO: 1 - protein, 894 aa, Alkalitalea saponilacus
MKKCYIVLLKLFIAAFIMSATAQEYQLVWEENFEGAELNTSVWNYETEVGVWNWGANQELQHYRAENVEVGPDGEGNNALIITAKRESFGDYQFTSGRINTSGKVAALYGRIEARIKLPVLADGLWPAFWMLGTQNTWPASGEIDIMEAGHREGIDAGTQDRTFNGALHWEHAGNYAGYGPQWTAPEGASLYEYNVFVMEWTPQRIEMYFNDHPTPYFAMDITGEDAEEFRDWPHYFILNLAVGGSFPGITNPDDITAPLPAQMFVDYIRVYQREGEGVLVVSEPQTPQADYFGIFTENPSISERFVFDDFSNTLQVWDNSLQPLENAPSYDGAEVLSFYGYPARTWFGFGINAAAGMDFSHFSNGSLHLALRTSSDNDFWIGMGGAAEGRINFIEGSDPYGFQRDGQWYELSIPVSELVAAGLDLSDVRNIFMLGGDGAISNILVDDIYLSVDGQPLMNSELNPNRNDDLQLFENKIVADYYGIFTENPNVEEILLINDVDAHIYIWEGTLNNIQSSPYDGEEYLAFTSVGAGWWGFGIHDDKAADLSHFENGYLAFSVKASSQESFRVTITGASGTSGSFDFVTGSDPEGFERDGEWHRVRIPISSFASVDLSAVPIPFSVTQGPGSTSISDIAFDDIIYTTGIDPENPNLYDGSGEIGDPNGGDQGNWEYWFGDGGQGSVTFPSEHLATVNITNAGWQPWSVQLFKDNLDTPDGEYVLTFRARADAPRTLNVNFGKGLDAAPWFIEFMSPKEFNITTEWDTYSITINKENVEVVGKLVFEMGSTGGDNLITSVYIDDVSLELKNATNLPVASELRTEVYPNPASDNFIIYSEVNIADITVYSLAGVRVFETGNINSSSLSVNTYGWNDGVYVLVITDYNGERVSKRIVIKK

SEQ ID NO: 2 - protein, 487 aa, Alkalitalea saponilacus
MKIVTLIIVIMFSMSVFSQEEPQWELVWSDEFDTEVSQDWIFEIGNGCPNLCGWGNNELQSYKRENATVEDGLLVITAKKENYDNREYTSARMITRGNAFFRYGRVEARIKLPAFQGSWPAFWMLGENITSVGWPQCGEIDIMEQVNTDMDTHGTLHWNAGNGHHYQGSATGFEVDVTDFNVYAIEWDRNSIRWFVNDQEFYSINITNGINNTHAFHKPHFIILNMAIGGNWPGFEVDDSALPAKMYVDYVRVYQIPGYDEQEDPEVPMESFIIEAEDHSYENNTSVFNFQDTDGQYIRFNSSGSWAAYPPSNITQAGKYLMELRMAAEQEGGQIRLEANSGNILFDILDVPSTGGIGEWTIISSEIDLNAATYYFGFNSASGSYYLDWIKLTPLEASMINSNDFYTAKLIISPNPVRDGAFELQLAERAFNSAVVSVVGIDGQIVFQKKISALETTIQLPENISKGLYIVNVIGDTVNVSGKVLVR

SEQ ID NO: 3 - protein, 270 aa, Alkalitalea saponilacus
MQLRFKVVLLFCLVLLKPGCTTTRSSSDWQLVWSDEFNYHGLPDPLKWNYDTIGNTYGWGNKELQYYTYAEPKNVWVEGGFLHIKVQKERIHSFDYTSARLTTRHKGDWKYGRVEVRAKLPGGRGIWPAIWMLPTDSEYGRWPNSGEIDIVEHVGFIPDSVFVTVHTETFNHMINTQKGTSVFLPQSEYEFHIYAVEWCSEKIDFIINDELVFTFNNSGQGSAEWPFDQKFHLLLNVAVGGNWGGQQGVDDSIFPAAMLIDYVRVYRFRN

SEQ ID NO: 4 - protein, 736 aa, Alkalitalea saponilacus
MKHTINILAACFLLLIFAVSCVDDSIDFFEVEKPESIAELEYLNDYDFLKSYVDRAASPNFKLGAGVTVSEYLRLGHVYRVMNSNFDMLTAGNAMKYSSVVGDNGSMNFGSVIQFVEAARSAGIEIYGHTLVWHSQQNRNYLNRLIADREIEVDPDAKDEVVDGFKDYRVEGFTGWVGGPVQPVVEDGRLVVTSTEAQPNFWDVQYHVANGISIKEDTRHKVTIRIKGTSEASITVALGTWGAQQNTTIPITQEWEEVSVELNSTVTANDAFVMLQSGHYVGTYEIEWVRVTHEVAAAVTYYVNQLENSEMLVGGSMDNFIVRESGQADVPGAILEGEGPDGMNAIKINSVDNPANPWDTQFFIYTPNKAWEAGENYRISFWYKASAEANSESQCHGAPGSYMHWQMLPQNPQFTTEWQYYEATSTIPGQGDGMRSIAFNLNVNPTAITYYFANIVWESEESGNTIPLSPEEKADTLTYALRNWISGMMQATDGYVKEWDVVNEPLAGQGNVGEGFYDLKSAVRGTVSEEAAENSFYWQDYLGDDYVRVAVKLAREYGPDGLKLFVNDYNLESFWDDNHKLKSLIYWIDRWESDGVTVIDGIGTQMHVSYHMDPAQQAVRDAHIIQMFELLAETGKFIKITELDMGLIDEDGNTVRTADVTSEQHRAMSDHYKFIIQKYFEIIPANLQYGITHWSPTDSPQGSSWRGGEPIGLWTESTFRRKHTYGGFADGLAGKE

SEQ ID NO: 5 - protein, 400 aa, Alkalitalea saponilacus
MNAFMPYTDKNPTKIMKKVFFIAAALVFMFAGCSEDIIDADLMNDEMSDVTLKSYDSGTHDGYFWQLWTDDHSGWIDYRNGEGGNYSVSWDYNGNFTCGKGWSSGSKTRIIGYNIGVHNHSGGGVFGYYGWSRSPMIEYYVNESWGTQRPTYGRFLGTVNSDGSTYDIYTDTRVNAPSIEGTQTFTQIYSTRRSKVPVGQNRTITFANHVNAWANLGYHLNDMSPYAILLTEAYGGNSQGSVNATVWSAGEGTGDGGNTGGGGATYYRIQNRATGLFLDGVGRTSDGADLGQYANTNHQNAQWTREASGGFERFRNRGTGLYIDGMGRNENGANVGQWANTNHNNAQWSLESAGSGYYRLRNRGTGLYLDGMGRTSNGSDVGQWANTNHHNSHWRFVPVQ

SEQ ID NO: 6 - protein, 1060 aa, Alkalitalea saponilacus
MKRLFILISICIIALNSEAQDRPPHPELENPAIQGINKELPRASFNSYASRELALKNNREASDRFTSLNGTWKFNFVTGVSNRIKNFADVNLDISGWDDIPVPSNMEMHGYGYPIYTNVSYEFYPNWNFKPPYVNDLEKNNIGYYRRDFEVPQSWEDMQVFVYFGSIKSVGFVWVNGQRVGMSKDSKTPQEFDITPYVKPGKNSIAVEVFRWSDASYLECQDFWRLSGIPREVFVYAQPKVRLRDFYAKATLDESYVNGVFDLDVELKNHTGNSTLKSFSYEIIDNKGQSVASDSKSIEIVDSVGHLNFKATIPDVDSWTAETPNLYTLLLTSKDQSGNITEAASIRIGFRTSEIKNGQFLVNGEPVLIKGVNMHEFCPINGQVVDEETVMLDLRRMKELNVNAIRLSHYPQPSFFYDLADKYGFYVVDEANIESHGMGYDRAKGRSLGNNLDWTEAHIFRTRNMFERSKNHPSVVIWSLGNEAGNGYNFYKTYLFIRSRDEMRPIQYEQAGLEWNTDIVAPMYARPHNIEHYAQNHTDRPLILCEYAHAMGNSIGNLKDYWEIIEKYPQLQGGFIWDWVDQGLANENEKGEFWAYGGDYGPEGTPSDGNFVINGVLFPDRSIKPHSLEVKHVYQNIGFEPENIEEGQITITNKFFFTNLIDYAFSYEITANGKVVRTGKLSVLDIPPGQSKTVNIDLRRIKAKPGVEYFIILSAKTKKAENLLPAGWEIASQQIKLPVEAPRAQFDITKAGKVSYSEGASINITGRDFSLAIDSETGIITSYKSKGKELFLNGFGPRPAFWRAPIDNDYLWRMQQRCRLWKEASEQLPVAASVRANQLGNAVQVEVVYNLDSLQSIWTTKYTIMGNGMIKIDNELITFGDDVPIIPRMGMKMQLPADLTQVEYFGRGPWENYSDRNSSTFIGRYKTTVADMYVPYVRPQENGHRTDVRWLALSRKDGTGLLVVADSIIEFNALNNPIEDFDAGMNKDSNLRHINDIKPQDLVELHIDYRMIGVSGDEPWGSPPHEPYLLRPSAEGHKYSFTLVPVSSVRDIESKAILRY

SEQ ID NO: 7 - protein, 458 aa, Alkalitalea saponilacus
MKAMKSRTLRVTLFLVISFMMIQNSFAQRPIIQTKYTADPAPMVYNDTVFLYTGHDADDAMGFKMFNWLLYTSTDMVNWTDHGVVASLDNFDWVPYDNGAWAPHCIERNGKFYFYCPIPNGIGIGVLVADSPYGPFVDPLGKPLIQNSHHDIDPAVFIDDDGQAYLYWGNPKVYYVKLNEDMISYSGDIMVEETTPANYQEGPWVWKRNEHYYMAYASTCCPEGIGYAMSSSPTGPWGYKGMIMDATELSRGNHPGIIEFKGKWYCFGHSYDLLKLTTTKFYERRSVMLDEMIYNADGTIQNRPYWTVEGPEQVGTLNPFKRVEAETMAWSEGVKTRSETEWEGDFDWARGERIADRKFVTSINHGDYIMVKGADFSTGAKTVEVSVASLYGGKIEIRVDKLDGPIIATVDVNTSREGGIWRTFSAPVNEHAKGVRDVYFVFRGEKDLFDFDWWKFNQ

SEQ ID NO: 8 - protein, 563 aa, Alkalitalea saponilacus
MRKNFILSFFVLAFAVLHSCTERSNDIAVFEHFRYKGNDALFDKEFDPQNQYLNPVLAGFYPDPSICKKGDTYYVVHSSFSLYPGVPIFKSNDLVNWEQIGHVLDRPSQLELEGLQISNGIFAPAIEYNPYNETFYMITTSTWGIGNFYVKTKDPEQGWSDPIVFPQVRGIDPSVFFDDDGKGYILECAEPMGGADYRGQRAIHMHLLDVENDVIIGEPKEIVRGGARPEDRPIWIEAPHIIKKFGYYYLICAEGGTGLNHSQVVFRSKDVWGPYIPYENNPILTQRDLPEDREDKITTAGHADFVQDENGRWWAVFLGVRPYEFDMTNVGRDTYLLPVEWPEGGWPTILPQGEQIPIVNNKPGLNPDPNIPPTTGNFEFIDNFDSEDLGFTWMHIRTPREKYYNVGSGKLELRPRDITTEEIGNPSAILRRQQHTTFEAETKLEFYPETEADFAGFTLFQNEEYQFLFGKTIVDGKTSLVVNRLEKDKETLATVELTGRDRNRPVYLKVTGDAADYSFLYSMDGKNWVTMVENADGRNLSSRVAGGFIGALIGLYTTNNFEL

SEQ ID NO: 9 - protein, 760 aa, Alkalitalea saponilacus
MLIGISIFPISVQAQNYTSWYNNAQERIEELRMDSYGIQIFDRNGEPYTGEVAIRMQKHEFPFGIAFDFSQGAQSMGNVFSTNNVVQAEKDAEIYRTERWGGYIAYAIPVEAGKDYEVTLKFAEIFHGGNNARIFNVRVDGELFLENFDTHAVAGGRDIAVDRSLVVTSSGNQILIEFEAVVDNVAIKGIVVEEVDGDFTLRINCGGSALTTADGNEYVAEAGFFDPDANTVASNDDWRKATMYKYFNAGVTENSFKWSGVQSQPGPPNYTVFENAVRWAQKVGWELRGHALIWGGNDNHSTPNWVRSLPTPDDIYEACKERVLRDVERYRGIIKEYDVVNEPLTGHADWLRNEVGDRIIWDSFKWARSVDPDAELYINDYNVEYNWGQAEEYRDLIFEMLNQGAPVTGVGMQAHFWDCCRPGINELVRNINIVAEPGLPIKLTEYDFGGNLTQAEQAADYIMVLTIAFSHPSIVGLYHWSLRDGWAWRENSGFFDRDGRPKLAADTLLYYTKTKWATNFDAVMPANEPLTFNAFHGNYTVEAEFDGVVKVFEVPLLKANADAVFVLNEEDAVVKGPQFLETELVGRNSVRLLFDKPIDGNSLRGSNYRFFSSGNIGVEAANVDPDNGNAVILSLSSNVSSGQYISVSYFPGSLRALDGSVANAFGPEEIANKASSVGTTNIEQSRVRIYPNPATNNLNIAYESSPFRISIFNSMGVLVYSGTSANESYSLDVGGFARGMYVIQLTDQNNQIRVEKFLLK

SEQ ID NO: 10 - protein, 871 aa, Alkalitalea saponilacus
MKAIFLLSVALFFLSCQNQFVKSYLKESNRVTFHTDEGVLLVYPLTDNTVRVQFTLENSKILPEFVIQNDLEVPPFEVFEKGNIVSISLDRMVVEVNKRTGQISYVDKEGEVFLKEMPGTRLLKPDSIMGESCFFVEQKFESPSDEAIFGLGQFQDGNFNLKGLTRRLTQVNSQIVIPFVYSNKGYGLLWHQYGLTDFNPTDNFVQLEKQDDANLDQGSIAEVTTTAGTQKVAQDQSLYTGSFTVPRSGEYSIFLDLGDMGNRHYVVINGIPVMDQTNMWLPPTAGVLVNLEAGEHDVQLICKSDNEPTLSWKLKEDVTTYRSPHAQMIDYIVFYGPTADEVISSYRNLTGVAPMLPKWAYGFWQCRERYSSSNQLIENVKEFRKRNLPMDVIVQDWQYWGNKGWGVPQFDERYYPNPTGFIGEIHDLNAHFCISIWSNPDINSELGREYQRNNHFIPNTNWLDYFNPKTRKAYWNTLYENMFVHGLDSWWMDAVEPENDALTGEMTHIGPGDFYRLIYPLLVSQSVYEGQREVTSDKRVCILTRSAFAGQQRYGVINWSGDVGGTWDEYRRQIVAGLNFTITGLPYWTTDIGGFFRPGHSQYTDENYRELLTRWFQWGAFKPIFRNHGYMSETEPWKYGETVEENMRKMLNLRYRLLPYIYSEAWQVTSSGSTMMRALVMDFREDETALKQPYQYMFGNGIMVAPIIEPGVDEWDVYLPKSEGWYDFWTGERFNGNQTIKTDAPLDVIPLFVQAGSIIPMGPIMQFSTEKPADELEIRIYEGADGEFVLYEDENNNYNYEDGVFETITFNWDDSSRTLTISNRNGAFPGMLSERKFNIVIVSSNFGFGIEPSGYYNERVVYNGKQVSINM

SEQ ID NO: 11 - protein, 830 aa, Alkalitalea saponilacus
MKHPFVFTTKKNLSAIDMRTVRPRNEGRNFFHFLMTRLMLIYLFLFFISSSAVSQSYQETETGVVVHCNSMQVEIQFFSNSIVRVIKWPEGTNFKKESLSVVKSPESISLDISSENDLISLQSDDLTVNLNTNNGQVSFYKNNGKALLKEKNDGAVFVEIDDAGVKSYSVSQTFGLETDEPIYGLGFQQQGRMIQRNLEMNMIQNNTESFVPFFQSVKGYGLFWDNYSPTIFSDSTEATSFNSEVGDCIDYYFMYGGNADGVVAEMRELTGQVPMFPLWTYGYWQSKERYKSQEETVGIVRKYRDLGVPLDGIIQDWQYWGSNYLWNAMEFLDVEFPDPQRFVNEVHELNAHMIITIWSSFGPKTKQYRELDAGGMLMNISTWPESGSQLWPPRLDYPSGVRVYDAYHPEARDIYWKYLNEGLFSLGIDGWWMDSTEPDHFNWQPEDFDFNTYLGSFRRVRNAYPLMTVGGVYKNQRAVTSDKRVFILTRSAFAGQQRYGANTWTGDVVASWNALRNQISAGLNFSLSGIPHWNSDIGGFFLWEYPARLDDPDYRELYARWIQFGAFCPMMRSHGAEAPREIFQFGSKGEPVYDAIEKFINLRYLLLPYIYSTSWDVTANQSSFMRALVMDFANDPKVLDIDNQYMFGKSILVCPVTEPMYTTNGREDFSTVKSSEVYLPKGTDWIDFWTGEKHSGGQTIKKQSPIDIMPLYIKAGSILPVGPKVQYATEKKWDNLEIRIYPGANGKFTLYEDEKDNYNYEEGYYSTITFYWDDANSTLTIDDRKGSFPGMLNERHFNVVKVEKGKNTGMVPMVIDRKVFYNGGKIEVKL

SEQ ID NO: 12 - protein, 865 aa, Alkalitalea saponilacus
MKNLLSITICLLCSLAISAQQYPFQDPSLSSEERARDLISRLTVEEKAALLCDQSDPIPRLGIKRFNWWSEALHGYASNDSVTVFPQPIGMAASFNDELVFQIFDATSDEARAKYHQAMRRGEENRRFLSLSVWTPNVNIFRDPRWGRGQETYGEDPFLMSNMGVQVVKGLQGPEDARYRKLLACAKHYAVHSGPEWSRHELNVTHVCPREFYETYMPAFKALVQDADVRQVMCAYQRLEDEPCCSNTRLLQRILREEWGFEHLVVADCGAITDFYTTHNVSSSREHAAARALLGGTDLECIWDNYHYKDLPKALEMDLITEEDIDISLMRVLIGRFDLGDMDDDSIVPWAQIPETILNNERHRQLTYEMAQQTMTLLYNPNGVLPLDKTTIQRIAVIGPNADDEEMLWGNYNGTPINTITILDGIKSKLPNAEIYYEKGVDLVDDQVTISYFPLTSIDGSSGFKATYWNHPNFEGEPVAVRQMANSIRQTAAGQHEFAPGVWLEEFSAVYETTFTPTVSEEIVFKGGATGFFELSVNDEVLESYTNWRTLSTRIPFKVEVGETYHIKIRYAHRENWQANIEFDFGREEDVDYAALVKRLEGFDTVIFVGGLSGHLEGEEMPVSYPGFKGGDRTDIELPAVQRNALRALRDAGKTVVFVNCSGSAIAFEPELETTDAILQAWYGGEKGGLAVADVLFGDFNPSGKLPVTFYANSDNLGDIEDYSMQGRTYRYTTEALFPFGFGLSYTNFEIGKAKLSRSKLSGDQTTTITIPVKNAGHRDGTEIVQVYIRKVGDVNGPLKTLRGYQRVDIPAGKKRQAKIELSQSSFEFYDWEQQKITVTPGEYVVYYGNSSHESDLKKATVTIK

SEQ ID NO: 13 - protein, 536 aa, Alkalitalea saponilacus
MKMMKFIEINKAFMIAFLFVLGYSINVNSSMAQGNSPVKITINPDEEGPVINRNIFGHFAEHLGFGIYGGIWVGPDSHIPNTRGIRNDVVEALKEIKVPNVRWPGGCFADRYHWREGIGTPEERRVRINVSWGGAVEPNTFGSHEFFDFLNQIGSEAFVSANVGSGSVKDASDWLEYLTATGTALGDERARNGNPEPYGVLFWGIGNETWGCGGPFTPEEYITELKRHLTFTSNYNPNVNTQFVAVGPDSFDEYSFGYTEAIMEAWADRTWTWDIQGLAIHNYTRGGWPAEIPATGFNELQYAEVIEEALGMDQYIANNRAIMDKYDPDTEVSILVSEWGSWLAPTEGTEPGFLIQQNSQRDAVIAALNFNIFTRHAERVHGANLAQMVNVLQSVIHTEDEKMVLTPTYHAFRMYVPFQDATRLAINFDPGVYQVGDISLPQVDAIAAKGKDGQIYVAITNIDPNNRASFDLSLDGYSIRNVKGETLYANAIDAVNTFENPNNVKPKEIKAQASRNKVSVTVQPQSVTILSITTRN

SEQ ID NO: 14 - protein, 458 aa, Alkalitalea saponilacus
MRGLRLSAALIASLMFLVTNAQNPFVQTMYTADPAPMIYNDTLYVYTTHDEHTTSNFFTMYDWQLFSTTDMVNWTAYGTVASLEDFKWSNVENGAWAPQAIERNGKFYLYCPIHGDGIGVLVADRPYGPFKDPIGRRLVRSSDYIWDDIDPTVFIDDDGQAYLYWGNPGLHYVKLNEDMISFDKSIGNNGVVSLDMTPEAFGERAEPSEKYTTNYEEAPWLYKRGDIYYMIFAAVGIPEYIAYSTAPTAEGPWTYQGIIMGRHPGLAFTNHPGVIDYKGNSYFFYHSEELPGGGGFNRSVCVEQFEFNADGSFPEIIPTREGIVEGVAKLNPFIRVEAETIAWSEGLNIDRDEKTGVFVTNINNGNYIRVRDVDFGRGARNFKASVASGRAGGNIEIRIGGVDGELLGTCKVENTGGDKNWVVKSCRLKRVRGVHDLYFVFTGGEGNLFNFDWWMFSR

SEQ ID NO: 15 - protein, 526 aa, Alkalitalea saponilacus
MKTLLSLVLFVFLLAGCKSQANIEEARDKATNPVVWADIPDMSIVLVDDTYYMASTTMHMSPGLPIMKSKDLVNWEIVSYAYDILVDNDRMSLRNGESAYGNGSWAPSLRYHNGVFYASTFSATSGKTHIYKTTDIENGTWEEISFRPSIHDHSLFFDDDGKVYLIAGVGRITMVELKEDLSGVKEGSEVLLIENASAPAGDNIMLPAEGSQMFKFDGKYYLFNITWVRGGMRKVIIHKADQITGPYEGRLALRDRGIAQGGLIETTEGDWVAFLFRDFGSVGRIPYMVPAKWEDGWPVLGVDGVVPDTLDIPVKNINAAGIVASDNFERESGDNSMPLVWQWNHNPVNEYWTLQERKGYFRLKTSRVDENVLQARNTLTQRTFGPESSASTVIDVSNMKDGDFAGMIALQRRYGFVGVSRDGNSTSIIMVSNESEEPVELERIELNQDKVYLKIACDYNDRNDKAYFYYSLDGQAWTEIGESLQMAYTLPHFMGYRFGLFNYATKSVGGYVDFGHFEISDSMGGN

SEQ ID NO: 16 - protein, 865 aa, Alkalitalea saponilacus
MKKIYTLILLPVFILFLTAGGIYAQTATMVIDNSVQHQNITGFGGFVNGPQFQFNHMTTAQVQQLWGENSQMGYNIMRIYIPVGEENFPQAIPTAQLAQSLGVMLFASPWTMPPEWKTNNHINAVHNGIIGELKEEHYEDYANYLNNFVELMRENGVELAAISIQNEPDYLPGYHGCRWSPEQMANFIRDYGHIITAPIMAAEGIGITDNYANAMLPDEVFNNLGIFAGHQYGPIQTAHKKLQEKGMEVWQSEFLINWNADLPSDRNFTWSIDAFDFAMAVNTALLSDINAWVHYASKRYYGMMGDGTNGTPYGVITKRGYILSHFAQYTTGTTRVESSWRGGSDILDGSAYLSASGDEVIVKVINPSDDPYTLTIDLPFYTNMATSITTTINANMVESTIDIPEETFRPRIDIAASSFTTLIFSIGDDRPESEMEGVQIFPNAIENQFVTNPSFGTDYQMSGQTFIFDNGNHLISPNTNSSNGYLQLDDRYNKLVFHIKEISSPATYTSANTTLYYINRNGQVRSHNYGTISFNQQGNYNWVLDISTDVLTDGITGVIGLRNGNWTSVLSITFGDVYFMIGDEKMYKFSGAYSSGDGFLLDCLEDMTTTSIDFSEVTGIPAGTDWHSMAVNKNAVYYVGEEQGVSAANLISDNISEELILSDVGGSFYIHEDITVGSASYTIQLNGYRIISLPFDANIPEDIGVYTLEYESGHIYGYRVENGGIYANTPVLVVGNGTFTFIGNGLVSTQQQSLVDDMTNVYVSVRAPRNSYVLKNVGGIYSFHRVQSGEQHIIMPFSAYFEFDGSVTAANLPLVLDDVSNINDMPEFQDWNDGDNVYYDLLGRPVRNPQKGVIYIKNGKKVIYQ

SEQ ID NO: 17 - protein, 1190 aa, Alkalitalea saponilacus
MKKCLLRIALLAVLIMVGNQALAWVGMPTPRLHVDGRYLKDPHGNIVNLHGVGITPSPWFNGGHVGEWRWHDFDVEGALAYNNSVIDVLSDPSKGWYMSYIRLHMDPHWTNTPGCTPDAHELPNCFNVDRFIKYLDEVYIPLAEHAISRGLYVVIRPPGVSPHVIGVEDDYNYAEYLMTVWDIVSSHPWIQQQEEIMFELANEPVQIRLADGSVGANTQPHFDVLVEIFQPIVDRIRENGFHNVLWIPGSGYQSHYKGFAVNPILGDNIGYAVHIYPGYWGGVRNYERFRQAWDENVKPVADFAPIIITEIDWAPDGVGAWGDGITGVAGGEGFGANFKKITDESGNVSWNLLMVENLLENGDPDGGIAYGGNPEACGYPTFHWWQEYAGYEYPRPHFENRSISDNGNGTFKNPVIYGDFPNADVILVDNMYYMLSSSKIIAGGLSLLKSNDLVNWEYAVNPLQRAESAHGEGFYSDLIPNGLSRISFHEGVFYIVFNTDNNTYILSSENPEGIWSIDELDTYYDNPVLMFAEGNKYMIHGAGDIMLRELNEDFEAVGGNEVIIGFRDYDFYGTRAYIIDGQYFITSGNVSTGSQIVFRSDELTGPYEESVLLDHTLINSVAIVETQTGQWWSLLSYNHEELGQLPSLYRLEWNDGWPSVRIVSEIMGNMQKPRVGMSFFPTALSTNDNFRYYQLGAQWNWYNSVNHSNWSLFERPGYLRIHTGNVVDNIGDAENVLTQRVLGFKDNDKSYATIRMDISEMVEGDVAGLSILQNPYAFIGVMVENDQPKIIYNNNGTIDIGSEISDAYIYLRIIVNRDEKKAAFYYSLDNEDYIPFGIDFELGFDENLSFANRFAIFNYATIEEGGFVDIDWFSTEEVFNEDMFYDPNFVGYTEDQLILESLSVESSNITMMTGSSRSLNVSALYQDGRVENVARRADILNSSPDVVRIVNGQIVALKDGVANITVTFSGELAGSETIYFDVNVTTFPLTNELFNPSIWESGTFDEETGALITGQWGFGGWTYDQGLDLSDYKYLVVKLKQPTTSGASFRIFNETSYWSTPYSYVVGSATEFVVPLQHMYKVVDGQQVKLDPKALYIIGFWSHGGIPIYIDDVFVSNSDEYYVDIPNSISEMDKPVLSDDDIVDVYSISGVLIRSSIYRRDAVNGLPGGIYIIGNAQKGYLKELVNSNRY

SEQ ID NO: 18 - protein, 580 aa, Alkalitalea saponilacus
MKKSQINYFGKWPMVFLSVFMMIYSFSAVEAQRRANRNAPVFSEFVYQGDDQVYRDYPLEDDEFYSPILQGCYPDPAIVKRGDDYFMVHSSFSMWPGVPIFHSNDLVNWTQIGHVLDRPSQLKVVDSGISAGIFAPAIKYNEHNETFYMITTQFAGGIGNMVVTTKDPFKGWSDPYRLNFNGIDPSLFFDEDGKAYVVHNDAPDPGKELYEGHRVIKIWDFCLEENQVIEGTDKIIVDGGVDITKNPIWIEMPHIYKKYDRYYLSCAEGGTGGWHSQVVFVSDNPRGPYTPAPGNPIMTQRYLNPNRANRVEWAGHADIVEGPDGEYYAVFLAIRPNEKNRVNMGRETFILPVDWSGEWPVFVNGLVPFEPKLKMPKGVVNRTGEDGFVPNGNFTINEDFSAENLDFRWIGMRGPREAFINRTRNGLQITPFENNIKAMAPVSSLFIRQMHNTFTATTTMSYTPRSESDLAGIVCYQNEGFNYVFGVTRKGNDTYLLLERTERGESTILASTKIDVRNPIHLQIRAEGDNYRFNYSLDGTEFKNLGGTVSGDILSTNVAGGFTGNLIGLYATSGNDVQPE

SEQ ID NO: 19 - protein, 712 aa, Alkalitalea saponilacus
MKKNFTVLLTLIFIANYTLSGNLLNDFTPPPYFDTYHEFATDPENWSIFNVHDPTVTKDGEWYYMFNTDVAFGGHNIGTGAMVRRSRDLVKWEFLGTAFNGVPQSAKEFFLPHNPNYDDSGIWAPFVIKVGDEFRLYYSAPGGLDGQNLAYIGFATSQSAAGPWEDQGHIVHSLPNDPINAIDPSVVIDPETGKHWMVYGSYQTGMFVLELDSETGGILNEGDKGVKIAARSGGRHGSIEGPEFSYRNGWFYLFVSYDWLEDFYNVRVGRSRNPEGPYYDINGRDMAAYTDDYPMILAPYRFNHHMGWQGTGHNAIFNDNGDYYIFHQARPSTSIFCMNLHVRKIHWVNDWPVVEPQRYANVPQTPISENELIGQWEHLLLIYNKSIPHQRPSIIELLENGTIDNNAANRWSLDGNKLTMSWGNGQHIDQLIVSRAWDWELRRLTITYTGMNEGGLNIWGKHITQDAVDAVSNVFTDSVYVIRNHNSNKVLEVFNGNDAFGTNIIQNTYTGANSQKWMVENAGSGYVALRPISSSQGRYLEVANNNANNGANIRLGTNVIDNSKRLKFNYQENGYFSIHTASSNDIRSFDVSNFSTQDGANVVQWEYMGGNNQLWRIERIPQSPTSLMKTPELRISIYPNPTTQKSVTIDLNSVNPESNLKISIYNISGSMVEQYEGEWLNQYQTKVRFENGIYFIRVETPSFTYTERVISR

SEQ ID NO: 20 - protein, 917 aa, Alkalitalea saponilacus
MRIKFKPLLTVTLFGVLLGWSCQKWDQMDPPAGNQKNPEPEPPAMDPSYSNVTDPTIGKDNYYYIISSNASLEGVEYEDGLMVRRSVDLVNMTMTEGNEYILSDVISNWAGARLLELDDAVVETNIRIGQPDLVKVGDEWRLYYSVSAGTNASIIGYAVTPSLDDPKWTDMGEILSSEPGMEYKAISPSFCKSPDGGSHYLAFGNSGGGVHIVPLNPATSMPSASAVRVASRADNTLTGNPSMFYHGGYYHLLFTVDNGDLPITAHTYSTDPMGPYSDFSGRSALGIANFWEISRVLSNLQHAGGTAWQRVNGVSVFKDDNNQFFAAHHAVAAGSSEPVLHIRRMEWIDDSRRNVGAGIPVPGISPVRYAGPLPDDITIADIAGDYYYGTIWGHTLSAINDPKSFNADGTYSGGSWDFDPGRGILHMHSTEWGGEDIYIRLFKGHDFEGNNEVIIVGAGINDTFGDFPGVWIRKIGDASGPDPSNVRAGIYDPAMAVDNKYWFFSSNAGVDGFDYERGLVVRSSDDLVFFDDHGYVLSSVINNWAGARLMELDSSIEDEDIMIGQPAIARVGSQWRLYYSVEAGTDASVIGYATSSSLENASWTDQGEVLFSDVSTSYKAMSPSFVATADGHFLAFGEGVGGVHIVELDQSTGMPLGSPVIAVTSSDPNLNVGSPELIYYNGYYTLIATYNNVSVLQSASINPMGPYIDYGNRNLSDGSSFGESRILTPYQFSGGTSWSYTDGIKTWRDGDNWYVVHQARKTDGEDYEMHVRVMNWLEDTRMVTSEQPFPVISPERFSGVESGTVSVDDIPGTWHYGTFWFQGSPASVNNMSAPMMVFNADGTYLHSGEEVGGSWNFDESSQVLHLSSDAWGGEQIFILLNPVFDWDHSVNTFAGGGVNDTFFFHPGVWMKKVVNGQ

SEQ ID NO: 21 - protein, 457 aa, Alkalitalea saponilacus
MLLKKISITILLMGAYCVHAQNPIIQTSFTADPAPMVHDGTLYLYTTNDEDETVDNFFTMYNWRCYSTTDMVNWTDHGVVASLKDFEWSDITNGAWAPQCIERKGKFYLYCPIHGDGVAVLVSDSPTGPFTDPLGHRLIEGTNNVWHDIDPTVFIDDDGQAYLFWGNPGLYYVKLNEDMISYDRSIGNNGIMAVEMTTEAFGSHEGRDGRMRTTYTEGPWVYKRNDLYYLVYAAAGIPEYIAYSTAPAIEGPWTYQGFIMERAPHLAFTNHPGIIDYKGNSYFFYHSHELSGGEGFKRSVCVEQFEYNPDGSIPLMIPTKHGVAESVSNLNPYNRVEAETIAWSEGLKTKKDDETGIYVTNINNDDYLIVRSVDFNNGAKVFEASVASDSDGREIEIRLNNPDGELIGHLTVGNTGGSKSWEMKSCELKKVTGVHDVCFVFKGQEGNLFNFDWWRFQ

SEQ ID NO: 22 - protein, 1044 aa, Alkalitalea saponilacus
MNISSRFLLKFKTTLILLLVSMFCYPQETSDWENPSIIGINKERYRSSLVLPSNKSEHKEIISLNGNWKFKWSPKPDDRPVDFYEVGFDAEVWDDIVVPGNWQLQGFGKPIYLNINYPFKRDQPFVTGEPPTDWFAYENRNPVGSYITTFILDEDLDDKQFYLYFEGVESAMYLWVNGQKVGYSQNSYSPAEFDVTQFIKPGENLLAVEVYRWSDGSYLENQDFWRLSGIFRPVELWIRPKTHIRDYALIAEPSTDFSSARVGAEIEVRNKSNRRIRNLNLEVSISGRDRNGRAVEKILVKPVPTIPGNSTQTVVLNDVIENPRLWSSEDPYLYDVVISLNDRRGEVESFQYHLGVRRIEIVGDVLKVNGKAIKMKGINRHDHHPRTGRYVDPKTTELDVQLIKQGNFNMVRTAHYPHSALFYELCDRYGLYVMCDANQESHGYGIGNLELGDNPDWTLAHVDRVVSMVQRDKNHPSILFWSLGNEGGSGMNFRAMRDTVRAIDPTRIIYCDSDRSVSDIYDDGYLPPNELKELAERITDRPVMLREYAHAMGNSLGNLQEYWDVIEADKSIAGAAIWDWADQSIAKKRDGSLQRYGVDPAMLTLQPDEFWAYGGDFSDIPNDGPFCLNGLIGADRVPHPHYYEAQRVQQYIDFSVVPGSSNVQVISKLDFTSLHEYEYFYEFLDNGKVIKSDQQPLNANNILEIHYPLEVDGELFLNVYAKLRRPTLWADKGFVVAQKQFQLHPYSFSHISSTGQTPVITKSNSSVEVKSTNSIFVFDIHNGALKSWNVNGDELLQGVLEPYFWKPANDNQRRNGYNTRLGSWRDAAKNRVVKKVESRIENGLAVVVFEMSLPVGASYQLKYQINGEGEIQVEAFYEPQTNDIAQMPKFGMRMRLPAEYDEIIWYGRGEFENYPDRKTAALVGHYNKTLEEFITPFVVPQDNANRGDVRWFSFSNGNSSHIRVKGLQPLCFRAWPYQEEDLETTSHNHLLPRRDFVNVNIDLNIKGVGGNDSWGARTMEQYSIDGNKPYSYGFILNVINEEYR

SEQ ID NO: 23 - protein, 491 aa, Alkalitalea saponilacus
MKQIIIKSFSYIILALMAYACNFSDGISISENPYKDDYSDITPLSNRDLWGAANVHDPAIIKSGEYYYVYSTDAYYHKRGVEFNDIGKNIGNIPIRKSKDLVNWEFIGWALDTIPAAAVEHIHNLTGGNGADNMWAPFVYKYENTYRLYYSVSSFGANTSVIGLATALSPEGPWTDLGIVIKTSPEDPMNAIDASVITDKKNGRMWMHYGSYFDGLYCVELDPKTGFTKKEGDLGHLVATRGEYKTRIIEAPEITYNAELDQYYLFVSYEPLFTYYNIRVGRSDSPEGPFYDYFGNNMADTTNNFPILTHSYRFRNHPGWSGNGHNAILNDNGRFFVLHQGRLAPENLMMIMHVREIKWLPDGWPVFSPQRYAGEFPDISIRSKDLVGKWEIIHLNDLPDQVELWQGQIPPGGWTYKDEAFNTSEIVQFGRNGAINHRLASQWSFDGDVLYLDDSFCAIFYGWDWENQKPALLFSGILPDGSGIWGKKIDD

SEQ ID NO: 24 - protein, 523 aa, Alkalitalea saponilacus
MKILILLTFIVIIGAFGCKANNNVARSSETIELIINQNKKYQIIHGFGASDAWSCQFVGKYWPEDKKEQIADWLFSSKFDRDSNPKGIGLNMWRFNIGGGSAAQGRNSGIRDEWRRAESFMVGDSQYDWNQQSGQRWFLKAAQERGVEHFIGFLNSPPVFLTRNGRAYSSDNHRYNLPEENYSAFAVYLADVVENVEKNDGVFLNYISPFNEPQWDWIDGGQEGAPAQNSEIAAITRIINQKFEKRNIVSQLEIPETAHYKYLYESNDKPGRGSQIRAFFDPESDNYIGNLSRVTPKIAAHSYFTTWPTENLVETRKRVREAIESNPMSIEFWMTEYCILENNSEITGPGRDLGMDAALYMARVMFADLVFANAQSWQWWLGVSPYDYNDGLVYIDHDKYDGEIYDSKKLWAMGHFSRFVLPGMRRVQVSRGDNIQDEAALESLMSTAFVSDDGQYTTMVLINYSETSIPFVMTTENGEFNTEFKYYLTDHRSENNLTRKGTIGIGDVVEMPARAMITITNVN

SEQ ID NO: 25 - protein, 729 aa, Alkalitalea saponilacus
MMIKRFYWLLLAVLFYSTTSCQTEEGLVLHYDFSRTTGSGNVVRDASGNGYSGEVHNNAFFESLGRIGILNLGSENGFLDMGAKTGELISSLEDFTVATYLYVDELTDLTAHGNFLWNFGNSDNLAVEQNGSMFFSARTTGYTISRQHWSGEQGAARLLTFPKGQWHHVAYVQKGNIGTIYLNGSRTAESSVTILPSVLGKTTHNYIGRSSYRGDAFLRNAKVADFRVYNRALSNEEMERFRNLTNKLQRATIDKQLKSAAQTALPGSFANVVENLELPSVVEYGVSVKWSSSKPDVLSDEGAINRPAEGSKAASVTLTGLFTKNGQSYSEKYTVVVQPWLSERASVEKDIENITLIGNVNNLRTDMILPVSGIEGTTIRWESSHREFLSDNGKLINLSPIGEGKKLVTLTAHVSKGSESKTRDFEVYVAEDEGYVAYLFSYFIGNGPGEEAIFYSISHDGYNFRALNNNRPIITADTISARGGVRDPHILRAPDGYFYMVVTDLYVPNDGWSGNDAMVFLRSSDLVNWTHAKINIADKFEEFSDVLRVWAPQSYYDEEKGKVMVYWSMLQPGGYDIIYYAYANEDFTGLETVPKQLLYHPDEVACIDGDIVYKDGVYHLFFKTEGAGNGIKKAVSDRLTEGYVVQEPYLQQTNDAVEGSCVYRLINTDTYILMYDVYSRGSYQFTKSTDLENFEVIDHKISMNFYPRHGTVIPINQEELNNIMTRWGR

SEQ ID NO: 26 - protein, 555 aa, Alkalitalea saponilacus
MKKRVFIVSMAMLMFFQLTSQNRNLKLHYDFKSVTPSGEILDMSGNGFNAELKNEAFLDHMGDYHILNLGFHNGYLDMGEKTGELVNSLKDFSVATYVYVDEGVSLSLHGSFILTFSNSTDIRSDGNGCMFLSARDQAYAITKTDNRAEQAVRVGEPVQQGAWMHIVYTQEGNQGNLFIDGKMVASNTVDIFPSAIGKTKFNFIGRSPYKEDNYLRGLLADFRIYDKALTAREINRLGRETSGLAEAHVEYAQRPIRLIANGNPLFSHKYTADPAALVHDDVFYIYAGQDVGDGRGYNMPNWVVFSSEDLETWYEHPIPLRPSDFSWARGNYAWAAQVIERDGKFYWYVSTQHYTGARAIGVAVSDSPTGPFVDAIGSALITNDMTTHCTNITWDDIDPTVWIDDDGQAYLFWGNTCCYYVKLKDNMIEMDGDIMTIEDLPHFTEAPWIHKKNDWYYLSYAAWFPEKTAYARSKSINGPWEYMGILNEVAGNSNTNHQAIVEFKGQWYFVYHNGALPTQGGSYLRSVCIDYLHHNEDGSIQRVIMTTEGVNPVRD

SEQ ID NO: 27 - protein, 1047 aa, Alkalitalea saponilacus
MKTLFSLLSIFIFFALSTNISAEKRKDWENQHVFDINKEKPRASFYSFPLLDQALTFNREESPYFKLLNGTWKFNWVPKPGDRPRDFFMESYDVSGWDEIEVPSNWELNGYGVPIYVSAGFGFTNDPQPPKIPHDNNPVGSYRKDFNIPDDWSNRQVFIHLGAVTSAMYIWVNGQKVGYSQDSKLPAEFDITPYIRSGSNTLALEVYRWCDGSYIEDQDFWRLSGIERDVYLYSTPKFRIRDFFFKTELKNDFRDAEVKVEVDLRNHLRSTERGSVEIKLIDGDQVALKTTGQVRSNGNDDTQIVLEGFLQNIRLWNAEEPELYTLAVTLKDRRGRELESLAVKVGFREVKIAGGQLLINGKAVLLKGVNRHDHDPFTGHVISEESMIQDILLMKQNNINAVRTSHYPNDTRFYELCDKYGLYVVDEANIESHGMGYGERSLAKDTTWMAAHIDRTRRMVERDKNHASVIIWSLGNEAGNGSNFEATYDWIVARDLSRPVQYEQAATGRNTDIVTPMYARIDRLVGHGTSIQDRPLILCEYAHAMGNSVGNLRDYWDVIEKYENLQGGFIWDWVDQGLAKYSDDGTLYWAYGGDFGPEGTPSSSNFCMNGLVRPDRSPNPSLHEVKHVYQYVKIEPVPFTSNQIKIENNYDFASLARFDFRWEVRSNGKTKLSGVISAPHIKAGEKSQYVLPLENLNIIPGEEYFVVIRKVLNQDWGILSKEHELAAFQLEIPNTAGEKYYPSYESLNFQRASGEFRYSGDDFEIAFNQNTGELSSWISNGLELIDNGPKPNFWRAPNDNDYGYQMPQLLDIWRHAADSARVVRVESSSVQNGKASVTVEYALNRDAGGCELTYTIYGSGDLIVRMRFKPGKNDLPVLPRLGMMMSLPGRFNNLTWYGRGPWENYPDRKTSAFIDLYHSTVADQLEWYPAPQENGYRADVRWLKLTDDDGNGFLIEGEELIGFSALNFTPEDFTLPGRGQIHTIDLNPRDEVYLNIDHKVMGVGGDTSWGARPHAKYSIMPRNYEYQFRIKAIDKNDNIKTGFDFLK

SEQ ID NO: 28 - protein, 705 aa, Alkalitalea saponilacus
MRVPSDFIKKIDLRMKKMILSVCLLLMVSFSYPQSAERFYPASELISVGAYYYPEHWDESVWERDLKQMAEMGFEFTHYGEFAWAQLEPEEGKYDFDWLDRAIELADKYGLKVILCTSTATPPVWLVRKYPEVLITHEDGTRMDHGARQHASFSSSFYREYSQKMIAELAIRYGNDERVIGWQLDNEPRTSVDYGSDAHERFRAWLKEKYGTIEALNKAWGNDFWSGLYNDFSQINIPLHSQWGMNLHQRLDHTRFSDWETSSFMDKQARTIRKHIKRDQWITTNYIPMYDVRYIGQSRELDFVTYTRYMIYGEGLGVGRKGYRIGEPLRIAMANDYFRPLSEIIGVMELQPGQVNWGQINPQPLPGAVRLWNWHVFAGGSKFTCTYRFRAPLYGYEQYHYGIMDFDGVRPSPGGLEFQQFIEEINLLRENYSGSSVPDDYLKRYTGVLFDPNNAIAMAHNPQTTEWHTENHVLKYYKALKSFGAPVDFVRDTMDISKYPVLVVPAYQQISRDLIQNLTAYAQNGGHLVMTVRTGHQDPYGHLWEAPYAQPIYDLIGSEIEFYDLLMPHAPDNVKMDGEMHPWTSWGEILKPFPGTESWATFEDDFYAGKPAVTWRKLGNGTVTYVGVDTHDGQLEHKVLTRVFERANIKTESYPEGILVEYRDGFGVAMNYSDKNYEVKIPSGSQILVGQPNIAPAEVVVWKVE

SEQ ID NO: 29 - protein, 860 aa, Alkalitalea saponilacus
MIRKITLAITTALGALFFLSCETSKENLPMVIEISQNWTFTQNGQDNWMPAAVPGTVHTDLMNNGIIEDPHYRLNENDVQWIENEDWIYQTTFKVDSEILDSDVIKMNFKGLDTYADVFLNNNKILSANNMFVGYSVDVKEHLTEGVNTLRVYFHSPVRVGMKKLQQVDYYIPSINEQAPDDKRTSVFTRKAPFHYGWDWGPRLVTSGIWRPIYLKAWNQAKIEDAYFHTTSANSDLAKITGHVELNVLNKGTHQVQLIINGQKSGVDIQTELEEGKHQIPFNFEIENPNLWWTNGLGEPYLYKFELRLVQDNLIIDKYDLNYGVRTLRLVQEPDELGRSFYFELNGVPVFMKGANVIPSETLTPSVTPEVYERLLKNTVDANMNMLRVWGGAIYEEDLFYELCDQNGILIWQDFMFACNLQPGDEAHLENIRKEAVYNVKRLRNHACIALWCGNNENLHGWHEWGWKEMYEPDVRDFMWRTYERIWHEILPEVVAKYDPKNSYWSSSPMAYGNQKADRKSGDEHDWTIWFGQEPFTSYGKNVPRFVSEYGMQAFPGMHTISDFSVEEDWDIHSEVMRHRQRGTMEYIEPGFDGNDMIKRYMERYYNVPDNFEDFVYVSQIMHAKCYRTALEAHRRNMPHCMGSLYWQINDSWPTISWATVDYYGRWKAAHYAVRKANEEIIISAEVDGNAGRIYVVSDRLTPVENARLHIKIMDFFGREIFSTSQNLTVKANTTMMVMENDIRELQQHANLASTVVSMKLTDGSTTLADNIFYFHKPKDLLLPEANITWSSEKTTDGYTITVTTDNLAKNLFFDTPYGDVFFTDNFFDLLPGESKTIELITKYDINLNEKLKIKHLNGL

SEQ ID NO: 30 - protein, 986 aa, Alkalitalea saponilacus
MKKKCLVIRSLLSLFLLAVAGELVSNNNQLLASDADVGSHSSSIISFSAVDGYFPLAVSGKPVPLYTHSDDYQGVIRALKDLQSDFELVTKNKPKLSINSVPKSKRVVIAGTLGNNQVIDKLAEDGKINAEELDGKWEKFIIQVVDNPVKGVDQALVIAGSDKRGTIFGIYEISRQIGVSPWYWWADVPVSHQPNLYVSPERFTLGEPKVQYRGIFLNNDEPALGNWVRHSFGGFNHQFYEKVFELILRLRGNYLWPAMWGKAFHDDCPHNAPLADMYGVVIGYTHHEPMMRAHIEWARYGEGDWDYQTNEEGLREFWIEGIERMKDYESTVTLAMRGDGDEPLSEEANIELIERVVNDQREIIQNYAKNPDDVIQVWALYKEVMDYYNRGMEVPDDVLILLTNDNWGNIRYLPDPDDAAKRSGGWGMYYHFDYVGGPRSYKWINTIQISRIWEQMNVTYRHNIDKMWLVNVGDLKPMEFPISFFLDFAWNPDAIPADVMGQYPKWWAQQQFGKEFAEEIAHLLNEYTRINSRRKPELLNEDTYSIIHFREGQRVVEDYNNLLKEAERINEKISEEYRDAFFQLVLYPVKASANLNEMYVSVAKNRLYARQLRSNTTEMADKVRYHFDMDAKLNDKYHSIADGKWMHMMSQTRIGYTYWNQPPWDVMPNVTVATPHDPADMGVAIEGSGYAWPQAGRNRQDAVLPKFDKFNQQSFYIDVFNRGRFSFEYSADTDVPWLLIDNPTGTVEKQERLLVSVDWTQVPEGTHRQPIRISGPDNRNIIVYAEVFNPSYPVREEVQGFVEANGYVSIEAPNFTRKIDSEDAWWKYVPDLGRTYASMVSFPVLADVQTPGDQDAPRLEYDMHLFSEGEVTVHVYLAPTKNFKHERTGLKYGISFNDEDPQIENIHTEILNWGDYSYGAPEYGVWASWVSNNINVLRTTHTIDKPGKHTLKIWMKNPNVVIQKIVVQTGEMGETYLGPPQSFFNK

SEQ ID NO: 31 - protein, 542 aa, Alkalitalea saponilacus
MKKIYFLPFFLFCFLGVNVMAQGPIHDPSHIIKGDDDRYYVFATGLNSDNGNTTVGIYGVSSSNSNFTNWREEPSPVDHINFPDWINTYVPGFNGHFWAPCIIYMEGYYYLYYSASNFGTSNSIIGVTRTPSLANPTWEDLGLVVSSDGTRNAINAIDPAMFKDDDGRVWMSYGSYFGGIGVIEINPETGKTIGSLTHIYGGNHQDIEAPYILKNGPYYYLFVNRGSCCRLLESTYYVEVARSTSITGPYTGTREFLPVQHGVIVGPGHIGFGEGVLSYHYYDGFSNGYPRLLTTTLDFINGWPVAGPTGVEMGEINGVFALVANHSNKAVTMEDAIPDFGTNIAQYTYNGGDSQKFKITSEGGIWHTIKPAVNDFFAIDVFEISTDYGANINLWESLGHVGQQFAFQVDGNGYRIINRNSNRCFDVQNASHADGTNILQWGCFGGNAPQQTFRLVDLQGTNIEEEQLPKSSVTPNPSNGSFNVILEQDNLRIRISNYLGQTLFETIGHKGSNSIDTPLKTGVYILNVESYNEYESHKLVIK

SEQ ID NO: 32 - protein, 777 aa, Alkalitalea saponilacus
MKFKTIIQYYFMHIIKALSLLVFVAFLLGCTCSSSDTVERIPYVEALIKQMTIEEKVGQTAQITLDVITKGGGHANYGGLQIDTAQINDALVKYHVGSVLNTAGNRALNVHTWHHLISSIQEVATNDTRLKIPVIYGIDAIHGATYTAEATMFPQQIAQAATWNRDLVYRIAKATALETRASNIPWNFSPVLDLGVDPRWARIWETFGEDTYLISEMGLEAIRGYQGKELNCSTRVAACLKHFIGYSTLASSGKDRTPAEISDISLREYHLPPFQFAVESGAASVMINSGLINGIPVHGSYDIITGLLKNELGFNGLVVTDWADIENLHNRDKVAPSHKEAIRLAFNAGIDMSMIPYNYVQYCEMLVELVKEGAVSMERLDDAVRRILNLKYKLGLFERPFVEPSLDAFSDAHKKIAYMAASEAITLLKNEKEILPLSKGTKILVAGPNANSMRTLNGGWSYSWQGEGVEEFTEDKNTILKAIEMKFGKRNVIHVPGVEYDFNGRTYRDEHNVNIEAAVNAARNVDVIVLCLGENSYTEKPGDLSDLMISENQEKLAIELAKTGKPVILVLNAGRPRLIRRFADDMSAILQTYLCGNYAGDALADILAGDVNPSGKLPYTYPMFSNSLVPYYHKHSEESESPEGVYNYEGGVYHQFSFGHGLSYTSFKYSNLAVSHVEFTNNDELLVSVDVENTGTVEGKEVVMLFASDLYASLAPDVKRLRRFDKIHLYPGETKSVTFSLSANDLSFINAQSKRVTEPGEFALKIANLYKTIKLIE

SEQ ID NO: 33 - protein, 810 aa, Alkalitalea saponilacus
MKNKLLIILFLFLLSFPAWLMSGGKYHIDLSDVNTEVLRGHLDLGGQSLSGEIIEVNSFYIERNGEPYIPVIAEFHYSRYPREYWDEQIKKIKAGGVTVVASYVFWNLHEFKEGEFDWSGNLDLRHFVELCGKNGLDVIVRIGPFAHGEMRNGGLPDWLYGRPIEVRSNDPAYLYYVNRLYHQIGEQLSGLMFKDNGPIIGIQIENEYQHSAAPWAFTYQGAPRENTVARRDVDITQIGVGVNEFGNEFAGLGRDHMKTLKMFAIEAGMETPIYTATGWGYATIVEKGSIPVMAGYAYPFWVPDNRPSPFYLYKNIHRNPDYSPVSYDVNLYPSMAAELGTGIAVTYSRRPRVPGESFLPMMVRTVGSGTNGLGFYMYHGGTTPSIGNFFMTEGFGLANKSYDYQSPIGEFGKASVGYYPLKLINYFLQSYGNVLAPLYPVLPESNESITPDNTETLRYAVRTDGISGFIFMHNFQDRIAMPDHRDLHINVNTIEDSFRFPHDGTFTLKSEASGIFPFNLDFDGVFLHQATAQPFMRFENDGRVYHVMVAIEGFHPQLVLNGDTDVSGTGIKTELINGRKVVSFPDDRLSEMVSNDVSFLVIPYEMALKAWLTGKAGNQHLIISNALVLEDEKSLSLISDHQTDICVRVYPAIRDLRSGEASVKKLEQELASVSGWILSIDPKEPVLQLIPSGDRHFVLRAEQLDMNGINDVFITFDYRGDRAVCMMNGELMTDHLYTSAPWTIGLKRYVEMLKNHEMYFYFIPMRSDAPYLNWLDEEVVPDFGERREFLEIKEPEISVEYRIDIILDKN

SEQ ID NO: 34 - protein, 692 aa, Alkalitalea saponilacus
MRKITVCLLFFALLFHAWGQDANRFFPEDRLLIPGAFYYPEHWPEHQWERDFEKMAEMGFEFVHMAEFAWAFLEPSEGVYDFDWLDRAIDLAAKNGLKVMLCTPTATIPVWMGIKYPDTYLMNNQYRRAEHGSRQNNSLVSGKYIELSEKIIREMAKRYGDHPHVWGWQLDNEPYAKDDYSPAAQEAFRQWLKNKYQTIEALNHAWGTAFWSITYSSFDEVRIHNTGAIDWWGNNPHAVLDFRRFTAWVQANDLDRQALILREYINPDQFITTNYVAVPGNADPRLTENLDFISYTSYPNNGTPNLGEYGFRLGNHTALMLANDYFRPINGVTGVLEIQPGQVNWASSNPMLMPGTVHMWLYHSFGAGSRLASSYRFRQKIYGVEQYHDGMLRTDGVTPSQGGEEYITFIEELKMLEGMDVDTEMPEDYAAKTTAILWSHDNMWDHNRQPQNDRWNIWNHTLKYHQILKSIDAPVDYVSESCDWSRYPTLIVPAYQSVDSVLVEKLTNYAKRGGTLVVTCRTAKKNRFGHFWEAGWSAPIYDLIGAEIEGYDMLPGYKHATVEMNGKEFKWNRWGELLKPFKDEYAVAKYSDQFYAGKSAVVQREIGQGTVTYIGVDTETGELEKQLIKGLFKNRGLPVSNLPEGVFSYWRDGFRVAVNYSSEVYEMPLPENAKIVIGEKKLPSPGVLVWIE

SEQ ID NO: 35 - protein, 771 aa, Alkalitalea saponilacus
MKNFFFLLCTLLFSTNLIATTITLQCENMNPHSPGGFGLITDQPTNGVWLYANGDQVSQTVTLPEVPGTYLIEVRGASDGSSQADAQLRIGGTTIHTFQFSGTDLQTLNIETTLSGDSEKEVILIRTQDDGTSNTFLDFISITLQEDSGDNGDPDTPGNDDEITLQCQSMNVHSPHGFGLITDNPTNGVWLYANGDQVSQIVTLPETSGRYRIDVRGASNNNNAAGAQLRINGDNIFLFSFTGTTPAIISREVNISGDNPSIDLLLIRTDDTGASNTFLDYISITYLGEIPPPPPPPVIPEEGAIYSGQYRNMFLEAGYTPEEIDDKINDVFNQLFYGDDDTERVYYPVGNDMAYILDAANNDVRTEGMSYGMMIAVQMDKQEEFDRLWNFAKTHMQHGPGNREGYFAWVVNRDGSIIDQNTASDGEIYFVTALYFASVRWGNGDGIYNYRAEADYILNQVMSKGWPHNTIIGSVPNMFTPDHQVVYVPYATASEFTDPSYYLPAFFEIWGMMADTNNEFWYQAAEVARDFLYDAAHPVTGLTPDYANFDATPRQQGEKMHFVVDAWRVIMNVAMDYAWFKKDERQKELCMRIQSFFHSEGMYTYWSGYELDGTPLPGRNHQSAGLVACNAVGSLASDDAMAWEFIHSLWNREPTTGQYRYYDGMLQMMSLLHLAGEFRAWTDNFSTSTPEAEGSYKPSISVFPNPSTGNITINTNDVIDQIIISDMSGKVILNRRSVSEPTVNITNMERGVYILTAQSGNQIFTEKIIIR

SEQ ID NO: 36 - protein, 771 aa, Alkalitalea saponilacus
MRQYLKHDEWRIIEEGFNPDYQRASESIFSLGNGKMGQRANFEETYSGSTLQGSYIAGVYYPDKTRVGWWKNGYPEYFAKVLNSPNYIGINVEIEGEQLDLFKCKTEGFVRTLDMQKGILSREFKATLNNGKQVKVDATRFLSMSEPECAFIRYAVTPLNFTGQLAFEPYIDGDVENEDSNYDEKFWNILTTNSKNGEGELLVQTKKLDFRVAYAMNWDINTRNHKVSSSHNAARTSNRVEVKASENETIIFDKFIGVTSSLNHQNEQLISKAQQRALQAKTVGFDKMLKIQINHWATIWEHSDIKIEGDVAAQQGIRFNIFQLNQTYTGDDERLNVGPKGFTGEKYGGTTYWDTEAYCIPFFLATAPQHVTRNLLVYRYKHLQKAIENAEKLGFTGGAALYPMVTINGEECHNEWEITFEEIHRNGAIAFAIYNYIRHTGDEKYLEEYGLEVLIAIARFWAQRANWSGEKQKYVILGVTGPNEYENNINNNWYTNKMAVWCMTYAAKALKIVETMNPSRYQAILENINFKYAEETAKWAEICEQMHFPFNKNLNIFMQQDGFMDKEQMMADDLPASTRPINQHWSWDRILRSCFIKQADTLQGIYVFEDEFDTDTIRRHFDFYEPRTVHESSLSPCVHVVLAARLGKQDKAYDLYLRTSRLDLDDYNNEVHEGLHITSMAGTWMSIVEGFGGKRVKDGKLHLNPIIPQQWKSYAFMVVFRGNYLEVKVSQDNIEIISHAKNEATLMVYNEKVTVKPSESVTLSLKPTYYA

SEQ ID NO: 37 - protein, 801 aa, Alkalitalea saponilacus
MLKFRFIIPQIFLIIPLAALWGSPAGNNNKVSLINHSQTRDCLVLSTNEGHIRMAAVTPNSIVISFCRDSIFSDPSDALIAHPGSQPLIIQEQDSRIMTRMGQNQVTIQKKPFEISLRTGSQHQETILIHGSMQNGNSTGVSIQLQPGEKITGGGSRAIPMDRRGYQLRLNNEPHWGYAWGAENLNYSVPVFVSDRPYLIFFDAPQRATADIGYSDENIFRLESNKENFTVYIVTGNDHKETLKEYTLLTGTQPLPPFWALGHLQSRFGYTSQEHAINVADSTIMAGFPLDAMIMDLYWFGKGIGDFRMGNLTWEAENWPQPQKMIDHFLDNGVKTILITEPFFLTDSDHYDEMAQKGYFGKDSTGNAFVIDDFWFGPASLIDVFNPDAMEWFWSKHVPHIEKGIAGWWGDLGEPEKHPAGIYYKAGSSDEIHNIYGHYWSKMLHDKYREHYPDQRLFFLNRAGYAGSQRYSVFPWSGDVSRCWNGFRAQLPIMLGMSMSGIPYMHSDLGGFAAGEKDDELYTRWMQFGVFNPVYRPHGESIPSEPIYFSDDAQDVIREFIKLRYELLPYLYTMSWQQTTKGTPLARPLFYEHPDKSEFFDIYDTYYWGDNLLVAPVLEPGITSRDVTLPEGYWIHLFNNQIYSGGQTISVETPFENIPVFVKAGSFITKAKPVMSTEYFSTDTLLVSYYHHPKTENGHGQMFMDDGENPTSIENGEYELVSYQATNTGRQLKIEVNCNKGNYYGKPEQRHYNVIIHNLEKEPRRVNINGRRSDFSFDEKRSKLIIPFNRQREKIEIVIRK

SEQ ID NO: 38 - protein, 535 aa, Alkalitalea saponilacus
MRFNLTDIRMRLVQKSKFGLLSIILVTFFGTVACAQVKPVATIPYEIAPIVAPFEMIQLERPTFPNRVFNIVDFGAKEMGSDKSFKSTEAIHRAIDAAHAVGGGKVLIPAGNWLTGPIHLRSNIHLHISEGSTVYFSEDKEDYLPVVIQRYEGVEVYNYSPLIYAYRVRNVAITGKGVLDGQAGHWLADWTVQPRAEATKVPLSRRTNFGKGSGTEGMRPNFVVFWESEDLLIEGITVNNGPMWNLHLVYSQRAIIRDVTINSRDSHNGDGIVIDSSRDVLVEHTTLSTGDDAIVIKSGFNEEGLEINIPTENVVIRHFHAYRVVTGSGGVVFGSETSGGIRNIYVHNALFEDCDRGIRFKTARGRGNVTENIYIRDIEVINSTYEALNFNTFYTGAGVGPAPLLRNIDIRNIRIDGVPRAIVLNGLPEKWLEDIYLENIEVVNAREGIRLHRVKNLNMRNVSIQSEERAMVAHDVYELYLDNVSLSDKKGEEPIRLEGKYTGVVVMPNYEPGMVSFDRDVKEDVIRKELPTAAW

SEQ ID NO: 39 - protein, 622 aa, Alkalitalea saponilacus
MLKKSRFIILMLLATLLAGNGNQSFASNIKERLEPASWWIGFQNPTVQLMAYGKDIALLRPEIDYPGVSIERIIAVENPNYLFIDVNISQNANPGKMEIRFRDGRRVRTTRTLELLTREKGSAEREGFNQTDAIYLIMPDRFANANPNNDMIPGMLEKPNRDEPYGRHGGDLQGIKERLDFIKDMGFTAIWLNPVLENDQPEASYHGYATTDYYKIDRRLGTNEEFKALVDASRERGIKIIMDMIFNHCGSKHWWMNDLPTEDWVHQYPEFTRSNYRLSTVSDPYASKADFDLTVCGWFDTTMPDMNLKNELVLNYLTQKSIWWIEYAGLQGIRMDTYPYPDKDAMADWVLRVKKEYPDFSIVGESWIGNTSQLAYWQKDFPNQDGYNSYIKNLFDFPLAYAISSAFNEGEGWDSGLQRLYDVLADDHLYRYPKHLVVFAENHDFGRMMHFFNDDINKMKLAIAFLGTVRGIPQWYYGSEILMGGDGAASHAAIRQNYPGGWPGDEVDAFTRAGRTAEQNEVFDYLTTVLNYRKNSHVIHHGNTLHFVPQNEVYVYFRYLDGEAIMVMMNNNNENNTEVDMSRFNEILANYSGGREIVTGKRYEKLDKITVPAKSALIIELK

SEQ ID NO: 40 - protein, 250 aa, Alkalitalea saponilacus
MIMKRLNLLILVMIVMAACGGVAKFASEKGAEESKVLTFCSDPDNDQFKGEHDGYAYELWNQNGAGDACMTIGAGALFSGHWQGIDNYLARRGLVFDETQLHHEIGRFSTTYSCIYEPTTESGNSYLSVYGWTVEPLIEFYVVEDWRRWIPSMAEGSQLKGTFEIDGSIYDIYESTRYNQPSIIGDATFQQYFSIRRDVRNSGSIDISAHFDKWESLGMELGKMNEVAFVVEGYMSNGRFEFTELEVKVE

SEQ ID NO: 41 - protein, 958 aa, Alkalitalea saponilacus
MKNLLFNLFLVLLVASCSSRDAMEIDLSGNWKFKMDIHDEGVEGRWFESRLPDLMVLPGSMMEQRLGLEITLETQWTGSIYDSSWFFNPHTEPYRQPGNLMFPFWLTPEKYYAGAAWYQRVVKKPSNWDGQRVFLHLERPHWETTVWVNESKAGMQNSLSVPHVYDITDLMSKGENVITIRVDNRIKDINVGPDSHSVTDHTQGNWNGIVGDIKLIARPNSYIQNVQVYPDVASNKVRLVGKMVNKSPKKFSGEIEVLATLTNVNVSASPVLASFPVTLEAGEQLVELEFDMGENVQLWDEFHPAFYRLEVSLKTDAGATDVFRTQFGMRTFTAEGTRFAINGRPVWLRGTVECAAHPLTGYAPMDKEYWKEIYQKAMAFGINHFRFHSWCPPRAAFEAADELGVYLQPEGPFWTNHGTWVGDGLPVDQYIIDECDRILEEYGNHPSFVMFAYGNEPAGRNQIPFLNELVEYWMEKDNRRLYTHAAIGRSWPLAPSNEFIIRAESRGLPWDQRPQSLFDYAERIAPYDVPYVAHEMGQYCVFPDFNEIPKYTGVYQPKNFVMFKAELERKRMGDQAREFFMASGHFQVICYKSEIEASLRTPGNAGTQLLALNDFPGQGSAIVGVTDVFWDAKDYVKPEDFRRFFGTTVPLTRFPKFVYTNDEELLVEAEVAHFGEFPLQNVTPVWKITDENGQVIDEGTLPPTNIPFGNSELGAIRFPLDFSMEAGKYNLELSFKGFVNDWDFWVYPAELPELTGDEIFITDDFNDAAVEILNNGGDVLLLAAGNVEKGKDVVQYFRPVFWNTSWFQMRPPHTLGILTNPNHLAMADFPTDFHSNLQWWELLHNQQVMNLDNFPAEFKPIVQPIDTWFINRKLGLVFEVRVGEGRLLVCSADLDSDLDNRIVARQMRHSLMNYMLSDDFNPAITVDPDLVAELFTEGDYDIYDVHTAGSPMDLIPEQ

SEQ ID NO: 42 - protein, 970 aa, Alkalitalea saponilacus
MISFRKVLFSVFCWMIFFVPAISDHFIKHGTNYPLTILYDEADDQPVQIAVMALADDLELLTGIRPLIKTSVEEVSGEAIIIGSLAKGRYIQQLIDLNKITAENVMDLWEVYSIQSIVNPLDQIEKALVIFGSDKRGTAYGVFELSERIGVSPWHWWADVIPEKRKAVEIDQMNFVSKSPSVKYRGIFLNDECWGLNPWATNTWEPEEGNIGPRTYAAIFELLLRLRGNFIWPAMHPCTNAFYKNPENPKTADAYGIVVGSSHAEPMLRNNVDEWDHEKYGQYNFFTNRETVLNYWEERVKESSGFESIYTLGMRGIHDSGMVGAETMQERVDALHDIISQQRELLSKHVNTDPAKVPQAFTTYKEVLDIYDAGMELPEDITLVWPDDNYGYMHRYSDAEQEKRIGGSGVYYHISYWGRPHDYLWISSTHPALIWEEMIKASYFNSNEIWVVNVGDIKPLEYNTSLFLDMAWDTSCFPDGASVRKHFDRWHKNIFGDEAGQKIADVKWNYYDLNFQRRPEFMGWSQTEPTRKVHPTEFNHFQAGDEAQKRIDAFNSLTQKSAEITEMIPERLMDAYYQLVEYPLLGAAYINKKFLYMEKAYYYAAQNRIVANDYALKSKAVYDSIQFLTDYYNNEMAGGKWKNMMYMSPRSLPVFDMPAIPQWTFVTDSHWGIATEGAKDVRRVNEIKGPLYLPSFNNLLHQEFFIDVFLKEDKLLEWKAEVSNDWIVLSHSSGVLTGEKESRQQRIWVSVDWDRVPTDVRANGYIRFSGAERNYTIQIYTNRHNPSIPDKHIFVEANGYISIHAENFNRKHATESFEWGIIDGLSYTGQSVWVNPLLIKEKQFDPELNNPSVLEYDIYTTRGREVEVTIYAIPIHPINQNYGARLGVAINDEVPQIVDHQTYGRSEEWKINVLRNSAVVKTRHEISSAGHHTLKIFALDPGVIIDRITIDCGGLISTYSVLEETIVFDQ

SEQ ID NO: 43 - protein, 596 aa, Alkalitalea saponilacus
MVLVKLHRYKIFGFIFFLFFWTLLSLNCGEAYTEKSNTSVVCFWEQLENESRIWVDSVYNSLTLEERIAQLFWIAVENPTNAAAFRRAISETQTYQPGGILLFRMSPETALEVIDEFQKVSNTPLFVSIDGEWGLAMRFPDVEPYPYAMTLGAIQNDSLIYRMGRKMAHQFRLCGIHINMAPVADVNSNPANPVIGFRSFGEDPDNVARKSIAYMQGLQDGGVMAVGKHFPGHGDTSTDSHKTLPLVAHSRQRLDSMEIYPFKRMIDEGLWAVMSAHIEIPELESEAGLPVSFSQKVLKDLLRDELEFRGLVITDAMNMEGARVMGKPGERDVLALAAGNDIVEFTEDLPAAIIAVKEAIENETLSLEEIEDKCRRSLAFKYWLIARKSMEKDAIDDDTDSLMKMTSTENILELLNNEKVNELNRELYEAALTLLRNENDVVSWFENQQYEGAFILLGEAPAMLNKISNRFDCPVYQLPLNNPSLFIQRVRQLEKYRQKVFVITDTRWGSRAGNATQLAEIGALADENSVVFFLGNPYHLENYEVLTNASGLIVAYQNNEQAQLAVINMLSGHVNFSGRLPVSVGELFNVGDGIKR

SEQ ID NO: 44 - protein, 568 aa, Alkalitalea saponilacus
MDKHRFVIYQLLPRLFGNSNNINVSNGNIDQNGCGKFSDVSKEALTSIAGLGATHVWYTGVIEHATCSDFSKYGIASDSPDVVKGQAGSPYAIKDYYDVAPDLAVEVNNRMAEFENLIARTHAADLKVIIDFVPNHVARNYTSDAAPKGIEPFGKKDNKKVSFAKDNNYYYLPGTTFKSPLQITNIKPWKESPARATGNDCFSPAPSVNDWYETVKLNYGMDYQGGTHADFEPEPDTWRKMLDIVLYWSQKGVDGFRCDMAGMVPVEFWRWMIGEVRAKFPEKLFIAEIYEAERYEDYIFKAGFDFLYDKVVLYDTLRNVMEGKAPASELTDCWQKTDGLHHFLLYFLENHDEQRLSSDFFMANGHKAIPGMVVAATMFNNPLLIYFGQELGERGMDEEGFSGRDGRTTIFDYWSIDLIQKWRSNGDWTGTELPKAAADLRSFYQKLLTIIHQKPAFYKGRFYDLMWVNRHEFFCHDKIYAFMRYEGGHCFLILANFSDKQQSFKLKIPLDAMDTCGMKNELFYNGIDLLGFNRPLQFPAAVASNGGLGGRLEPYTASIYELKGHVLD

SEQ ID NO: 45 - protein, 323 aa, Alkalitalea saponilacus
MKRNYFYFTLSLVLLLVSCHQSEQDQVVGNPLFGGYFGADPAIVEYEGKFYIYATKDPWGGDDLAVFVTEDFLSWEEASLNWPTKEACTSPTSLDANVWAPDVIQGKDGRFYMYISVGSEIWAGGSDHPLGPWENLKADNTPLIPSDFIEGIHHIDANCFIDDDGKIYLYWGSGWDWVNGRCLVVRLDDDMKTFLEEPQDVTPPNFFEGAFMIKRNGQYYLMYSDGMAINETYHIRYSVGDTPYGPWREGKYSPILQSTPDGAVVGPGHHSVFRVHNQDYILYHRIYPQEQEYVLRQLCLDSLNYDAKGNILPISLNSVPPFE

SEQ ID NO: 46 - protein, 959 aa, Alkalitalea saponilacus
MNRILRKMGVLLAVLILSLSAIAESSPRERLLMNYDWKFAFGHATNIEKDFNVGTSYFTYLAKAGYGDGAAAADFDDRSWRLLDLPHDWAVEAEFHPDASHSHGYKAVGPGFPESSVGWYRRSFYIPEEDLGKRIFIEFEGVFRDARVWVNGFYCGNEPSGYTSFSYDVTEYLNYGGNNVVSIRVDACMEEGWFYEGAGVYRHVHLTKTDPLYVPQYGTYVTTQVDDSRSEVTARITVMNKNLEPASFQIENKIIDAEGRVVASGRSGIKELKSMFHGEYPMILNVDNPRLWDIDDPHLYQLVTNIYQNEVLVDEFKTTFGIRTIEWTPDRGFFLNGRHVKIKGTNNHQNHAGVGTAIPDALHEWRIRQLQYMGNNTYRMAHYPPSPALLEACDRMGMLVVNENRIMGTTDEILDHLRRLMIRDRNHPSVILWSIGNEEWMIEGNEKGARIALNMQAFAKKYDVTRPINVAVSGTWGGGISSVIEVMGYNYLRHGDTDKHYAANPWQASLGTEEGSTNTTRGIYFDDFEKQHLAAYDRPTNGFIRIRDGWKHYAERDYLAGMCIWTGFDYRGESTPFEFPSVVSYFGMMDLCGFPKDNVYYLKSWWSNDPVLHVFPHWNWPGREGEEIDVWVYSNFEEIELFLNGESLGRQTMKPNDYLSWMVEYQPGTVKAVAYENGEVAMTTEVSTTGAPSTVALVADRTEIRGDRADLSVITVRVEDENGALIPDAMHDVVFDISGPGRIIGVGNGDPVSHEPCKFVETIKAFKIENIREKPLSDVRMRRVLAPGFDCSSWKPGLQGDGLAPGTESVPMVVRGTFNLSNEELLKGKIQWMYKSIGHNQSVYVNGTLVGENLSGDVPFHQFDLSASELRTGVNVVTMVANPYVKTHVWNSENTDPGLVRVEIPANQWRRRVFNGLAQVLVQSTGEAGDIILSAKSEGLKRDDIVITALESDMSPVVK

SEQ ID NO: 47 - protein, 805 aa, Alkalitalea saponilacus
MKKYNWHVFNKKTVLILAVVLLSVPVKGQMQGMQLLNEPQELTPDFRSFRNTYFVADRLADFNPETATGKIVYERYNYETRQAFSNMLGVLAPAEPNEFPAGEYEVSPALPFSLEFISPRAVRIRAQSGVVAPQVAAQKSLMLINNDMPPCKNWVYSKVDEGHKYTSPYGSVVITEQPWRVTVYDENGRILTSTNNYEDNTSTYTPVLPFSWVRRARDYSRSFNAAFNLQPGEKIFGFGEQYTEFNKRGQSVTLWVNDANGTQNETSYKPIPFFLSSRGYGMFIHTSTPITADIGKYFSGVNSLMIGDEELDLFIFIGDPRDVLNEYTNVTGKPTMPPLWSFGFWMSRITYFSEAEGREAARQLRENRIPADVINFDTGWFEVDWRCDYQFAESRFDDAEKMISDLKADGFHTCLWQLPYFVPKNRLFQEIVEQGLFVRNTKGNIPYEDAVLDFTNPAAIKWYEDKIRGLLEMGVGSIKVDFGEAAPVYGIYHNGRTGWYEHNLYPLRYNKIVAELTQEIKGENIIWARSTWAGSQRYPLHWGGDPAPTNSAMKATLRGGLSMGVSGFTFWSHDVGGFVDPTPADVYKRWLAFGVLSSHTRAHGHPPKEPWEYGEEFLNDYRDAVNMRYKLMPYIYAQSKHGVENGLPMMRALFIEYPDDPGAWLVDDQYLFGSDMLVAPHFENLEARDVYLPGNHKWIDYQTGKVYNPGWNRIETAHIPAVILVRDGAVIPHIGLAQATKYMDWSNIELKVFSADETTAKGKVCLPADDMLKEVVVNKRDGKAELVSNPFGRRTKLNVSVFDVK

SEQ ID NO: 48 - protein, 286 aa, Alkalitalea saponilacus
MKLIAVLCTSLLMSCIAADNGDNSQIRTPDGYALIWSDEFDQDGRVNEKYWEYEEGFVRNEELQWYHRDNVYIKGGILVFEGRREQIENPNFDPNSRNWRRNREFAEYTSGLIKTRDRFSFQYGIMEVRARIDPRKGSWPAIWTLGVDRGWPSGGEVDVMEYYRIDGVPSILANAAWDVNNNYNPKWYSEVIPFLYFLEKDPNWAKEFHIWKMDWTEDYIRIYLDDELLNEIDLNETINYDGFNPFRQPHYILLNLAIGSNGGDPSETDFPILYEVDYVRVFQKIE

SEQ ID NO: 49 - protein, 381 aa, Alkalitalea saponilacus
MHKNPICLTALIITVFCGCNEITEPANPIDKNATPETVALFQNLMKISENHVLFGHQHATEYGQGWYGDDDRSDVKSVTGSHPAVIGIDFMHLSNRSREEIETEKERLRKNVVDTYNRGGITTATWHFHNPVSEGRFYWVDSVSVAAVQHIIPGGYAHEDYKVILADIADWAHSIRGEDGTLIPIIFRPFHEFDGDWFWWGKAHTSREDFVSLWQFTVSFLRDSLNVNNFLYAFSPDNRFETEEEFLERYPGDEWVDMLGMDNYGDLGRDRYDLETASQKLMIVSDYAKKVQKLAAFTETGLESIPDTTWWTNTLLEILKTEGMRMSYVLVWRNDVNSPTHYYAPFPGQVSAPNFIEFYNDPFTIFENDLKEIDVYRFNSL

SEQ ID NO: 50 - protein, 582 aa, Alkalitalea saponilacus
MKSYLFIIGVIFLFSCSKNSTIKVNPGEAYFEYVKYTGNDPYYDQHPLGEGQFYNPILPGFYPDPSICQKGDDYYLVNSTFSFFPGVPIFHSTDLVNWTQLGHVLDRPSQFNNDSLPVSAGIFAPQISYNPHNDTFYMITTYVRGGGNFYVTAKDPAGPWSDPVWLPEVPDIDPSIFFDDDGRAYITNNQDPEGGSTYVGHKATWIQEFDWKNNKTVGPRKMIRDGGHDLAEKPVWIEAPHIFKLHGYYYLTTAEGGTSIHHSQVIFRSKDIWGPYETNPNNPILTQRHLPADREFPVTNVGHADYVQTSEGDWYAVFLGCRPYTVNNEYNIGRETFLLPFNWDNEWPEFLPMDATIPLTLDKPNLENKLPSDKPVMGNGNFSWTEDFIGGELAFDWVFLRTLREKWYTLEEGKPGITIKLRDVNIRELKQPSFLARRQQHHNMSIETKLAFNPQNEQELAGLVLFQNEAYHLTLGVTLIDGKTHVVVQNAKEDPSIVRNMSGDNFDGTVEKVILAQKDISDHYNGEILLRASMKDGEFSFEANSNGTWEKLADGIDATYLSTEKAGGFIGTMMGLYASSNE

SEQ ID NO: 51 - protein, 269 aa, Alkalitalea saponilacus
MKKMKLYSLFIWVLPFVLFMSCTKISSDWKLVWSDEFNYHGLPNPLKWNYDTIGNAYGWGNKELQYYTYANPENVWVEGGFLHIRAQKERINGFDYTSARLNTLNKGDWKYGRVEVRAKLPGGRGIWPAIWMLPTEWKYGNWPNSGEIDIVEHVGYIPDSVFVTVHTEMFNHMINTQKGASVYLPQNEHEFHLYAIEWCSEKIDFFIDDELVFTFYNSGKGAAEWPFDQKFHLLLNVAVGGNWGGQQGVDDSIFPVTLLVDYVRVYRRS

SEQ ID NO: 52 - protein, 383 aa, Alkalitalea saponilacus
MKRTLFYAAAFLFMLSGCSEDIIDVELIADEEINDAYLKSYESGTHDGYFWALWTDDRPGWVNYQNGPGGNYTVSWDYSGNFTAGKGWNSGTVNRIVGYNIGVHNHSGGGVFGYYGWTRNPLIEYYVNERWGNARPTGEHRGTVTSDGATYDIYTAMRVNAPSIDGTQTFRQVWSTRRTQAPTGQNRTITFANHVNAWASVGLGLGSDWTPAAILLTEAYGGNSQGSVNATVWSAGESSGGGGGSGATYYRIQNRATGLFLDGMGRISDGSNLGQYAHTNHQNAHWVREASGGFERFRNRGTGLYIDGMGRTSNGADAGQWANTNHNNAQWSLESAGDGYFRLRNRGTGLYLDGMGRTSNGADVGQWANTNHQNAHWRFVPVQ

SEQ ID NO: 53 - protein, 425 aa, Alkalitalea saponilacus
MKKHFKLLIAFIAVTMIISCSPAEKYMGKTAADILGNPEYQAISYGGYREISREIQPTIPQLKEDMKILSAMGIKLLRTYNVHYDEAANLLEAIRQMKDDDPEFEMYVMLGAWIDCKNAWTDLPDRIRSEESDRNAVEIARAVELTQLYPDIVLIIAVGNEAMVHWAWDYYVEPAIILNWVNYLQDLKQKGELPETLWITSSDDFSSWGGGGSEYHVEDLTKLMKAVDFISMHIYPMHYTHYQPHFWGVRDDELHLSDLEKIDAAMLRAKNEAIDKYNSVVSYMQSLGIDKPVHIGETGWATVSNEFYGADGARAIDEYKSALYYWHIREWTNREGITCFYFEAFDEKWKDSNNPLGSENHFGLINLQAQAKYAIWDLVDEGVFNGLTRDGMPITKTYNGDKEAMMKDVLVPPTDQEIRERISND

SEQ ID NO: 54 - protein, 341 aa, Alkalitalea saponilacus
MKTYFYLLQFSILFFCLSTTIKTEASGSLPRISVEGNRFVTPDGETIIFQGVNFADPDRLVKEGQWKRDLFRVARDWGSNIVRLPVHPQAWRERGKEDYLILLDQAVEWAREFDLYIIIDWHSIGNLRTELFQHEMYKTSLPETYDFWLTISRRYADEPIVAMYEIFNEPTTYQGQLGSLTWDQWADILTDIIYVIRANSPEAIPLVGGFNWAYDLTPLMYAPLNVPGIAYVSHPYPQKRDQPWIPQWERDFGFAADDYPIIATEIGFMQPTDRGAHIPCIGDEEYGRTLMRYFRDKGISWVAWCFDPDWSPQLIKDWNYTPSRSGKFFRDVMLGKENLDE

SEQ ID NO: 55 - protein, 357 aa, Alkalitalea saponilacus
MKLLTVILASILMLSCSNQTENSSEKGLKDYADFPIGTATSPRQLFNNEQLRGMIKADFNSITLDNDMKMHRIMPAENEFNWEEVDRVVEFCQENNFRLHGHAFIWHSSTPRWLQEKNPDSTWLAQFMEDYILTYGSRYRGKVAGWDVVNEAIMDHTGEFRSSIWYDAFGEEFIARAFRLAHKADPDAILFYNDYNIERDTVKFNATLRLVERLLEQGVPISGIGFQMHIRMDIDEETIEYTLRRAAETGLQIHLSEIDVIFNKHDDNPGGGIQIYDEVTEEMLEAQGKKHQWFAEAYIRNVPAEQRYGMTFWGFVDSHSWIRPFFRLNDWPCLYDADYNPKPAYFGFIEGLKSSQN

SEQ ID NO: 56 - protein, 376 aa, Alkalitalea saponilacus
MKSLQKLATIALAIILMGSCTAQEEATTLKDALKDYFYIGTALNVPQVAGQDPQAIEIVKTHFNSVVAENCMKMMYLQPEEGVFFWDEADAFIEFAEANDMQVIGHTLVWHSQAPRWMFVDENGDQVSRERLIERMKTHVQTVVERYKGRVHGWDVVNETILDDGSWRQSPWVRIIGPEFVQMAFEFAHEIDPDVELYYNDYSVSRPEKRDGIYNMVKDLIDNGVKIDAVGLQGHLSMDFPTVEMKEEALQKLASLGVKVMVTEMDITVLPWPSRRHSAEVSLNYEISDEYNPYPNGLSEESYTALMDKYVDFFEMFMRNKDIISRVTVWGVDDNQSWRNNWPIRGRTDYPLLFDRDYQPKSAVTRIIELANAKKQ

SEQ ID NO: 57 - protein, 387 aa, Alkalitalea saponilacus
MHSSLLLEIEEAKRAAIEVLVHNMHGPFHGLPRTAGWGYPEPYTRDLMLSILGIAVSGNQQLMDSIRKVLETLALNQTKLGHIPSLVHDSEDRGASDTTPLFILAVGIYRRVTLDKHFLKSALEKALLWMEYQSPSDRSLVAQQPTSDWRDEQWVTGYGLFVNTLTYSYLKLLGLYERADKLRHAMGRFTITSGVMHKHVHEGLVVMYKPYYAFWSYKIFSSERFDLLGNSLAILSGLASSSRANEIITWIENECINMRKNGELKSDLPPNFFPYIKPTNPDWHERYKKYNNPGEYHNGGIWPFICGLYVAALVAAKRYRLAEKKLIEFTMIVKLARKTSLKYGFNEWIKAQDGMPMGQDWQTWSAAMYIYAAKCVETRETPFFSSS

SEQ ID NO: 58 - protein, 709 aa, Alkalitalea saponilacus
MSDDIQIWPGKPYPLGATYDGEGVNFALFADHAHGVELSLFDAADKEIRIKVVERTHNHWHVYLPGIKPGQRYGFRVHGNYEPKAGHRFNPNKLLLDPYAKAIDGVINWNDAMFGYEINNKKKDCSFSISDSALYIPKCIVIDDEFNWENDRSPEIPLHETIIYEMHVKGFTKLSEKIPENLRGTYAGVGHPESIKYFKELGINAVELLPVHQFVADRHLVEQGLTNYWGYNTIGFFAPDARYSASGMKGEQVWEFKQMVKDLHAAGIEVILDVVYNHTGEGSHTGPTLSFRGIDNVSYYRLIEEKPRYYMDYTGTGNTLNTVHPNILRVIMDSLRYWVLEMHVDGFRFDLAPVLAREFDDVDKWGSFFDVLHQDPVLSQVKLIAEPWDLGEDGYHVGNFPAGWMEWNAQYRDCMRDFWKGEDEMLPEFANRLTGSSDLYFDNWRTPTASINFITAHDGFTLLDLVSYNEKHNMANGENNNDGESHNRSWNCGVEGPTDDVNINNLRKLQVRNFLATLFLSQGVPMLVAGDELGRTQQGNNNAYCQDNELSWINWDKMDRDLLLFTSKLIHYRKKHPVFCRRQWFKYQPIKGQDVTDIEWFTPNGIEMSDEHWNSSYAKSLAVFLSGYGVRAKSKTGEKIVDDSFYLMFNSYHEPLTFTLPADKWGGGWLKIMDTYTAFFDEKGDGSSYRAASEIVVQGRSVVLFCHPR

SEQ ID NO: 59 - protein, 493 aa, Alkalitalea saponilacus
MTEYNGVMMQFFHWYTPADGKLWSNLSQQAGELARAGITAVWLPPAYKGIAGKSDVGYGVYDLFDLGEFDQKGSVRTKYGTKDEYVKAIMDAQKAGIHVYADIVFNHKLGADHQEEFKATPYKPDNRHEPLGELQPIKAWTHFSFPGRKGKYSELKWHWWHFNAADYNAFDKHQDAIWLFEGKTFDDSVDLEKGNFDYLMGCNLDINNPDVKKELFYWGDWYLKTTGVDGFRFDAVKHVNSSFFLEWLKHIKKNAGKKLFALGEYWSGESEALHNFLDETDGAMMLFDVTLHYNFAAAGKQGRDYDLTKIFENTLVASHPMLAVTLVSNHDSQPLQSLESVVEAWFKPLAYALILLRKDGYPCIFSADYYGAHYKDKGRDGNEHEIWMDSHRWLIDKFLEVRKEHAYGEQYDYFDHPNCVGWTRTGNGDSGRGMAVIMSNGDDGEKKMQTEHPNTTYTDITEHIKNPVTTDGEGWGNFFCKAGSVSVWIPAKT

SEQ ID NO: 60 - protein, 671 aa, Alkalitalea saponilacus
MAKRLTEIDPWLAPYEGHMIRRRSLLNDTVDVIENRYGTLKNFADRHLFYGLHKTNDQWVFREWAPSASAIYLVGAFSGWQPQQEFKLQKSSGGNWEIALPESIFKHGDYYKLWIEWDGTGGMRLPAYATRVVQDPETLLFSAQVWQPEPFIWTDQNFRVADEPVLIYEAHTGMAQEEPMVGSYIEFADKILPRIKAAGYNTLQLMAVQEHPYYGSFGYHVSNFFAPSGRFGTPEDLKFLINSAHNLGISVIMDIVHSHSVRNEEEGLSRFDGSYDQYFHSGDRGNHPAWDSRCFDYGKEEVQRFLLSNCRYWIEEFHFDGFRFDGVTSMLYTHHGLEKAFTSYDDYFDGSLDDDAVLYLTLANKLIHEIHPKAISVAEEMSGLPGITAAPNDDGLGFDYRLSMGVPDFWIKLIKEKADEEWQVGTLFHELTQHRPEEKVISYAESHDQALVGDKTIIFRLADKEMYDHMAIDHKSLVIDRAIALHKMIRLLTLSTAYGGYLNFMGNEFGHPEWIDFPREGNNWSYHYARRQWSLFDNEKLKFRWLGMFDKAMIGLARKHSLNGIPEIYLKMDNETDQVLAFERGSLLFVFNFNPSVSYTDYGIPVYPGKFRNILSADNPVYGGFDRVNENTVHFSQPVPLNKSHHQVKLYIPARTAFVLERQKVRSVYDV

SEQ ID NO: 61 - protein, 489 aa, Alkalitalea saponilacus
MQVSVNRKNITFVPDAGRVIARFLFTGEERAVNTIRFVLNMSEEEASFSLKQTLRDFSMRHRNISRIFEKHFNNVAHLLSRLDINIDEVDYQKKILIGSYFTMEYSIEAAAFFNPSMVEHPDQTEIGPGSKRVIISFRATGEGHISSIVFRTGVLDKNNDLTIEPIGNLLEEAEHIWRHTYNKKLFADKLEEMQELHSIIPYELVLDKLNENFTYGELRKCIEESRKAIHLASDKEYLFNQIKWLASSHYELQFSLDTNISERVIFPVSVNEKNGIEDARFVKFTDENNNTKFYATYTAYDGITIMPKLLETNDFYHFKISPLHGEIASNKGMALFPRKINGKYAMLCRIDGFNNYIAFSDNITVWREAKILQQPKHSWELIQIGNCGSPIETEEGWLIIMHGVGPMREYVLGAALFDLENPEIEIGRSKTPLLIPNVEEREGYVPNVVYSCGSMVHNNDLIIPYAMSDYSSTYASVPLKELLDELKSI

SEQ ID NO: 62 - protein, 485 aa, Alkalitalea saponilacus
MAIIFGIQFGSKFGSTKKFESKLIKEKVDFERFNELDQSETLRRYNELDQLVHSGDFEKKVQFLKTAKFKNSEEYRQLEQFKSMKASKDIKSYLEYSKSGKLDRMKSILESDLLKEFNDLKVFVNSSAFHSAKVKKDFKQSEAYAKQEQYSALKKDPDIIFYLKQDKSNEYRTVAKLENSERLKSFFKLESIIQSPEFIEKKVFLEDKNRFKKSEEARLIEEFKELQKNEDVKWYQKTKKLNPFKEIRKWELTFEDDFDALQLDKSRWMTGYYWGKALMNDNYVLAGEKQFFKEDNIEMHDSVVRINTQKETYRGKVWDATLGFTMQDFEYTSGLISTGQSFRQKYGKFEAKVKFSQAYPVVNAFWLVGEKMLPQLDVFKSSVTKGKALESGIHVGAPEGQPLNLLKKITGANFKNGYYIYTLDWSPEALIWKINGIEVHREVKHVPNEPMYLSFCTILPEYPSDKQMPSFMDIDWIRCYRKKEE

SEQ ID NO: 63 - protein, 809 aa, Alkalitalea saponilacus
MKFTILSFLLLVSTVGFSQRHLERINFDWKFTIGDFTDGYKVDYDDSRWETVHLPHDASIAGPFVRDSLNSDRQNGFLPRQKGWYRKNLELNKDLDGKRVFIEFEGIYRDARVFVNGDKVAHQLNGYMDFIIDVTDHVSQGSNLIAVSYDNTDMESSRWYNGEGIYRDVWLLITEDVHVDYYGTYITTPFIVEDYARVNLQTEVKNHRNDSLTITLKSDIVCPAGEVLQTIINTVPFGPDELFIFRQYGQVNNPKLWDLDTPYLYKLKSSVIVDGEVTDTYETNFGIRTVEFCRYQGLLLNGRKVLAKGVNIHHDLGPLGAAAFERGFERRLEGLKKLGVNAIRLAHNPHAKFILDWCDRNGMLVVDEPFDKWSDQFFGQGNDFEKHWRPTLKAFLKRDRNHPSIIIWSAGNEVSQQRSPRYDFGVPMMKEMYDFIRKHEPSRMITTGLHPSRARGVHRTANYYRAGPPEMVFYMDVVSTNYREEFWPVDKAKYPQLIFMLSEAQVGNLGNEWFNFDHRSSVGLFYWGGTDYIGESFGWPAKGWVNGIIDWNDHWKPFSYYIHSLFADEPMVHITSFDRGSVVEKYWNEVELRYQPMFSHWNWEGLDSISVYTFSNTHEVELILNGRSLGVKQVPEEYYTKDIRGYTAEEFDPDNPINLGPPMHENLEWRIPYEPGTITAISRIDGREVARHELQTAGEPYRIVLEPDRDVINADGLDLSYITVKVVDRNGILVPHADHNITFRVTGAGSNIAVSSADMVSDESFVSDQRKVFQGKGLLVVRADQKPGTIRVRASGRGVRNANLVIEVR

SEQ ID NO: 64 - protein, 784 aa, Alkalitalea saponilacus
MTTIIYKKWKNLFTLLLISIFIFSGCMVDDHDYPSSRITISFNNDWMFMEGDHDGAQARRFNDRSWRALNVPHDWSIEGEFDQNNPTGRGGGYLPNGIGWYRKSFDIPSAFEGRRVFIHFDGLMANSDVYINGEHLGHRPYGYVSMEYELTDYLRYGRSNTIAVRLDNSKQPASRWYTGAGIYRNVRLIVKNDVHIDNWGTFFSTPKVSEESATVRVFTTLKNSSEISHQVHLNTLIHNPTGDLVSEKGTVIDLAPGEKIDIEQILEVLNPQLWSLDSPQLYKGISQVTIDNELQDDLVTNFGIRSFHFEPATGFYLNGENIRIKGVCLHHDAGAVGAAVPLAIWEERFNQLQSIGINAIRLSHNPFAPEFLELCDRMGFIVMNESFDTWRARKNHGDYGYQHHFDEWWEEDTRSIVLRDRNHPSIFMFSIGNEIRDNLDNEQGFETFRMQYDLVHKLDGTRPVTMGLFRPNQANVYQNGFAEMMDIVGQNYREEELLQASIDNPHWKVIGTENGHTRQAYLIWRDNPAIAGHFLWTGFDYLGEADWPEVSHDFGLFDRAGFTKPRTYERESWWSDKPMIRIFRREQHLGEGGLVDDWTPTDFDTYDEAHIEIYTNCDEVELIFNGESQGVRKRPADHSPIRYRLTYQPGSIKAIGRIDGKDVAIHEMQTAMPPSNIALSASKTTLKNDWDDVAIVRVMLTDENGVHSPNFDRPLTFNVSGNGELIAVDNGQRDSHEPFKTNVRRTSRGQAIAIVRANADVGQILVSVSGEGLEESSIEININQ

SEQ ID NO: 65 - protein, 1043 aa, Alkalitalea saponilacus
MKRCLITFLMVALGLPFLSGAERPQRDWEDPTIFTRNTEPPRATFYNFPDERRALEHNHQESPYYYLLSGQWKFYWAPNPKQRAKDFYKEDYIVDHWDEIPVPSNWELHGYGIPIYSNIRYPHKTDPPFIGDEDNPVGSYRRDFTLPAGWENRKVFIHFKAGTSGMYVWVNGQKVGYHQGTKNPVEFDITPFVRKGKNMIAVEAYRWTDGSYIEDQDMWRLSGIERDVYLYSTDDTRIADFFLRPDLDNNYRHGNLNGEITIRNYSPSSVSRVVSVALIDEDGNRVFSENLSVTVPANSDRDVNINRRIRNPRLWSAEFSNLYTVLITLKDNGGNTIESTSWRIGFRSIELKDGLLLVNGKPVKMKGANLHEHCPINGHYVTRDVIKKDIEVMQRHNINAIRASHYPHSPDLYRLADEYGMYVVNEANIETHGMGAEHQGWYNRDIHPAYLPEWHAAHMDRIYRMVERDKNHTSIFAWSMGNECGNGQVFFDAYDWIKDRDVTRLIMFEQAGEQSNTDIVAPMYANFRSITEYSQRENVDRPYILCEYAHAMGNSTGNFYKFWDIFYAVPHMQGGFIWDWVDQGILADDGFGNKFYAYGGHMGSGHLHHDENFCMNGLVFPDRTPQPALMEVKKIHQNINFTEENLQNGTIRVENRFYFTNLSDYNFTWELLKNGEKVDEGTFSLNLAPQQSRVVRPGFSYSTPQNGDEYLLNVYAFTKEERQLVPAGHEIAREQFKMTGSDYFNREFVSKDGSFEVTEDDNSVVIEGENFNIRLDKRRGVLGHYRVGYRNLIQGSPEPFFWRAPVDNDFGNNMHRNSTIWRQAGRNKDVRNVTVEKSENEVRMEVHFFLRDVQSDYHVKYTVTPDGAVRVDVNYQAGVEGLPEIPRFGMEMFLSRQYDNFTWYGRGPWENYSDRKLSSHVGIYNSKVADQYVPYTRPQENGYKTDVRWLTLTNDEGFGLRIEGIQPLSVSALHFHTEDFDPGFTKKGQRTVDVFEREDIVLNVDFLQRGVGGDTSWGSHPHREYRLHDDSYSYSYIIRAEIP

SEQ ID NO: 66 - protein, 819 aa, Alkalitalea saponilacus
MIKRIVLSCFTFLLVSTMLSGESVRQQITLERNWKFTRGDFPEAINPGFSDANWETVSIPHDWAIYGPFNEEHDLQIVAVEQNYEIIPTRKTGRTGGLPYMGVGWYRTSFDVDGFIKGEQRVNILFDGAMSEAQVFINGAKVGFWPYGYNSFHFDITEYLNDDGKNNVMAVRLENQEFSSRWYPGAGLYRNVHLIVTNEVHVPVWGTFITTPHVTKEFASVKLVTELNNAENGQNVRVNTKIYDRWGRMVASQETNQMFFEDRPYEQHFLINEPELWTPESPRLYEAVSRIYYREELVDIYTTRFGVRDIKFVPEKGFFLNGQRRKFQGVNNHHDLGPLGAAVNIAALRRQLVLLKDMGVDAIRTAHNMPTPELVELCDEMGFMVIVESFDEWDRAKVKNGYHRFFDEWAEKDLVNMIRNFRNNPSVIMWSIGNEVPTQCSPDGYRVAKFLQDICHREDPTRPVNCGMDRVSCVLDNGFAALIDIPGLNYRTHRYLETYERLPQRFVLGSETGSTVSSRGVYKFPPEIKINAIYDDHQSSSYDLEYCSWSNLPDEDFALADDYEWTMGQFVWTGFDYLGEPTPYDTDAWPSRSSLFGIIDLAFIPKDRFYLYRSVWNREDATLHILPHWNWEGREGEITPVFVYTNYPSAELFLNGKSQGFRTKNDSTLQHRYRLMWMDVKYEPGELKVVAYDEAGRAVAEEKMVTAGRAHRIELIPDRTIIDADGKDLSYINVRVVDRYGNLVPTDSRLIRFDTSGAGKYRASANGDPSSLELFHKPQMSLFNGQLTAIVQSGNQPGTIVFEAKAPGVRNARIEIQVK

SEQ ID NO: 67 - protein, 937 aa, Alkalitalea saponilacus
MHNFMHHAPPLPRNKIKCNLTKFNSMYSITSFRRQRQLSVFGFFFAILFFYSCTERPDHQVRERLSINDGWRFFKYDDAKNADGLIYDVRSDIDEDIDQREADDQPVEGEWVEGEESVLKAWILPSGNDFIKDSAKRHVRPEGYPGFDFPFVQASFDDGNWEKVNLPHDWGAREPFTYEVSGSMGRLPSHGVAWYRRSLDVPSSDAGRQIYLEVEGAMSYAMVWLNGHLVGGWPYGYNSWQLDLTPYIIPGGKNQLAIRLDNPPISSRWYPGGGIYRNMWLIKTEPVHVGQWGTFITTRDVSEESAVVDLEVTIDNKSNENADVEIVTFIYELDLNGNRTGKRVIEFAPQSANVAAGTKTAVNSSVTIANPRLWGSLPTQIPNRYLAVTEVQKDGKVVDVFETPFGIRSLEFDAVNGLFLNGEHIYIKGVNQHHDLGPLGAAFNKRAAERQLEILREAGVNSIRMAHNPPAPELLELTDKMGFLVVNEVFDVWERRKVPFDFHLIFPDWYEQDLRSMVRRDRNHPSVIMWSYGNEVGEQYTGVDGAALSQKLNDILKDEDPTRPTTASMNFAKPDMPMPATMDIISLNYQGEGIRIHPGYEHLQGIRTHPLYSEFHETFPNKMIISSENAAALSIRGEYLFPVTPNSSAPVSDGIGGDSESLIVCAYELYTANFGSSVDRVFAAKAQHPFVAGGFVWSGWDYLGEPTPYYDARSTYFGIVDLAGFKKNRFYLYQSHWRPELPMAHILPHWNWPDRVGKVTPVHVFTSGDEAELFLNGVSLGRKKKGEYEYRLRWDDVVYEPGELKVVAYKNGEEWAQSFVKTTGAAESLNAEADRDRIKADGKDLSFVTISVTDEDGFVIPDAKHPLRFSIEGPGEIVATDSGDPRDFEAFPSNERNAFNGLSLVIVRGISGKPGIIRVMAESDGLKNAVAEIQTVR

SEQ ID NO: 68 - protein, 785 aa, Alkalitalea saponilacus
MRTFLGLILTISVLWSCKNGETSHYSNRENLFNDGWEFVKDVEEEDLWQNRVEWESVNLPHTAHVEPLVIKGRQWMGTSYYRKRFTVPSELFGKHLALHFEGAMHLSDIYINGNRVKTSYSGYLPFYVELTEHLKYGEENTVLLRVNNEDNPQVPPGKPVDELDFNYFSGIYRNVWFLVKDRLHISDPIGAKRVAGGGVLVTYSDVSIDKATVNVQVDVNNEYTEEKSAQIRLKLRNENNRIIKDVTSDVEIISAEGNGLFELSFDVENPDLWSPSSPSLYHLHVSLIKDNQLIDKVSERIGIRTFTFSTDGFELNGEPLFLRGTNRHQEYPYVGYAISDNANYRDAYKIRKAGFNFVRLSHYPHTKSFIDACDEIGLLVMNAIPGWQFFGDDVFYANSINDVRKMVRRDRNHPSIVLWEASLNESEMPKQYILDAHNAVYEELPSSDLYTCSWYEDIFDVFIPARQHGYPPHYWNHYDKKPILIAEYGDWEYYAHNAGFNQTAFEDLTSEERNSRQLRGFGQRRLAQQALNYQEAHNSNLIGSPAGDANWLMFDYNRGYAPDLEASGIMDIFRLPKFAFYFYKSQAAIGEFPQKEFNEPFVYIANYYNDPSFLEAKIYSNCEEIELFVNGQSLGRQLPDEDANSTHLNQPPFTFILSSFSPGELKAVGYINEKAVVESIRRTPGNPKEVKLWIDESNRPLTKNVNDLVFLYAAIVDDYGVIIPEAVNSVEFNVSGDASLIGMNPIEAEAGIATILLQAGQKGGVLNLTATSNGLLKGELSLEVR

SEQ ID NO: 69 - protein, 882 aa, Alkalitalea saponilacus
MKKKSIFLQIATASFFMLFSCTTDYNETVFERNLDKGWQLFSSEGLNATGSEISGADFDRSFGYPVTLPATVMHGLQQNGKFPDLFEFGVLEQMDTVPYQVPWWYRTTFNVNTEPGKDFFQITLNGINFKANVWLNGQKVAGDDLIQGSYGVWNFDVSELVVQGENHLAIEIIPPVFGVDVSKGFVDWNPKPADNLMGIWRDVTLKQSGPVSMRHSNVVTKVNKETLDEAEVTISTYLTNHSGVEQRAEITANFDILHLKKEVRLNPGETREIFFRPGQFPELHMKNPRLWWPNNMGEQALYDLELEVLVDNRLTDRDEFRFGIREIEDFWNENRYRGFKVNGQKLVVKSAGWVDDILLADSDQKVIDQLKYAQHVNLNSIRLESFWGRNRTIMETADELGLLLMLGWTAHWEWESYIGIPHDDYVSIRGEEAKTLHANNYRDQVLWHRRHPSVAIWTYGSDKLPRPSLEVMLNERMAKADTTRPILSYCGGAMLMGDSDPRQSIISGPTGVKMEGPYDWVAPVYWYIDERYGGAFGFNTEVGPGPQIPPLSSIRKMIPEEHLWPVDDVWLYYSGRNQFENLDRYLGAFHARYGEFNYLEDFLFVNQMASYEAIRPMFEAFSVNKYNSTGVVQWMFNSAWPTFYWQLFDYYLMPTGAFYGTRKAAAPLTLIYNYGNGNIYLNNDFLESQQNLNVAVKAFDLNSNLLFETGLTTNIDANSAKMVVEMPGLNIPSTTWFLDLRLKDDAGNEIANNFYWLSTVDDVPDFDRTTWYWTPNKQHADLTQIQNMPQANVIFSYDVKKYDDEFIFTVNLENQADVIAFFAEYQIVDKNTMEPVLPVFWDDNYISLLPGEKRVIKGSVGAKGINGDSLTVTLQGSNIIVQ

SEQ ID NO: 70 - protein, 525 aa, Alkalitalea saponilacus
MNKNSANILNLAFPLFAILLIGISCNKVPKIDISNADLIPVPKEIIPAFGAFEVTQSFRIMVDSEHDEVMRSAEIFAELLRKSSGFDVPVFQKSGQSIEESLVLLVDDFPELGEEGYELFVDDDHVRLNANKPVGLFWGLQTLRQLFPVQIEMNDVQSERWLIGTGVIRDYPRYEHRGAMLDVSRHFFDVDDVKRFIDFMAAYKMNRFHMHLSDDQGWRLEIKSWPKLTEIGGSTQVGGGEGGYYTQEEFLEIVKYADERYITVIPEIDMPGHTNAALASYPELNEDGVARELYTGMEVGFSTLATRKEITYQFVDDVVREIAALINGSFFHIGGDESHVTPKDDYVYFINRAQDIINSYGLTMIGWDEIATADLSPTSIVQLWASPENARLAIEQNARIIMSPAKHAYLDMKYDSTTVLGLNWAGYTEVDEAYNWDPTTFIDGVPEEFIIGVESPLWTETVETMEDIEYMVFPRLPGIAEIAWADMDQRNWDEYKFRLAKHGERLKAKGINFYRSPKVPWNDNE

SEQ ID NO: 71 - protein, 370 aa, Alkalitalea saponilacus
MKTAIISFLLSLFILAGCANPSSQTGEENKSVAQKLFDDLMSITGKATLFGHQDDLAYGIGWKYVDGESDVKRTAGDYPALFGWELGGIELGHEMNLDSVPFNKMRQFAIWAHQNGGVNTFSWHPFSALDESKSSWVTDEKVVKHILPGGSHHEVFLKHMDKLVAFFKELNEENGEKLPFIFRPWHEMDGGWFWWGADLTTPDEMKELFRFTIDYMWEQGLDNFLVAYSPDRFFNSIDEYLTWYPGDEYVHVIGVDNYYDMRRGPDGLQDAILKLEIAAKYAKETGKIAAFTETGLDTIPDENWYTQSLAKVLNANEWTRRMAYVMVWRNHDLDHFYVPHPQHPAADDFRQFTSQQHIWLLNDWANYQQK

SEQ ID NO: 72 - protein, 561 aa, Alkalitalea saponilacus
MNVIKKIGIYALPLVFALGACNSGTIKSPDYSWVYDNIEFDMPIVQEPVIPNNSVNIADLGAIADGITLNTHIFEKAINMMASKGGGKVIVPAGIWITGPIVMKSNINIHLKEGALVRFSDNFDLYPVVESAFEGIMTYRCQSPISGRDLENIAFTGSGVFDGNGQAWRPVKRFKMTNNQWRNLINSGGVLEDNESYWFPTEQAARGYVISNRGNLPQLETYEEFVEIKDFLRPVMVSLINCKKVLLDGLTFQNSPAWNIHPLMCEDVTIRNLTVRNPWYSQNGDGLDLESCKNVVIYNNNFDVGDDAICFKSGRDKEGRDRGMPTENVIVKNNIVYHGHGGFVVGSEMSGGVRNVHVSDCTFMGTNIGIRFKSTRGRGGVVENIYISNINMIDIPTEPIRFNMFYGGRAPVLDDDVSNHAEAMPINEETPLFRNIYVKNIVASGFGNAALFMGLPELKLKNIVLENAILKAPKGFSIVDADGIELKNVTIIQEEGPALIIFNSNNIEISDFNYNKKTGDAGLVVSGASSGSIKISKDDFNRPDQQIRRVNNASDNAITIR

SEQ ID NO: 73 - protein, 455 aa, Alkalitalea saponilacus
MVRKILFLVMTLIPVMLFSGEYNKDKTVDLFPDGTPIPEWFRIIEPTDINKLGKHYRVTDYGVKNDSTILQTEQIQAVIDKAYEAGGGVVIIPPGTFLSSSIFFKQGTHLHLEEGAMLKGSDDISDFPIMMTRIEGEWRKYFPALVNADGLDGFTISGKGTIDGNGMRYWKAFWLRRAFNPDCTNLDEMRPRLLFVSNSRNVQISGITLQNSPFWTTHFYKCEYVKLLDLYIYSPYEPVKAPSTDAIDLDVVRNVLIKNCYMSVNDDAVALKGGKGPNADQMEENGGNYNIIIEDCTFGFCHGALTFGSESIHNRNIIMRRIQVNHAQRLLWLKMRPDTPQNYEYVLVEDIEGSHVGNFLYVRPWTQFYNLQGEQEMRMSYASNITMRNINMDCDVLFMVEIEDPWGTVERFDFELSDFTFENLDIEARKDARINKDLVDNLRLINVVVNGEKVE

SEQ ID NO: 74 - protein, 471 aa, Alkalitalea saponilacus
MKRFFSILLVALITFGANSQEWLSKVGAQSFPDGERVYRVNDYNDVFEGYPPIASTSGIQAAIDDCAANGGGKVVFDPGVYHTGALFLKDNVNLVIGEGVELRALIGLEYYPEIKTRVAGIEMMWPSGVINILDKSNVAVTGGGLIHAQGKYHWERYWNLRHEYTPQGLRWASDYDCKRVRTIQVSNSTDVTLKGFRVKQAGFWTVHILYSRHVTVNGLTIRNNIEGMGPSTDGVNVDSSSFVHIFNCDVDCNDDNFTVKAGRDADGLRVNIPSEYVYIHDNIARRGGGALVIGSETSGWIRHVKVENMKAIGTNHVMHLKSAFTRGGGIEYIEMDNVQAENVRTFLTVTLNWNPEYSYATLPDGMDEMPEHWKVMLQEVPREQGIATIRNVKLSNIHTINAQTAFHVTGAEESPITGFGFSNIFVQAQRAGVLSHVRDWTMESVTIKTPGAQELDLRNTRRVRMNRVEYK

SEQ ID NO: 75 - protein, 769 aa, Alkalitalea saponilacus
MKKSLLIGMSVMLFIFGCTSEKKDDAAAMVERIPEVEALLAQMTLEEKVGQMAQITLDVITKGENEMVSDEPLVLDMDLVRRAIVDYGVGSILNTANNRARTVEKWHTVISQIQDVAINETRLGIPVIYGIDAIHGTTYTAGATFFPQQIGQGATFNRELVRKAAEITAYETRASSIPWNFSPVLDMGRDPRFARLWETFGEDVYHTKVLGLEMIKGYEGDDISSPYRVASCPKHFLGYGTPLSGKDRTPALIPEIELRERHLPPFEAAVNAGVQTIMVNSGLINGVPVHASYELLTELLKEELGFTGLLLTDWADIENLHNRDRVAASQKEAVKLAINAGIDMSMIPYNLDFCDYLVELVREGEVPMSRIDDAVRRILNTKFKLGLFDTPVTHYEDYPLFGSEEFESVALKTAQESITLLKNENNILPLSKNSRILVTGPNSNSMRALNGGWSYSWQGEKVDEFAQDYSTILDAIRDKIGAGNVLFREGVRYDNDAAYWVDEAFDIPGAVRAAANVDYIVIVLGENSYTEKPGDLHDLTLSQNQIDLAKALARTGKPMILVLNQGRPRVIREIEPLMSAVVNAYLPGNFGGLAVADVIFGDYNPNGKLPFTYPMYVNTLVTYDHKPSENQARMEGVYDYESDFAIQYPFGFGLSYTTFEYSNLIVSNNELRPNGSLEISVNVKNTGDRQGKEVVKLFTALHYASITPDVQRLRRFDKISLEPGEEKTVTFTLTPQDISFINARNERVNEAGDFDVMISDLVETVSFIK

SEQ ID NO: 76 - protein, 769 aa, Alkalitalea saponilacus
MKKQLLSGLIVLVILFGCSTPKKQDAASMVERIPEVEALLKQMTLEEKVGQMAQLTLDALTVGANHFHTEEPMRLDMDLVRRALVDYNLGSVLNTASTRARSLEEWHTIVSQIQDVAMNETRLGIPVIYGIDAIHGVTYTAGATFFPQQIGQAATFNPELVRRAAEITAYETRASSLPWNFSPVLDIGRDPRFPRMWETFGEDVYLTNVLGVAMVEGYEGDDIGSPYRVASCPKHFLGYSTPLSGKDRTPALIPEIELRERHIPPFKAAIDAGAHTIMLNSGLINGVPVHASYELITELLKEELGFTGLVVTDWADIDNLHNRDRVASSPKEAVKLAINAGVDMSMIPYTLDFCDYLIELVEEGEVPMSRIDDAVRRILNTKFKLGLFETPVTHYEDYPLFGSDEFIAEAIKTAQESMTLLKNEENILPLSKNSRILVAGPNANSMRALNGGWSYTWQGSNADEFYEGYSTILDAIRDKIGSANVVFREGVRYDNNAAYWVDEAFDIQGAVSAARNVDYIILALGENSYCEKPGDLHDLTLSRNQIDLAKALAETGKPIILVLNQGRPRIIREIEPLVSGIINTYLPGNYGGIAVADVIFGDYNPNGKLPFTYPMYVNTLVTYDHKPSEHQERMAGMYDYESDFAIQFPFGFGLSYTTFEYSNLSVSSDVLRPNGSINISVDVKNSGERQGKEVVQLYTSTHFASITPDVRRLRRFEKIALEPGETKTVSFSIAPEDISFINAQNKRVTEPGAFDVLIDDLKATVHYTE

SEQ ID NO: 77 - protein, 316 aa, Alkalitalea saponilacus
MKLFIIFLTLISFSLNGCSKQETEDHVYLFSYFKGDSRDGLHLAWSEDGLVWKELNNGNSFLKPTAGRDQLMRDPCIIKGADGLYHMVWTVSWAERGIGYANSPDLLNWSEQKYIPVMEHEENARNCWAPEITYCEKEGIYMIYWATTIEGAFPETWVPEDNGLNHRMYYVTTLDFKEFSDTKILYEPGFNVIDSHIVPFEGEFIMFLKDETRTPPAKSLHVARSENLTGPYSQPGDVIHGNYWAEGPTSLYIDGNWIVYFDIYRDRRMGAVTSPDLVNWTEITDQVSFPPGTRHGTAFKVKRSVLDNIIASTSVD

SEQ ID NO: 78 - protein, 540 aa, Alkalitalea saponilacus
MRKISLLSALLILITGLTAQTPFVSDVWVSDQGDGTYKNPILYADYSDPDVIRVGDDFYMTASSFNAIPGLPILHSKDLVNWELIGHALDRQMPYDHYSKPQHGNGVWAPSMRYHNNKFYIYYGDPDFGIYMLKADDPAGPWSKPHLVQGGKGLIDPSPLWDDDGRAYLVYAYAGSRAGIKSILVVSEMSPCGTHLLNEGKIVFDGHDAHETIEGPKFYKWNGYYYIFAPAGGVTPGWQEVLRSKNVYGPYESRTVMHQGNTNINGPHQGGWVQLDSGEHWFIHFQCKDAYGRITHLNPMTWTDGWPIIGIDNNGDGIGEPVSHHRKPNVGGTFPIVTPPDSDEFDNVELGMQWQWHANPKNTWAFINPGTQQLRLFSDLIPEDAVSYYQVPNLLLQKFPGESFTVDTKMTFRPNENKLGERAGVIVMGRNYASFALEDREDGIYLVYNINNGAQHGEKEKEVFAQKIDTNTVYLRIKVGADFMTEFSYSTNGRRYRSMDTKFRATRGHWIGAKVGVFCTRQQTTNDSGFADFDYFRFSK

SEQ ID NO: 79 - protein, 336 aa, Alkalitalea saponilacus
MIKAVFISAFFLIVNLTVNSQVTEDPILNRISRYVGVETHKDTTMTHDPVMIREDGVYYMFATGWGITMFSSPDMIHWKHEYPIFTEVPEWIMEIVPDFRGHFWAPDVAYFNDQYYVYYSVSSFGRNTSAIGVVTNKTLNPDSPDYEWVDHGEVIRSIPGVTNWNAIDANIILGEDGTPFMSFGSFWGGLMLAELKPDGLSLAHPIEDLTLLATRTTGENPIEAPFIFKKDDYYYLFVSFDFCCRGEESTYKVVVGRSEKVEGEYFDKDGLSMLKGGGTIVVEGGDGYAGVGHNAVVAFDGVDYLVFHAYDMSRGGGSYLRILPIRWEDGWPEVDF

SEQ ID NO: 80 - protein, 343 aa, Alkalitalea saponilacus
MNLKSLFLNILIFIMTLIVVSCQSSTEHCGEPAPKPLFRDPVYDGAADPVIVWNHDEEKWFMFYTNRRAKDISLDGFEWVHGTRIGIAESYDGANWSYRDTANINYRMPDYTHWAPEVIEHDGLYHMYLTYVPGIFRDWRHPRDIVHLTSKNLLDWDFESVLELASDRVIDACVFQLPDGTWRMWYNNERAGKAMYYADSPDLYNWTDKGRVQIDRARGGEGPKVFEWKGQYWMITDVWSGLALYKSDDLLNWTNIPGNLVEEPGIGEDDKVMGGHADILISNDRAYLYYFTHPGRRDGVDPNDLFEQRRSSIQVTELFYENERLVAYRDSVTYVCLVPPVRF

SEQ ID NO: 81 - protein, 385 aa, Alkalitalea saponilacus
MNNSIYLSFIRLSFLLISLLVACSHNSEKGYYSSFIPGELWFDTDSVHINAHGGGILFHEDVYYWFGEFKTAGRGGNTALVGVQVYSSTDLYNWKNEGTALEVVDVLGHDIERGSVIERPKVLYNEKTGKFVMWFHLELKGQGYSAARTAVAVADHVTGPYEFIESLRPNAGHWPMNFNQEFKELTETIDDFEWWTPDWEEAVHKGLFIRRDFEGGQMARDMTLFLDDDGTAYHIFSSEENLTLHIAELSDDFLSHTGRYKRIFPLGHNEAPAVFKHNDLYYMIASGCTGWEPNAARSFVAENVFGPWTALGNPCVGSGAEITFQSQSTFVLPVQGKEGAFIYMGDRWRPHNPIDGRYVWLPIVFKNDRPIIEWYDEWDLSIFDN

SEQ ID NO: 82 - protein, 723 aa, Alkalitalea saponilacus
MKQMNSVYSVFKPILYGCIVILTLLNVSCSNKDKYTAYLFAYFIGNGPGEEAIFYAVSPDGFNYVALNNNRPVIAADTISSRGGVRDPHILRAPDGKFYMVVTDLFVSNDGWSNNQAMVFLKSDDLINWTHSVVNVSELFPNFHDVRRVWAPQSYFDEEEGKIMVYFSMLQPGGYDIIYYAYANEDFTSLETEPKQLFFHPENRSCIDGDIVKKDGQYHLFFKTEGHGNGIKKAVSDRLTEGYVMHDEYLQQTNEAVEGSCVFKLIDSDTYILMYDVYIRGEYQFTQSTDLKNFTVIDDEISMNFRPRHGTVIPITQRELESLINKWGTAGDLGIASVIGENVKTNNVVIHRDNGTIYVPVKYGTDLSSFEPVFESFFDARIRPSGPQDFSQGSVEYTVSVKGLTDKKFNVTVKVDNNPVLTGYYADPEIIWSEKHQKFYLYPTSDGYHGWSGDYFKAFSSTDLVNWTDEGVILDLVEDVPWGPRNAWAPAMIEKKMGDTYKYFYYFTAAQKIGVAVSDHPAGRFEDIGEPLIDWKPDGVRGGQEIDPDVFTDPVSGNDYLYWGNGYLAGAKLNEDMISIDKSTVKVMTPVCGTFREGIEVFYRNGIYYFLWSENDTRSEDYRVRYAMSDSPMGEFYIPENNLVIAKDPSKGIYGTGHNCVIQIPGRDEWYIIYHRFTRPEGITMGGNAGFHRETCIDQMTFDENGYIIRVQPTLEGIVPVSL

SEQ ID NO: 83 - protein, 319 aa, Alkalitalea saponilacus
MKKVNLLIYSIIAAFFLLFSSCNQQTSSEENRYLFSYFKGNGESGLHLAWSEDGLIWHELNNGQPILEPTAGEDKLMRDPCIIQGPDGRYHMVWTVSWNERGIGYAWSEDLINWSEQQYIPVMEHEPNARNTWAPEITYDEKNDKFMIYWATTITGLYPETFSELEDGLNHRMYYVTTKDFKEFSETKLLYEPGFSVIDSHIVPHNGEFIMFLKDETIEPPAKSLHVATSKNLTGPYSQPLVQITGDYWAEGPTSLYIDGTWIVYFDKYIEWTMGAVKSTDLENWEEISHKISFPSEVRHGTALKIEKEVLNNLKQQLN

SEQ ID NO: 84 - protein, 573 aa, Alkalitalea saponilacus
MKNLLIVLCCLLISCKTTEHLNTTDFTTICNPMDLSYRFGMEEPSRREAADASIVWFKDRYYMFVSKSGGYWHSKNLADWIFIETTEIPVEEYAPTAIAIDDTLYFLGSSNDLSTLYKSVDPLAGTWQVAVEELDMPVWDPAFFLDDDKRLYLYWGCSDVNPLYGVEVDYHNYFAFMGDPVALVYAQPERYGWEVPGDYNELINQAPWIEGAWVNKINGIYYFQYSAPGTEYKSYADGVYVSENPLGPFTYQPHNPFVYKPEGFAAGAGHGSTIEDQYGNFWHVGTITISMKQVFERRLGLHPVFFDDDGMMYSITRFGDYPLIIPNHKVYSHDELFPGWMLLSYNKPVEVSSSYEGHPSSKMTDEDIRTYWAAESGGNNEYAIIDLQELYDVYAIQLNFAEHNTNIFGRQPGLFHQYTVEYSLDGETWNMLIDKSENKSDNTHDYTQLPRKVNCRFLRINNIRVPDGQFALSGFRVFGKGFGDKPLEVNRLEVTRNVEDRRRVHLSWQASDGAIGYNINFGIDPDKMYHHYQVYDLTSLDINSLAIDSEYWFTIESFNENGITESSLLVGPK

SEQ ID NO: 85 - protein, 325 aa, Alkalitalea saponilacus
MKKSLLFVAGLILAISFIRCDQTQEIKYSGNPLFDEPFTADPTAIVYNDTLWLFTGSDEQEEGVDGFLMRRWYVFSTADMVNWTNHGAVLSVDDFEWGSHNAFAADVVENHGKFWWYVPIVHADPAARVHEGFAMGVAVADHPAGPYHDPIGKPLIADTTANSIVLNIDPDVFVDDDGRVYMYWGSWDEVRVVELKSNMVELAGPVMNVEGLDNFFEAPFMHKRGDIYYMSYAAGYPSRTEYAISDNPLGPWVEKGVINDVIPNSPTNHQAIVHFKGNDYFIYHTAGLPNGGPFRRSVCIDKLEYDENGLIKKVVRTTTGVPQIK

SEQ ID NO: 86 - protein, 316 aa, Alkalitalea saponilacus
MEKYNSNKPLIEQRADPFIYKHTDGFYYFTGSVPSYDRIELRKAKTIDGLKDAKTFDVWHKRETGIMSQHVWAPEIHYLDGKWYIYFAASKVDDIWRLRPYVLECKGQDPLSDEWIELGQMQAADGDEKSFIDFSLDGTVFENNGKRYFSWAEKTGGQFAASNLYLAEMESPIKLKTPQFMLTTPDYDWERIGFWVNEGPAVIKNSGKVFITFSASATGACYCMGIMEADEGSDLLDRNSWKKSRYPVLKTDYQKKIFGPGHNSFTVAEDGTTPLCVYHARDYEEIVGDPLYDPNRHTRVLPVKFDDEGRPLFELW

SEQ ID NO: 87 - protein, 527 aa, Alkalitalea saponilacus
MRAYLKLLVLSSLIFTIGCSDDDDLIPNGDETGNQQEFRGPRYSDDYSMISSWSSRNSWNLANVHDPTVVKDGDYFYMYQTDASYGNVHVGHGHFPVRRSRDLVNWEFYGMAFDHVPLWVKDSLNNMRSRMDPPLPAIENPEYGFWAPHISKVGDEFRMYYSIVVINPIVGNNSDYSWTERAFIGLAVSRDLASNLWEDRGMVVCSEPDGLETYSRTGPHDWSGYFQFNAIDPSFIVTPEGEHWLIYGSWHTGIAAVQLNPETGKPDSWNSLEDYGVRIAGRGNLATNRWQALEAPEIVYNEETGYYYLFLAYDELSVAYNTRVARSKSITGPYLGIDGGNVTEGAECWPMLTHPYAFSGHHGWVGFAHCSVFRDPDTGQWFYASQARLPENLPGVNASNAIMMGHVREIEWTSDGWPVVMPQRYAAVPETDINKEDLVGRYDVIIKSYDYQKIQNSRTAEFHSDGRVTGALSGTWNFDEEKKRLTIGNLELIVKDAWDWEASPRKTTITFSGLTSDGRPVWGKLRE

SEQ ID NO: 88 - protein, 584 aa, Alkalitalea saponilacus
MELLTSAKLKILFVMIFKKAKTILSSLLIIIAFAMCTSPYETVEVNNPILPGFYPDPSVCKGPDGYYMVHSTFGYFPGIPIFYSPDLINWEQIGHVMHRPDQMQLDSLSLAGAGMFAPTIEYHEGTFYVACTEVYGRGNFVVTATNPAGPWSDPYFFPEVIGIDPSLFFHENGKTYIIYNSDAPDDQPLYEGHRTIRMFEIDIEKMQVVGNQSILVDGGVDISEQPVWIEGPHIYRVGDYYYLSAAEGGTSVNHRQVIFRSEDIWGPYIPWENNPILTQMHLDPNRPNPITSTGHADMIQDLKGNWWAVYLACRPYEGNHYNTGRETFMSKVEWTEDGWPVINPESEVIPFQFEFDAALKDKRVTKPLHGNFTVRDDFDQPSMDFKWVQIRTPKSSWFNLIPEKGVLNMSLLPASTIKQFNPSFLGRRQQHMVCNATTSLEFKPESEGQHAGLAVLQNEHRYYYLAQSLEDNLPVISLYKSVPNAIEDEMVVLATKRLSDSLGENLYLRIESDVDVYRFFYSYNGDKWFQIGDEQDARFLSTETAGGFIGSMFGLYTKTTESSEGGISANYHWFEYTGNDDIFK

SEQ ID NO: 89 - protein, 333 aa, Alkalitalea saponilacus
MIRSLVVLSLLVAGALVEIAHSQEFNYDNPLIRQRADPWIHRTDCGIYYFIATVPEYDRIEIRKSNTINGLADAEPVVVWRKHDSGPMSHHIWAPELHRVDGKWYIYFAAARAENIWKIRMWALSNDSDDPTTGEWVEEGQIRTERDDFALDATVFEHKGEYYYVWAEKTRPDNNSGLIMSKMKDGVTLIGPEVVISEPEYEWEMHTYAVNEGAAVIKHGNRIFMTFSASATDHTYAIGLLWAYKDSDLMDPNSWHKLPEPVFYTNEKFNRFGPGHNSFTVAEDGKTPVLVYHAREYKEIDGFALDDPNRDTRVRTFRWNDDGFPDFGQEIGD

SEQ ID NO: 90 - protein, 526 aa, Alkalitalea saponilacus
MKRNLFTATFLILILAVSCSTQKETPMATNPIIFADVPDIAIVRVGDAYYMSSTTMHMSPGLPIMRSYDLVNWELVSYAYDILIDNEMMRLENGQESYGFGSWASSMRFHDGVYYVSTFAATSGKTHIYTTTDIENGEWQEISFEPDLHDHTLFFDDDGRIYMIYACGELRLVELKPDLSGIIPGSEIVVIEDASSIAGEHIGLCAEGSQLLKHEGMYYLFNIVWPVNDMRTVLVHRADNIAGPYEGRVILKDRGIAQGSLIDTPEGDWYAYMFRDHGAVGRIPYLMPVDWVDGWPVLGIDGKVPDTLDIPAGDGGISGIVASDDFVREPGDEKLPLVWQWNHNPDHRFWSLSDRPGYLRLITGRVDANVLQARNTLTQRTFGPQSSAYTRMEIGNMNNGDCAGLIALQRDYGFVGVRKENDKNYLVLELAENNNPQELERVLIDQDHIYLRIDCDFEDMVDLAYFYYSLDGNEWIRIGKPLQMVYTLIHHFMGYRFGLFNYATETAGGYVDFDFFKVNDEIINPY

SEQ ID NO: 91 - protein, 322 aa, Alkalitalea saponilacus
MVRKHFLKNMYIADPHAHVFNGKLYIYPSHDYEAGIPEDDLGSHFAMKDYHVFSLENIDDEITDHGKALDVDDIPWAGRQLWDCDVAEKDGKYYMYFPLKDKTDIFRLGIAISDKPEGPFKPLPTPMDGSYSIDPAVFKDDDGKHYMYFGGIWGGQLQRYRNNKAIECGQQPADNEPALCAKVAVMSDDMLNFGEEPKDLVILDENGNPMLAGDNDRRFFEASWMHKYKGKYYFSYSTGDTHKICYATGDNPYGPFTYQGVILNPVIGWTTHHSIVEYKGKWYLFFHDSEISGKTWLRSARVADLNHLPDGSIETITVEYDK

SEQ ID NO: 92 - protein, 339 aa, Alkalitalea saponilacus
MDTFVKFRIVIVTFTIASFFQSCTEKKEEIRFNNPLVLQRADPWVHKTDDGIYYFIATSPEFDRIEIRKSETINGISDAEAHVVWSKHASGPMSHHIWAPELHRFNDTWYIYFAAGRSEDVWRIRMWVLSNDSEDPTQGEWVEEGQIHTQRDAFALDATTFEHRGQRYLIWTENGLNDFRGTGLLIAEMKDHATIDEREVIITKPEYDWEIQGHWVNEGPAVLKRNNRIFVTFSASATDHNYAIGLLWADKDSDLLDPASWNKLPEPVFYTNPEFNRFGPGHNSFTVAEDGKTDIMIYHARDYMELQGSPLSDPNRHTRARVITWTEDGFPDFGQDIDD

SEQ ID NO: 93 - protein, 332 aa, Alkalitalea saponilacus
MKTYTFFSLMALLALASCKSNHTSLDGVAYVKGRHVYTANHEKLVMRGVNEMFIWSDDLTGDTIIPEIAKTNSNTLRIVWLTDSENINATPENLDKIIQNTVDAGIFPMPELHGATGKWEKLQEQVDYWVRPDVVKVLKKHERYLLLNIVNECGGHDVDAETFRIGYELAIDRIRATGLRCPLVIDASGWGQDLDILLETGPGLLKHDPLSNLIFSVHMWWVAEDGSTQRIIDGIEQSVNLNLPLIVGEFAPMGVNCARHIDYETIMEQCQKHDIGWLAWSWGAVGNGDCAEMDMTRGELRGKFKGLTDWGLEVAVTHPYSIKNTSIKPSLE

SEQ ID NO: 94 - protein, 577 aa, Alkalitalea saponilacus
MKQKLLLLIICTSLSLAVFSQTRQPAFEMNERLGRGMNMGNTFEAPSETAWSNPWQPQYFEMMADLGFNHVRIPIRWETEARSMDEYPYTITASFMERIQEVVDNAIENGLIAIINMHHHELLLANPSEQYDRFIAQWVQIAEFFKDYPDEYLLFEVLNEPHQAITPQMWNDMFADALEVIRETNPTRVVLMGTAEFGGLSGVRHIELPEDDYLILSVHYYNPFQFTHQGADWVEGDADEWLGTKWYDTVEERNFIINEFNYTIQFSNDNDVPIHVGEFGVYSRADMESRARWTTFVARWFEEQGFSWAYWEFSSSFGIYNRNTGNYRTELVDALLNNSMPEPASLNSHIIYESDFTEGEDGWAFQLGGEAAGTMSVENNQLEIEITNGSSLGWHAQLFRPNISLENGKLYRFSFSASASFSGNSTVYMGRNAPDWDAYSDHHGVQFTSELQHYSYSFTMNADSDPEARMAFDLGGNTGLFVLRDVKVEEVLLPSSTNEMAASLQSVYPNPVMDRLYVRSNQIISRIKVYSISGVQHFSSDFNSYETDISFSEFSPGYYLVKVMDANGKFQIHKILK

SEQ ID NO: 95 - protein, 570 aa, Alkalitalea saponilacus
MKVFLVFLSVLIFAACKDDDEVFNLLEVDVSEIELDADKTTGVFTITTDADSWEITNPATEWLSLSRTSGTGSIAMIMVTVDGKTPEVRSAELVINAGNAPPVTVTVTQLDSEFVYELTSNRTSLTIRRLGGSQTFDINTSAPEWSLEIEGDWINVDRRTGTESSVTITVSADGNESGAERKGKITIRAEYAPQRVVEVSQLALYPSYNISPPEPDMTGVERTASELAQDILIGWNIGNSLEVPSGETGWGNARTTQALIDAVQAAGFNAIRIPCAWNSYADQNTAEIDPNWLARVKEVVDYCINNDMFVIINTHWDGGWLEENPFYSKQDEINLKFTAFWEQIATYFRDYDERLLFAGTNEVRADYGIPTTEHITVQQSFNQNFVTTVRSTGGRNAYRNLIVQTYNTNIDHGINFHVMPEDNVENRLFAEVHYYDPYQFALQDSGSGIYTVWGESFIAADSDWWGQEDHVDRQFAKVKSKFVDNDIPVILGEYGAIHRSALTGEDYEAHKASREYYLEYVTRSAIQHGLIPFYWDNGHRGNNGFALFYRSNGNIFDQGALDALMRGANE

SEQ ID NO: 96 - protein, 518 aa, Alkalitalea saponilacus
MKKSILLLMVVALLIGCATNDEKVVKGNQIFLNFDQAELVINKDVYGHFAEHLGRCVYDGIWVGPDSDIPNYKGYRLDVLEALKELQVPVLRWPGGCFADTYNWKDGVGPRSERPKLVNVFWGGDVEDNSFGTHEFLELCQILGADAYIAANVGSGSVREMIEWIEYMTSDQDIPMANWRRENGREEPWDVKFLGIGNESWGCGGEMTPEFYVNLMRQYSVFARQYGGSDMIRVGCGSHQFYYHWTEVLMREGRNHMEALSLHYYTIPTGDWGIKSEATGFDEDLYFSALRNALRMDELLKGHIEIMDRYDPEGRVELYMDEWGIWTDPEPGTNPAFLHQQNSMRDALIASLTFDIFHRHARRVQMANIAQMVNVLQAMILTDGDRMILTPTYHVFNMYKFNQNATYIPVEITTEKYAFENETIPAITGTASTKDGKVFVGLSNLHASETLTIDVDISGGNANRVLKATILTAPEFNSHNTYDNPNVVAPAEFAGYELTAGNLQVVIPPYSVVTFEME

SEQ ID NO: 97 - protein, 692 aa, Alkalitalea saponilacus
MRQFIYISLLLLISGFVSAQTFYRGNDLSYVNQMEDCGAVFKEDGIPKDPFRIFADQGTNLVRVRLWHNPDWQNRLSQPEGVKSQYSDFEDVKLTIMRAKAEGMKVMLDFHLSDFWADPGQQLIPSAWLSVANNVDLLADSVYNYVSKVLLALDEDDLMPEIVKIGNENNAGILRHTTLSDNFQVSGSVSDNWSRHARLFNAGIRAVRDVGADASVNPRVALHFSNIRNSINWYQRLIDNGVTDFDIIGLSYYYAWHGFSIADLGNTIRSMRNRWSQYDVMVVETGYLWTTENFDSLGNIINTPDPEYLPVTPLKQLEYMVDYTREVKRSGGIGVIFWEPAWVSTPCRTPWGVGSSHDHVVFFDPLENNFMENGGGRWTNAEFYENVSNSRKVTFKVDMEERDTEGGVYLSGSWGNGELLKMESLGNNVFWTFAYLPVGSEGGYFFVDGNDISNRETIPEGCANWEGIDRKYQVGNSNVIYEFVFGSCAVITKINPTVTFMVDMSGQDVSRGVFITGEITQPEWTIEEMSHLGDGIYSWTTQLTPGDDVLAYYFMTNSNWDNLSAYREVVPAECHGKWSDRGIVVGRNDTIVRNVWSSCETFGLTSAAELNQINDQLAIVTNSGNFKEIHIHLQSLHPYFDIVVYNSLGTKLYKRKVYDGIVDVHVAINSSGLHFVHVSNGINTEVHKVILR

SEQ ID NO: 98 - protein, 404 aa, Alkalitalea saponilacus
MRKAGIFVMLIFGVLSMVLSQACSDDKKKLVDVIDDENENDNSSKEFMMGVDLSYVNQIEDNGGVYLENGIATDPYEVFKKHGANYVRLRLWHNPDWVFDLYDNNPPLYSGFYDVMRSIQRAKDAGMSVLLDFHYSDTWADPGHQDVPKAWQDITSIEVLSDSVYNYTYHILNRLHSKGLLPEMIQVGNETNCGMMFTNTKPGFPSLNVCQGNWSHFGQVINSAIKAIRDIDSRVGQETIVALHVADPATMQWWLPDVIQKGGVMDFDVMGFSYYHIWHTTISFNQISGVIEDLINRFNKDIVLLETAYPFTTANNDNYPNIFYTQNVVPGFPYTVEGQKNFMISLVQNLKNAGAIGAFYWEPAWITSDMRDLWGTGSSWENCAFFNFSGNLTEVVEYFKYEYE

SEQ ID NO: 99 - protein, 716 aa, Alkalitalea saponilacus
MSGKICRLLVLFFLLPNIILAESGEKLWLRYLPLDNAKVVDYTNAIRSLVVAGDDAVISAAAEEIQMAFNGLTGNDLRNVNRPGAGALLIGTPENRLIRDLELSSELEKCGEEGYIIRTFPVRNGQMTVIAANTSAGVLYGTFDLIRRMQTGESISKLEVNESPAFKIRVLNHWDNLNGTVERGYAGHSIWFNRPEDWSVRSAQYKYYARANASVGINGTVINNVNADPNVLTAEYIEKYARIADIFRPYNMKIYMSVNFASPAVIGGLENSDPFNPAVQQWWKDKAAEIYQSIPDFGGFLVKANSEGQPGPMDYGRTHKDGANMMAKALQPHNGIVMWRAFVYEPGDDERSVQAYNEFMPFDGEFEDNVIVQVKNGPVDFMPRESFSPLFGGMQKSPVMIEFQITQEYLGHSNHLAYLSTMWKEVLDAETFAKGVGSSVAKTTDGTLFNHELTAISAVSNIGRDINWTGHHFGQSNWYAFGRLAWDYDLLSEDIAEEWVKMTFVHDQKFVEPVVDIMMRSREAVVNYMNPLGLHHIMGWDHHFGPEPWTDIPGAREDWLPRYYHNASEFGIGFDRTTNGSNLVSQYHSPLNKIYNDPLLVPENLLLWFHHLPWNYRLQNGLKLWDAMVYKYYEGVEEARLFQNRWDRLEGYIDDRRFKEIQYKLKLQTTEAIWWRDACVLYFQTYSNLPIPAELERPVHDLDELKELKFDMKHHN

SEQ ID NO: 100 - protein, 573 aa, Alkalitalea saponilacus
MKNFFRLFLLSMVSIQLFSCTGHENIEKEMPVLYNQVGYITDAPKLLLVREEVNQVIIIDAQGNEVFSAIPEEPLFWDQSGDAVRKVDFSQLNVPGTYVVVLPETNENFEIRVKDQPFREITKAALKAFYFNRSGMAIEPQYGGRWARPAGHPDTIIYVHSSAADDNRPEGTIISSPLGWYDAGDYNKYIVNSGITTYTLLSALTHFTDYYKKLDVSIPESGSGVPDLLTETLYNLKWMLTMQDPYDGGVYHKLTTKNFEGMVMPHEATNDRFVVSKGTAATLNFAAFAAKAHRVLADYESHFPGLAEKCLQKAEKAWGWAMSNPNLPYVQPDDIFTGGYGDRNFSDEFFWTASELFLSTGKDEYLDVIIEKYSKPVVPSWNQVYALGFISLLNNYDELPEIIRNLGLKNDFIALVDELVGVSKTAPYGVSIQNFVWGSNSQVANEGMLKIKGYQLTGNRYYLYSALSDLDYILGRNATGYCFVTGFGYKRVMNIHHRPSEADDNEAPVPGFLAGGPNISVLTDCGPEVERSPYPAKSYVDLECSYSTNEIAINWNAPLVYLSGAIDALLTQN

SEQ ID NO: 101 - protein, 849 aa, Alkalitalea saponilacus
MRRIILAIIGLLTTFCLVGNEANINRSYVDDEGVLRWSADDSEITGFGVNYSLPFAHAYRMANRLGITHEEAIKQDVYHFARLGLDLYRVHIWDVEISDVEGNLLQNEHLRLFDFAVSEMKKRGMKFVITPIAFWGNGWPEPDFDTPGFATKYGKEGCLTHPDAIKAQENYLYQFLNHINPYTGLAYKDDPDIIAFEVSNEPHHDGTVDEVINYINRLVGSMRKTGTQTPIFYNMSHSIHLVDAYLNADVQGGTFQWYPAGLVANRQINGNFLPHVGEYYIPFADHPLFKKMAKIVYEFDPADVGGNYMYPAMARSFREAGIQLATHFDYDAMFLAPYNTNYGTHYMSLPYAPQKALSLKIASAVFHEVPRYSNYGGYPNNNHFEDFRIDYENDLVEWVTNETFLYSNNTTSTPDNPALLKKIAGYGNSPLINYDGKGAYFLDRIGKDSWRLEVMPDAHWIDDPYGRVSLENQVAAVSYNIREMKVDLSCLGTDFTIAAINDGNDYNTEAKEGTFAIVPGVFILQNKNSVLEFSPYQTLGNIRMNEFVAPEADLSEIMIKNNTVSQACAGTRTSIHFEVISPEPPQKVEVIMYGNGGSSRSEAVYMGADIYKVDIYKNHLVHGILNYYIVLTFNEKIKSFPAGLEGQPGDWDFYDHSLYTIKFIPDGEPVLVWSALDDWSETLRIWHPGVSLKPLGNRNAALHLKMDELPDRNLKKGSRKDYSFKFFFGDLLSGRSSRIANSKNLVLKAYTQLNDSQPIIVGLVDVNGIAYSVEVDIIPGKLIYNISLDSLIQSEFAVTPGAYPEYLPHFQSSEYQFQFKPEKVESVQVSIRQGKLDEVDLWIESIWME

SEQ ID NO: 102 - protein, 618 aa, Alkalitalea saponilacus
MNQAVITSIILLFSFSSLLSGQTGRNQIECWPSEWWIGMQNNRLLLVIQGNNVAQSQAEINQPGIIIRNQYPAQNRTHLFLEIEISNNASPGIYPIRLSNRNQAVGVVNFTLNNRVTNFNPARLTGADAIYQIVPDRFVNAVPANDNINGYFERADRMNPAGIHGGDLQGIINSSNYLRQLGVTTIELTPVYETNQLVLSYERFSPTNHYKVDSRLGSINDLTNLVSHYRTRNIKVILTKVLHKAGNQSSLIQNLPASDWIYQRDNIHSGSDNPIVFADPYASREDIGRQTNRWESFDSPSLNHNNPEVRRYLIQNVLWWIQKTQPDGIKIEKTHLLHPLLLQELSQAITLDFPSLNLIASAETSSVVHNKYWKTGANGEFSFTHITDQPLYRNWMDVFAEYSRPNDMLFNIYKTKARDRAYSDAASQLIFAGDNHDLTRLFTLAEKDLSIFKMYAGFLFTTRGIPSFLYGSEVMMEGLAAQGTGFLRGDFPGGWPGDQVSAFNPNTLSNQQREALRYFTALLNWRKNNPDLMTGNTIHFEPRDNIYAYIRESEHKLLLVIINNHISSPKRIEPGRFSASIGNIGQVTNIATGEVSSGFGNIILNPKSILMLELVKNQ

SEQ ID NO: 103 - protein, 964 aa, Alkalitalea saponilacus
MKLLSTILLIGMLTCSVFAGMAENNSYVFEEKGEAFFVLSDMEYTASLLINSDDSPSVTRAFGDLQEDIYRVTGRKPELKYDEVSTAKYAVIAGTLGQSKLIDDLVNRGHIDKQELEGKWEKFIIKTVENPLPGIENALVIAGSDRRGTVFGIYDVSEKIGVSPWYYWADVPIKKKNQIYIKPGTYTDGEPVVKYRGIFINDEAPALRNWAIENFGGLNHKFYSTVYELLLRSKANFLWPAMWLPSMFYVDDPLNPKVADEYGIVISTTHHEPMMRAHNEWNHFYGGEWNYETNKENLREFWREGVERIGDYETFVTVGMRGDGDLAMTDETATELLETIIADQREIIADVTGKPASETPQLWAIYKEVQDYWDQGMRVDDDILILLCNDNWGNVSLLPKEHELDHKAGFGMYYHFNYVGAPVSYRWHNVTQIERVWEQMKITYDFGVKELWLVNVGDIKPMEFPISFFLDFAWNPEAIQAGDLPNYYINWAERKFGDTHKHDIAELIALYTKYNARRTHEMLSPETYSIENYREADRIINDFRLLLERSKEIYEQMPETHKSAFYQLVLSPIEMSSNLNELYVTAAKNRLYALQGRASTNIYVDKVRDLFFKDDELTRQFHEDLEDGKWNHMMSQNRIGYTSWNHPRANIMPAVSYIHIPNKPKLGFEVEYGSEAVWAGFSIEGEPTFSDSFSEFDPYNQQEYYVDIFNMGEGRLIYSVEAKNDWINLSGTGGSIEFDERVYVSIDWEKVPDGNPVGEIMIKGAGQEHQVKIPVRNELPKASGFVENNGVVSIGAANFTNKFDSEELCWTVVPNLGRESSSIIVEPFNSPTQTLSENSPMVEYEFTVFDAGEITVEAYLSPTQDFKKQGGLKFAISINDEKPQIINMNEGEIVPDYKYADWWMQSVGNQIKIKTSRHHINEPGKQTLKLWVVDTGIVFQKFVIDAGGLRESYLGPPESKYIGR

SEQ ID NO: 104 - protein, 726 aa, Alkalitalea saponilacus
MKSFYSLLILFLLFAPLFADNPLYLDPDQEIEVRINDLLSRMTLEEKVSQMANTSPAIPHLNIQEYEWWNEALHGVARSGIATVFPQSIAMGATFNPELIEKVATAVSDEARVLHHAAARRDIRLRYGGLTFWAPNINIYRDPRWGRGMETYGEDPFLTGVIGTAYVNGLQGDHPRYLKTAAGAKHYAVHSGPEHGRREFNAIASTKDLYETYLPAFKTLVDAGVEAIMCAYNSTNGEPCCAHNYLINEVLRDKWGFKGHVVTDCWSLNDFFTSINVAEDAVEAAALALKNGVDLECGSVYNPNLVTAVERGLISEDQIDVALSRLLSTRFRLGMFDPEEINPYANIPDTVLNSSTHRTLSREVAVESMVLLKNNGILPLRDDLSRYFVTGPNASSIHALIGNYYGVNDRYVTILEGIAGRVQIGSQVQYRPAILLDRPNVNPIDWSTGSASVSDVTILVLGITNLLEGEEGEAIASPYYGDRLDYSIPENQLDYLRRLTRNENNKIVAVIVGGSPMNLKEVHELADAVLLVWYPGQEGGNAVADVLFGDAAPGGRLPVTYPVSLDQLPPYEDYSMEGRTYRYMKEVPMYPFGYGLSYTSFEYSDISLADRRIRRDGKTTVRATVTNSGNMAASEVVQLYITNPPSRVTRTPLFSLRGFEKIFLEPGESREVKFEIARDMLVLIDDNGQEIIDSGAYTIAIGGAVPTERSVELGMPVPVRATLNVR

SEQ ID NO: 105 - protein, 886 aa, Alkalitalea saponilacus
MVDSLNIGQIRGKINIIISFLMIFFLSSCNQEKMAFMDTSLDNEERVKDLVSRMTLEEKVFQMLHEAPAIERLGIPEYNWWNECLHGVARAGLATVFPQAIGMAAMWDDQMMFDIADAISDEARAKHHDFAKQGKRGMSQGLTFWTPNINIFRDPRWGRGMETYGECPYLTGELAVNFIRGLQGDHPDYLKLVATAKHFAVHSGPEPDRHSFNVHPSQRDLVETYYPHFKKAVKEAGVYSFMCAYNRLFDEPCCGSEYLNSLLRDEWGFEGYVVSDCWAILDFYNPGDHEVVENAAQASALAVRFGTDLNCGSSYPALLEAVANGYITEEEIDVSVSRLILARMKLGMFDPPSMVPFAHIPYDVVDSELHRKLALEAARKSMVLLKNDNNTLPFSKNVSSVAVIGPNAHNVDALLANYNGYPSEPITPYQGISRKLPSANVKYALGSRYAEEFPYMTVIPSHILFTDETLSENGLQSEYFNNIDFRGNPEFSGFDPKVDFQWWTNSPKPGVSNDEFSVRWSGYLVPDVSGKYALGVEGFSGFRLYLDDELIVENFSLYHSMTDFKFMQLEAGKKYKIVLEFYQDNNTHPMVRLLWDKPGQNLKQEAIELAAQSDLVILCMGLSPLLEGEEMAVDIPGFFGGDRTDIVLPAIQTDLVKAIMELGKPTVMVLLNGSALAFNWEADNVPAIIEAWYPGQAGGQAIADVLFGDYNPAGRLPVTFYKSINQIPDFSDYSMDGRTYRYFKGEPLYEFGFGLSYTTFDYSELNIDTQVMADESFDVSVLVTNTGSMDGDEVVQLYVSYPDNHMAPIRSLQGFRRVFIPAGESREVKFNISPDQIGLFHPEHGKVVSAGKIHVYVGGKQPDSISLKNGNVVMSKVEILGEFICR

SEQ ID NO: 106 - protein, 589 aa, Alkalitalea saponilacus
MIKVLLLLLSFWIFSDLIYSNDHPWGWASVNAEGVNGTTGGAGGTVVTVSNQSDLEFYANKSGSYIIQISGRINISPMGKDIRVGANKTIIGLGVDAEINGGVLAVESTSNVIIKNLIIADTVTDDWDGKDNDYDGIRIRRSHHVWVHHCTIRRHGDGAIDIVNGSRYVTVSYCVFEAHNKTMLIGGSDGETFSVENPHSVTLYRNWFKGTTQRHPRVRFGKVHVFNNYYSDMGQYGRQMGFTTWTGYAIGFGVDAKIVSQLNYFENVDRPTDRFDNSSRPAYIIDVGSVFVNSGSFTEQTTGTSWVPVDKYHFETIPAADVKSYVMLNAGAGRMNQDLGDGIYRGSGDLIDQLMLFEFSNAENWSVQNNFTFGKTVYGDRDFTILSVPEELEGKEWVSTAMNSRTNNTLDKYAAISLLSDGVVYVVHPNRVTEKPEWLSGYENTGLEVAVKESATVTRILTVFKKNVSAGVEVDLGINSNDGTTSTLMYFVIVDGEVSSSLTSPLESINCLHILQTGSGVKVEINVHTPGDFIVEIFDSKGRVVDLLHAGWKNSGSYSYDIIRGKYQRGLYVVRMRSSTLIQHAKFVL

SEQ ID NO: 107 - protein, 504 aa, Alkalitalea saponilacus
MSKKIFIISLLSFFAFFVLSACSDGNDSELEEIKSPKEENDENNQRPDPVEEEAFAFPGAEGFGKHATGGRGGRVIKVTSLEDFGPGSFREAVMASGPRIVVFEVSGTIELKTRLTIRNGDLTIAGQTAPGDGIAIANHEVYVDADNVIIRFMRFRVGDTADAEYDALGGRFRKNIIIDHCSMSWSTDECVSFYGNDEFTLQWCVISESLRMSAHEKGAHGYGAIWGGKNASFHHNLLAHHDSRNPRFGEFEGSAYALTNLVDFRNNIIYNWGNNSAYGAEGGNVNIVNNYYKPGPASRHRERIMSIDKYLRDPERATYDIWGRFFIDGNFVEGSTRATNDNWTYGVYNQFHSKYGTVSDEDKAAMRLDSEHPINGNVTTHTAEEAFDIVLEFAGASLVRDAVDARVIEETRNGTFTYSGSRGSTNGIIDSQEDVGGWPELDSLPVPVDTSGDGMPDEWKIAHGLDPEKNEANGRDLSTAYDNVEVYINSLVQHIMDAKAVFFD

SEQ ID NO: 108 - protein, 447 aa, Alkalitalea saponilacus
MNLSTKLILTVLIIISACSVSNSERINKTPAFPGAEGAGKYTTGGRGGMVYVVTNLEDDGPGSFRYGVNLQEPRIIVFAVSGNIHLKSPLNINHGNLTIAGQSAPGEGICIKGHGLRINADNVIFRYLRMRPGDIYPIEQDALTTMRHKNIIIDHCSMSWGTDEVFSPYNIENLTVQWCIISESLNDSHHSKGEHGYGGIWGGNRATFHHNLLAHHSSRNPRFQGARSLEKGQQELVEFVNNVVYNWGNKAAYGGEEGHYNIINNYFKPGPATNRSELSIILEPYTPIGKFYLSGNIVYGNEEASEDNTLAVSTQRGGPLDELIVYESFSVSDYQIRDTETAFKAVLKYAGVSNVRDTVDSRIIKEVKYGMATFGEGGIINSQNEVGGWPEFQYSEPLLDSDGDGMPDAWEIANGLDPNNPNDHNQYDLCSKYTNIEVYLNQLVEKK

SEQ ID NO: 109 - protein, 477 aa, Alkalitalea saponilacus
MKKLFFLLPATLLLLLFISCSKESESEKDDDEIIGFPTPDRSSIPAFPGAEGGGMYTTGGAGGRVYTVTSLEDTFEAGTLRHAVMQNEPRTIVFAVSGEIKLTRNLRITNGNLTIAGQTAPGDGITIRDYTVMVDADNVIIRFLRFRLGDETATEDDAIWGRRRKNVIIDHCSMSWSTDECASFYDNENFTMQWCLIAESLNESVHDKGAHGYGGLWGGNNASFHNNLLAHHKSRNPRFYGVRDGILSERAEMINNVIYNWGDNSAYGGEDGEYNIINNYYKAGPATNSHRSRIFEAYRGTDYGRFYISGNYVDGYPNVSENNWFGVDLKHGGSLNNLKVENPFEIYPVTIRTPEEAFELVLQHAGMSLSRDAVDTRIVEEVRNGTATYGGSWGSNTGIIDTQEDVGGWPQLATADAPIDTDGDGIPDEWEIANGLDPNDPTDGRKYILSPKYTNLEVYLNSIVFEKIGFGGTGIKQ

SEQ ID NO: 110 - protein, 800 aa, Alkalitalea saponilacus
MKRIQIFTKISLLLILFMLMPVVHAQQVTGNLLTEAATSVDFDERSFYMLVNRETGKAMDVEGRSILNDHNIIVADVDFAMHQVWRMDDLGSGRYNLVNGHSDKVVRHRDGNVRQERDGSSNNHRWNIEHLEGTYFRLVNAASINVVLAVDGNNVVGAAPNGSAAQQWEILRVYAEPIVPDFSLQGFASVGQGTTGGAGGEVVVVNNEADLIHYMQHPDPYIILIEGTITLGPGNHHSPSDNMHSIAPNKTLFGLAGATIKGGGFNIRGTRNDGVGEVTRSNIIIRNLTFDGPAPDDFINIEWGASHVWIDHNTFNGPNNDGIVDVKRESSFITISWNIINTNHKTMLLGHDASHHHDRGYLKVTYHHNYIYNSQSRHPRMRYGRAHLFNNYFKYIGDYVMGPGIEAEIISENNHVWESGRFTDWYHATGKVLERGQGSLINRINHDHDPRIVTSDIEWAPEDYYSYTLYPALSVRDMVQEYAGAGVLSWGDPMPESYTLSTSVEGQGSVNPASGSFGEDSEVQITATPASGWQFDGWSGDATGTDNPLTLIMNNNKSVTATFIEIPGGGDNGDNGDGQIGWKILYDWNFSAMPEYVSNFAVSGSQTIAGATLYNSIEVDGMADRSSEIDGATYTYNRRVKFGGAGSFSGGNPAARVYAFPVPGDAKITIVHQSASTSANRVLRVAHGANQVLETFTSPGSPHAMDVYFYAGDATTIYLYSESSGINLYHVRVEEPDYGAPTNMKDSFPVNKEVISVNYYNLNGVNLGKNFDALPAGFYIKVKKFEDGSFKTEKVLKERR

SEQ ID NO: 111 - protein, 956 aa, Alkalitalea saponilacus
MKKNLFTLFLLLLSASALISQNPDFSLVGYGDTTGDNSPRSNNTGRAGIHHTTTGGEGSNPQVVTYTGNDLRDVLRSGDYMGGMIYEIYDADMLAGVLLEFTRHHRNSNYSAPYQPVTFYIKSNLTNTGSTREIRIEDTENVSIIGMINGGEKADFHDLGIRIIRCSNVIVRNLRIYNVRQGASTGTEIAYSNNIWIDRNEYHSEGLLPEIHRDYYDGLLDIKHQSNAITVSWNIFRDHYKGLLLGHSDSPSAAPDNITYHHNLFLNLNTRAPLIRFANVHMFNNVFENIQGSATNCRMGAVVRIENNHYINAGSGTVDSQGNYQQGAVGWWYGSSTGYWHLIDNIFDNSPLDDKVWQNNLSSTSVPYEYAHVLHPAQDIYDLVYQFAGRVQSYEPDEDATLSALYIGDILADGFSPSAFEYSHEVPFGTPSAPTVSAITAQSEAGLSISQATSLPGTATVHVTSANGQESNTYTVQFTMYDPSDDATLAGITIDGEPIEGFSSTNFNYTIDLPFGSPVPVVNATLSWHEAGMAMYEAGSIPGTNSIQVTSADGTESNIYYIIFTQSDPSADATLSEINVNGSLISGFSPSQTNYTINIPDSEASIPQVSAVVNDELASVEINQADDLPGVATVEVTAQDGSKQTYTVTFTVTTNWLIYDASALPGSSSPSFSASDFDNPSFSLVDDTDGCIDDNQLLKLEHTSPSSKGNWRYDFPSGQIAVTIVARVKALPGAFDKVMVIDMQFAGSRERIYINSDNTYWLRHAGAGSVSGPNEQLPNGADINEWNIIRLTKQGHNVNFYLNEHPVPVESVVTGTSTNNNYFRFGDPFGDQTSGALIDWIIWDETGAYAPGEGSPIPSWICSTYGDNVSTVTPDYENQQKVDIYPNPVTNGLVNIALTGFEGNKKIKLLNLSGTVISISETSANSYVLPVNLPTGIYLIQINNADFGVTKRLIVR

SEQ ID NO: 112 - protein, 301 aa, Alkalitalea saponilacus
MKVYILTLFFLINIPLIAQDYSKNWKNVNYASDTLSFHNMDIFLPSVEKDSYPVIVYIYGSAWLSNSSKGADMNTIGKSLLDAGFAVVAPNHRASWDALFPAQIHDVKAVIRYIRANAEKYRLDTSFIGISGSSSGGNLAAMAGVTRNVRSFTLEGQEVDLEGEVGRYLDFCSSVDAVVAWFPPTNMLIMDSCGGTDFIHDDVNSPASRYIGGAIQENQTKTLLASPTTYASPNSPPFLIFHGNNDRVVPHCQSEVLYEALNDAGVDSELVIVEGGGHGPGVHEEEYINMMVDFFLQVYKN

SEQ ID NO: 113 - protein, 225 aa, Alkalitalea saponilacus
MKKLLLLISIFVLISVIVNSQSFIENAPEGFDLPQTEVLAGKIDTIVYESNTVGTTRNALLYTPPCFNFENQCPVLYLFHGIGGDEFEWYVNGSPNLIFDNLIAEGKMNPMIVVLPNGRAMKNDRAEGNIFERDKVEAFSTFEQDLLNDLIPHIEANYPVIKERKYRAIAGLSMGGGQALNFGLGNTNQFAWVGGFSSAPNTKEPNELIPNPSKINEDLELLYIS

SEQ ID NO: 114 - protein, 216 aa, Alkalitalea saponilacus
MRYPVLYLQHGSFENETSWSRQGKANIILDNLIAEEKAVPMIIVMDNGYAFKPDENQAVNNPNRPALVFEEVMMNEIVPLIDTRFRTKTNRENRAIAGLSMGANQTMRIAMNNLDKFSSYGGFSGTANFPSSDKIDVDTFLGGIFKDGEFVNESLKVLWLGLGTEEAEIFPLTVGAFRDMLHEQEIDYVYYESVGTGHDWLTWRRSLYQYTQLLFK

SEQ ID NO: 115 - protein, 519 aa, Alkalitalea saponilacus
MKNINLILLTLLALLIGSCSQQPGQVKVEGGLIQGVVTDDLLIFKGVPFAAPPTEDLRWKAPQPVEKWPGVLETFEYAPAPMQGGEPASGKSEDCLYLNIWTPAKSAKEKLPVLVWIYGGGFSFGSTSDPVHNGEHLARKGVVVVSIAYRVGQLGFLAHPELSAESPNGVSGNYGLLDQIAGLEWIQRNISEFGGDPDNVTIFGESAGGISVSMLCASPVAKGLFHGAISQSGGSFGPTRPTTYPGENMKTLQQAEQDGIAYVNRVGVSSIEELRQIDATELPLGMGMGGAWPIVDGYVIPGDQYELYEMGKFNDVPVLIGYNSDEGLSFPGGRTPQDYIDNVNRRFGPFADKLLKAYPVGETSVPRSARNLMRDAAFGWPTWAWANLQSEVGSSPVFFYYFDQHPEFAEDSPQADHGTPHGVDVPFVFMNLNADDPNVSESDLEISEIMGTYWTNFAKYGHPNGEGVTEWPKFTKENPNVMYLGPNAYLGPVPDEASLKVMDAYYKWRRTPEGKDWAK

SEQ ID NO: 116 - protein, 520 aa, Alkalitalea saponilacus
MKKMSFCSGLLILSLSLFLSSCKQSSDNNQNPVVNICSGDISGYLDDGIYTFKGVPYAKAERFMPPERVDGWQGVLECVEYGPIAMQINSWSPDSVMDEKDLFSVNIWTSGLDDTKKRPVMVWLHGGGFSFGSGSDPITEGKLLAEKGDVVVVSINHRLNILGFLDLSAIDDKYARSANVGMLDIVESLEWVNRNIENFGGDPDNVTIFGESGGGGKVGTLMCMPGASGLFHKAIIQSGTLVNVMTKEKSQEVGLALLDYLGISKDEVHKLKSIPYKELVVAGDSALRRTVGLRRPGTRRMFGFGPVPDGTDLLQQPFTPGFSNISQEVPLMIGTTFNEMMRTYYAETDLTFEQASVRLESQYVEETGRFVELFKQAYPDYTPQDLLSIDTVFRPITIKVADAASTRVAPVYSYMLTWKSPVDDGTRGSFHALDIPLVFNNIELGKHWSGDTEDAIALAEIMSSSWINFARSGDPNVAGVLPEWDAYTKENGVTMIFDDECKIVRNHDRELMDIVLSFEQ

SEQ ID NO: 117 - protein, 301 aa, Alkalitalea saponilacus
MRLYRVLIILYLIMISQLLISQQMIPLWDEIIPFNRDGIAVEEINENYRVSRVSVPGIFRFAACEMAVKQKPAIIIVPGGGYARQATNHEGVMVAKWFASRGYEAFVLKYRLPDEEIVENPAFAPLIDLQQAIHHVRSNADKYGVDAAKIGVIGFSAGGHLAGSASVMFDVPVNKNLKTEDVRPDFSILVYPVISMDDEITHRGSKINLLGENPMSVFVELFSLEKQASSEVPVTLLVHSMDDRAVPLENSLRYADALSEKGVDVTQLILPFGGHGYGFRENSGVEYWIEYLDVWLKNKID

SEQ ID NO: 118 - protein, 316 aa, Alkalitalea saponilacus
MPFNFIKIIRSTLVLIFAGLASNALAQDGTIYPMDNPDEPNAIVLGTGGVENQPAQESWFRQWGDPMARNITTATLTPFLPDPEKATGAAIIVAPGGGFRWLSLSNEGWKVAQALADQGIAAFVLKYRLFPTPESLEGFTESMNRTFAEATPREEGEAEAAPAPTRERRMAWSLDNQLEDAEAAYALIVKNAEKWGVDVSRIGMIGFSAGAGLTMHSTLNSEVMDLAFIGPIYGGMNAVEVPKNAPPMFNVIATDDFLFNGQFGIIESWYKAGIPVEFHLYQNGGHGFGLGNPDRTSNRWFDSFMYWLEVNGFLNE

SEQ ID NO: 119 - protein, 333 aa, Alkalitalea saponilacus
MKRGTKYFFAGILLTFALVLFLGPKPETPLYHTFVPKTPKTTLEAEAILTARESNLSIKPKNEASIVWVCDSSKARTRQVLVYLHGFGASHEEGNPVHRHVADRVGANLLLTRLYDHGLTDTLPMQHFSVQKFWDDALEYLSIARALGDEIILMGTSTGASLALLMASHFDDVNAIILLSPNIRVNDPNIWIMNQPWGLQLGRAITGSNKTISDHPAEWYDKYWYRQYSLNAVAELQQFLKIAMKPTVFKRVFQPALMLYYYKNEQEKDDVVRVDAMLKMFDELSTPSHLKLKQAIPEAADHVIGCHLRSGDIDAVKLALEVFIDDILNANVD

SEQ ID NO: 120 - protein, 347 aa, Alkalitalea saponilacus
MKHLILTVDYELFFGSDPGTVENCMIRPVRHLMEVLDDYGYKMTVFWDVLHFYRLKQLEDQVDSLRLEREMIEKQIRLLIKNGHDVQMHIHPHWLDTRWENNRWHFSYMRFSIHKLWDGWELNNIETIPGCITICKNLIEEICKKENPGYKVRAIRAGGYRIEPFERLKEALKHNNIRVDASAAYGMKSFNPAYPFDFRMMPPFLHYRFNTSVLKQEHDGFFWEFPKESIKVPVYIRMMFWFLRNMVYPFKSCYGDGTRLRFTRREQSGHWISELGARFYRLTPEDMDKYRWSWLVKKSRRNGMVVLHSKNMGPFTMEMLKDSLSKKEVAFHSLADRIKALKVYDDL

SEQ ID NO: 121 - protein, 378 aa, Alkalitalea saponilacus
MNQYLLLMVITVLSVISCADNRGEDFRNESPVNPGGFPDGDVPQMIVLGSDDNTNVEGMNWILDFMASRSHKDGTSLRMSFYSNSRSSADWHLPENHKLVEAHKRAYNLGHELGNHTSNHAFCVYGQTGEGQIRITQDSIFRIVDEFSHDLIHLVGMNPKHIVGFRTPYLAWSDSVFYVINNKGFWYDCSITESRLGPGRYIWPFTMDYGASGTIGSWWTENHGTSVGRHPGLWQLPCYSFQAPDSLFAYMDSLAGRTHNGLITGLDYNMWSAPRSGWLLNKDQSLAVLKHTLKLNLEGNRTPMTIGMHSQYYADDFNGFGFQNIPSAADRRAVVEEFIDYALQFDDVWFVTGAQVIHYMRNPVEKEYYNPDNYLFTK

SEQ ID NO: 122 - protein, 330 aa, Alkalitalea saponilacus
MNRTLIILIILISLVKYTALADSGEYAFVVASDGTGDFITVQEAINNVPDFRNNETVIFLKNGVYKEKLILPASKNNVTFIGESKDSTIIIYDDYASKLNRFGEEMGTTGSSGFFIFGNNFTARNITFENSAGPVGQAVAVRVSGDRIVFENCNFLGHQDTLYPHTSGSRQFYKNCYIEGTVDFIFGWSTAWFENCIIFPKKRGYITAASTNEDTSHGFVFNNCSITGSAPEHSFYLGRPWRDHAQTVFINCYMSEVVHPAGWHNWNKPHAEETAFYAEYNSFGPGASAENRVSWSHQLTSEQVAKYTIENVLGGDDNWNPLDRITNTNQ

SEQ ID NO: 123 - protein, 322 aa, Alkalitalea saponilacus
MTLKHFANIIVIFIFSISCAAQSTPHYDFIVAQDNTGDFTSIQEAINVTKAFPDEPVTIFIKNGVYKEKVRVYSWNTKLTLMGESTENTIITYDDYFDKINLGRNSTFHTYTLKVEANDFTAKNLTIENSAGPVGQAVALHVEGDRCSFINCRFLGHQDTVYSAGEGRRHYFYQCYIDGTTDFIFGEGTAVFQDCQIHSKSNSYITAASTPENIPYGFVFIDCNLTAEEDVDKVFLGRPWRDYARTVFMNCELGSHIRPEGWSNWSGTNRDESAFYAEYGNTGPGANTSNRASWAMQLTEEEAKHYTIENIFRFGIGEWLFD

SEQ ID NO: 124 - protein, 331 aa, Alkalitalea saponilacus
MTLLSNKFPLLIFLFLLPYAMYGQLVEIDGIPRDTSFNLISEFKKQQINYPDISLAKKGDTSALTIHHDITYLQLENRSLKLDIIYLSHLEKSKLPTVLLIHGGGWRSGDKSMEYPMAMELARRGYVSICIEYRLSPEAVYPVAVEDVITAVRWVRSNACSYPIDRQKIVLYGTSAGGQLASLVGTINGVDSVFNPPYHTEIDAVVNTLVNVDGLSAFIHPESGEGQDRPGRPSAATWWFNSTTDERPDLRYEASPITHVHSNSVPILFINSSIPRFSAGRDDMIEKLTEHGIYSQNFVHKNAMHTFWLFHPWFDKTVELTDDFLKKVLNP

SEQ ID NO: 125 - protein, 208 aa, Alkalitalea saponilacus
MKNTNLTTCPQLKTSFWNEEWKEIVFPKGALRKRYAISNYGRVVSFSDSFENARIVKGGTLKGYKTLPLRPFGKSTTFYVHKLVAEYFLPKPEEGQQFVLHLDYNKTNNFVSNLKWANRKETLAHQQHNPTVLDARQKVKERIPVEGPKLTMTQVMRLKKKLLDPDRKTKLRIIAKQFGVSEMQLHRIRRGENWGHVQVHFNDNVDGL

SEQ ID NO: 126 - protein, 256 aa, Alkalitalea saponilacus
MIDTHSHIYAKEFDQDRDEIIQRAKDAGVSGIFLPNIDVASIQRMHETEEKYSGFCKAMMGLHPTSVKEDYKEQLKQIEKHLNQRPYSGVGEIGMDLYWDTTFRKEQEDALNRQINWSRELNLPVVIHTRDAFPEIFSVFDKAYDPQLKGIFHSFSGSLEDAKHILSMPGFYLGINGVVTFKKSNLPEILVEIGYEKLVLETDAPYLAPVPYRGKRNEPAYLTNVINKLSEIFNVSIETLKETTTKNAIDLFGKID

SEQ ID NO: 127 - protein, 532 aa, Alkalitalea saponilacus
MKKLLCVLWISRFLLFLVLLFGCNRIPVTEVPSMPLIHLEFDNKISNEGVLPVTFRGDENVSFSNDGVSNYSLDLTSAAKFRKPVVVVKGDGQSFNDYPGLSIFFWVKAHPGDPYEYTIISQLADDELAPQGWLFGKTTSGSYRWMLTDGLNEAVYEPTSIRQPVANDEWHLLGYTLDFARKEARVYYNGENVAVFCLQNFNLDIFKGDIYIGGHPFSTNPIRDAFHGLIDEFTIWSRVLTPEQIKTLCGDERHLTRRRREARPDSLTIMTWNIWNGGRADGLFAGPQRVAEIIQESGADIISLQEAFDSGEMIADILGFYYYQRSPGLSILSRYPFGRTYNVYRPRHSGAVVVNLPRDNQIVMVPVALSYLPNLGPYIMSGHARADSVIIREMQSRGSEIRFIMWEMQSIQNSYSDYPIILAGDFNSGSHLDWTEANRENRFGLVIEHPVSKTIEDAGFIDAFRYIYPNEVKNPGFTWSPRYKEVMQDRINFIYYKGPGFNASWSRVIDQFEPGFPSDHAAVVVSFKWDDQ

SEQ ID NO: 128 - protein, 365 aa, Alkalitalea saponilacus
MFNNISKIIERDSKSTTYKYALLRGVIDIIQDNSPYISFVENRVQIPTGLLIEKWLLYYYPIIQSQTLIPQINGKTNLAFSSHLNKLISDYEPRGGFSAFYNDLKNKGIPEDLQGDLVELTKKIRDTITRMPMKYIGRSISNDFYSIFKYENQTLRSCSKIDLETLIVAFGTFSIPFEYYEAFKILGSFINGQDSILFKWAKFSVNASGNNLSVHRVLNEVLKSPITLREIKESKKLYKDILKKEGKVYCVWTGRNISNYDIDHMIPFSAWKNNDLWNLLPSDSRINNQKRDKIPTPEIIERQKNLILNYWEIIFKNQSKRFSKEIQVALLGNHSFDNWKNVGISQLQNRCSYLIENRGFEEWKI

SEQ ID NO: 129 - protein, 550 aa, Alkalitalea saponilacus
MVRFLRLHFTVFFLLTASILLSQNPHGYYNNAIGKKEAELKTALHDIIRYHTNLSYSALWVVFRQTDERADGTVWDMYSPIIRTLNTTRGLNREHSFPVSWWDGTRDESLAAYTDINHIFPSDAEANMAKSNHPLGVVGSNPTYNNGMTKVGQNIFPGYTGLVFEPDDEYKGDFARAYLYMATRYQDYVNRWRNFTMLQTNTYPVYQQWAINLLLEWHREDPVSTKELERNEEVFRIQGNRNPFIDFPELAEHIWGNKKDDEWIIEIDNYQSVLITPTNNTEVAFGTVVKGQTATRSLFFRGNNLTQPLSLFLYGTNSQFFNINVNEIPSSLANRAEGFELQVTYSPTQNTGNHTATILVSDGGMNGSVTVNIHGQSIAEDEIVPPTALPATDVTATSFQANWQAMEDTDFYILHVYEHDNGEAELLFSQDDIFDNFYEVVNLDPEKQYSYNVSREVSGIRTEASNTINVSAGTNINEETNDILVHTHQKNIYIHKTVSMLVNARVYNLSGHLIAQKTLINSVSKISVKTNGVYFLHIDGYGVEKVMINH

SEQ ID NO: 130 - protein, 213 aa, Alkalitalea saponilacus
MRLNERFKLIIEWFKENMPVAETELHYTNPYELLVAVILSAQCTDKRVNQITPPFFERFPSAEVLANAEISEVFEYIKSCSYPNNKSKSLVGMAQKLVGEFKSIVPSDVNDLQKLPGVGRKTANVIASVVYDKPALAVDTHVFRVSARLGLTRDAKTPLETEKQLVKYIPEELLAIAHHWLILHGRYVCLARKPKCNECGLKHLCHYYQKNGE

SEQ ID NO: 131 - protein, 834 aa, Alkalitalea saponilacus
MIYPDTFEEKLSFGKIRELLEEHCLSTLGKEWVDRMTFSENFTQVQTWLGQAAEMLRIEQEDAEMPASWFIDLRAPLKRIRVEGLFLEESELFDLRRSLGTIRDLIRFIKSREAEEYPHLNSLVANVMIYPAVIDRIDSVLNRQGKIKDNASPELARLRREIINQQQNATRRMASILRAAQKDGLVEQDISISIRDGRAVIPVPSANKRKLAGIVHDESATGKTTYIEPAAIVEINNEIRELTYAERREVTKILTEVSDFIRPYIEDLLFAYNFLGIIDFIRAKARFALRVEAIVPQVKEERAFHWIEARHPLLYLLLKAQNKPIVPLSIQFTPDERIVLISGPNAGGKSVCLQTVGLVQYMLQCGLPVPVMEGTSMGFFKNIFLDLGDEQSIENDLSTYSSHLLNMKNFVRNSNEHTLMLIDEFGTGTEPMLGGAIAEAVLEQLNQQGAYGVITTHYTNLKHYASQTDGIVNGAMQFDTHQLQPLFKLEVGSPGSSFAFEIARKIGLPESILEAAKNRLGEDHINFDKHLREIIRDKRYWEQKRRSIRERERKLESVSQKYEIELEQLTRERKDIIEKAKQEAAGLLAGTNKEIEKTIRTIREAQAEKEKTRKARVELDLFKESAIAGAGDNEELQKQLQAKMNKIRQRKERKKSQNQYSNTGELENQPAIPPQPVIDEIVEGDVVKLEGQPIPGEVMEVKGRDALVAFGQLITKVKISRLEKISKGDYKKAMRTESKVAAGLAERIRDKKLNFKPDIDVRGMRADEAIDRISVHLDEAVMCGVNQVKVLHGKGTGALRLMIREYLGTVPFVKNFRDEHVQFGGSGITLIELE

SEQ ID NO: 132 - protein, 300 aa, Alkalitalea saponilacus
MRYCLYIFLFAVVISCSRSGQLDVITFNSGSSIVSDSVNTWENRLPIIQQYFKNQNPDIIGMQQVNIKRLRSLSTILPAYSYIISQDIDEADADQLNPIFYKTDKFRVLSKSRFYISGEGVITQKDLVTCNQIHLINWTKLENIESGHIFFVFNVHFCKNNEDEDIISSALFLKRIRELAGNAPVIVTGSFHMNEASRTYRIMRSNWDRFLSIENSSELAKSGKNRIYPTYNAYGKEEFHAMSDYIFVNSYFDVRRIETHRVKNQNVYISDYYPVSVNLKFLFNRRMRQGNITELPWRNQ

SEQ ID NO: 133 - protein, 348 aa, Alkalitalea saponilacus
MMPSPKTLLPFLILLLFWFSQSVCCQFRASDTDTIAGIMFYNVENLFDTRNDPKKRDDDFTPEGVRRWTYSRMREKFNNIGRVILNAGGWNLPVLVGLCEVENSWVLNAMLRETGLDNLHYRVIHYESPDLRGIDVALLYRRDRFKVYESRPIPVDFGPNERPSRDILYVKGVLDQSDTLHVLVNHWPSRFGGAAVTQWKRQYAARLTRQISDSIRMVNPQALLIIMGDFNEPHKSDLFIKDLEVGLLEDDAWLISPALKIPPGVGTLKHQHAWEIFDQIIVSRSFFDGSSPIYMSEPEMRIVSLPFLLERDEQMGGVKPFRTYVGFRYAGGYSDHLPVWIDLVVTPQ

SEQ ID NO: 134 - protein, 353 aa, Alkalitalea saponilacus
MFLPKNRCFSVVAILILLFGATHFGQAQQTRAGVIAFYNLENLYDTINDPNIRDDDFTPEGVKRWNSAKYWEKIDRLAEVISKLGSHENIPGPAIIGLCELENREVLVDLVQNERIRHLNYQIVHHYGPDRRGMDVALLYQPRYFRVTNSRSVPLEYYREDGSRLYTRDQLLVSGVFDGEPMHFIVNHYPSRWGGEERSRPLRVAAAQLSRALVDEIKDEDADAKVIVMGDFNDDPINESIKVHLNAHGNQRRLEEGQLYNPFEPLHRRGIGTLAYRGEWNLFDQILLTQSFLNKDQEGYRYHSVRVFNESFLARDEGRFRGYPFRSYVGNQYMGGYSDHFPVYIVLVRTLSQ

SEQ ID NO: 135 - protein, 472 aa, Alkalitalea saponilacus
MVKEHILNRISDIFKHNPTPSQKNAIDALASFMVSAKSMPLQLIKGYAGTGKTSLISSFVNVLGEIGIKCVLLAPTGRAAKVLSNSAGQPAFTIHKQIYRQKSSKDGFGGFLLGKNLLKDTVFIVDEASMIANNSSSGAVFGSGRLLDDLIQYVYEAENCRMVLIGDSAQLPPVGLDVSPALDAGELEAYGLDMNEVELTDVVRQTELSHILQNATYLRELLMNNLCDDYPKLEIVKGGDVKNITGAELQGEINHCYEQFGEEETLIVCRTNKRANQYNIGIRNSILFREDELSTGDYILVMKNNYHWVKEDDKVGFIANGDIARVVRIKKHYELYGYRFADVVCELVDYRAVEIDVRIILDSISSDGAGFSHEQQEKFLSTVMEDYADVSPGRKKFELARENDFYNALQIKFAYAMTCHKAQGGQWKAVFIDLGYFTEEYLGRELIRWLYTAVTRATERLYLVNFPKEFLK

SEQ ID NO: 136 - protein, 1030 aa, Alkalitalea saponilacus
MIPHKLTLQGLYSYISKQTIDFDNLTRDGLFGIFGSVGSGKSSVLEAISFALYGDTERLNRKDNRAYNMMNLRSDKLFLEFEFSNGENRRFLCRVEGKRNSKKFEDVGKLNRICYEKAENGEWIPIDTPVEEITGLSYDNFRRTVIIPQGKFQEFLQLGPKERTAMMQELFHLHRYDLYAGVAELHNKSVKVLDGLDGQLKTLGEIKPEQIEELTLQLEKMKVELANLENEQKGVQDKIAALKRIQELKAKLESAQELLVQLVDKEKEINEQEKELNLYEKSVRLFKSLMDDSHRLKNDVAGNEKSLKESLLEQEKLKKYFDEASVQFQKTKKEYEKRDVMKREADELKKFSEVLTLKQAIGELTKRRQKGEQMLAEKKSVQTDLRGKIQVASEQLIKDKEQLPDYAMLMDIKEWYRHREQLNKDAANLVKQQQELNEQSEDFKSKLQNHGRELSLPMPDGMEALAFCKELLKETELQAVRLEEQLKEMDQNRIRLKVQSELQGFAVDLKEGDACPLCGSEHHPDLLKPHNVHEELAALNHKSDDIQKKRQKTLALEKEILKIEAELLSFRKEKARNEKEVDEIKKETETHLKKFCWEGHHPESPDKLTQELQKHKTLTEVIKNGEKLLEELRTKLDEADKDLKKYEELLTALGHELTAKESRVETLLSDIKHINTDDFREVSAEALNNKSAELIKRADAIENRFKKEEEQINELSRKRNELIGKVSELQKAEVHLKDSLAKNEWKIEELLKQNNDLNREKLAVILASEPNVNKIRKDIEEYRSLLATKRAEVKQLEADLQGQQFDPIEWEKLINRNETLSEKFKKLIDESGQLKSDKKRLEADFLKFKELTKAREEAELRTADLSDMRNLFKGSGFVNYISTVYLQELCKAANDRFYKLTRQQLSLELGDDNMFYIRDFLNDGRVRSVKTLSGGQTFQAALSLALALADSIQKHTSEHGNFFFLDEGFGTLDKDSLRVVFDTLKSLRHENRIVGVISHVEEMQQEITTFLKVVNDEKTGSQVTASWEMS

SEQ ID NO: 137 - protein, 121 aa, Alkalitalea saponilacus
MKNLEHKGYTGSIEYSKEDDLLYGKVLGINGLISYEGKTGSELEADFKAAVDAYLSDCKEEGITPEKPFKGSFNVRISAELHQKAALLAMEDRMSLNNFVAESIRERVFRIFGKLSPRTSR

SEQ ID NO: 138 - protein, 120 aa, Alkalitalea saponilacus
MISKRAERPVYLVDVNLPRRFSFFNTSEFVHVIEIDATLKDREIWNYAIDHKLTILTKDTDFYEMYLTQPQHPKIVHFKIGNFTINTLHQYFTANWDFIKKLLETNEFIMAFKDNIKAIN

SEQ ID NO: 139 - protein, 224 aa, Alkalitalea saponilacus
MYFDIHTHNTVRREGVFSIVNMRAGYADFKEITAPVSFGVHPWDTTCHKSIQEIDKVTNVKGLIAIGECGLDKYKSGSLSKQTELFRKHVNYSEQLHKTLIIHCVGRYNEIIYLRKQIKPTQPWIIHGFNGHPQLAEQLISNGFILSFGSAIFIGNSKATKSLLLMRDEPFLLETDDSGFMIEEVYNQVAEIQGDEINHLKNKIATIFFKTFPGMETSGSQTTC

SEQ ID NO: 140 - protein, 485 aa, Alkalitalea saponilacus
MTHPLKSLKPDKLWEQFYNLTTIPRPSKKEEKVVEYVKNFGEKLGLETIVDEVGNVIIRKPATAGFEDRKGVILQSHLDMVPQKNSDNNHNFETDPIETYIENGWVKARGTTLGADNGIGVAAILAVLASDDLQHGPVEGLFTIDEEAGMTGAHRLKPGLLNGEILLNLDSEDEGELYVGCAGGTNANMIFSFREEPVPDDHVAFRISLTGLKGGHSGLDINRGRANANKLLFRFIKHAVIHLGARLADVDGGSLRNAIPREAFAVLTVPKEEVVEFVEEVHNFEVQFCQEYNTSEPDILFKIEETDIPAFVIEEIVQDDLINAIQACPNGVIRMSADMEGLVETSLNLAIVKTEGHEVKALALLRSSVESTKEDLESSLESLFRLAGAEIWFDGHYPGWKPNLQSGILKTMQEVYNQKWGVTPEIKAIHAGLECGILGSAYPHWDMISFGPTIRFPHSPDEKVDIASVEKFWEYLAAMLKEAGK

SEQ ID NO: 141 - protein, 408 aa, Alkalitalea saponilacus
MLLFSHTLPNGIRLIHHPVDSPVGHCGLIINTGSRDEKEDEHGMAHFIEHVLFKGTKKRKTYHILSRIDDVGGELNAYTTKEETCIYASFLKQDFNRAMELIHDIAFNSTFPVKEIEKEKEVIIDEINSYKDSPADLILDDFEELVFSKDAIGRNILGTPETISKFGQKDIRKFMAENYHTDQMVICSVGQIPPGKIMKIASRYFGSITPNYRQLKRQPNSPYLPQTVEKTMDTFQSHVAIGNVAYDLNHPNRLSLLLLNNILGGPGMNSRLNMSLREKNGIAYNIESIYTPYFGTGVFSIYFGTDEENLKRSIKIVHKELKKLREKKLGKLQIHNARRQLKGQITIANENREHLMLSIGKSFMLYNKVDTIEEIYNKLDNITAEKLLETANEIFAPEQLSYLIYRQS

SEQ ID NO: 142 - protein, 1261 aa, Alkalitalea saponilacus
MQRIVFFSVLFLFAISSLYAHKHGLEVSKQIVWGEYTINETLPFEGDGHWEDGGVPVYRFRVALPNETDPSSINVQIQDLQLLPGDSEFSHLADYRNVLPELRSLVVSIRMNTYLEIEIIPFHLADNEILRVSGFTALIEFQTSSVEALKSADLKASTSLFKSNSVLSSGFWQKISVSETGIYRIPYSTLTSWGFSNPQNVAIYGYGGQMVPRINANARPDDLPEVGIMHHNNAIYFYAHGPVTWSWDYNKQMFTHQLHYWSNFAFYFLTEKDSPPKSVPLMDVETRTPTHTITTFDERKYHELENHNILKSGRKWFGEKFEGNGVRSRTVSFDFQGRDVSAPVKMNINVVGRSPNMHSFRVSVNNSSALLNLSIPPVSIFSSDGPFAHEASGLIEIQDDQEKLDVKIEFNETHNRAEGYLDYITFNARSALSMQGGQLHFRDKQSSGTDRVLRFRIQNGNSNHVVWDVTDIISPQKMQSQLFGGNLEFVADAEIYREYVAFDPSGQFPVPNRVGLVPNQNLHALQQTDYVIVVADEFETFAHQLAALHQQHNDLDPVVVPVSQVYNEFSWGHQDPTAIRSLMRMLFHRANGDQTIAPKYLLLFGNGSYDNRSKTAGLERGIVTYQSANSTHQTNTYVTDDYFGFLGQNEGADDRFDRLDIGIGRFPVNNEADAQVAVSKVRRYFEEQDPGEWRKLVTFLADDGDFNIHQRDADFLAERVLRNHAEFDVRKIYLDNYPHTSSSAGRRVPEAEDLVNRTISEGTILFNFVGHGGPGGLTEERVITTASINNWTNIRRLPLFVTATCEFGRFDDHSSVSAGERVFLNSSGGGIGLLTTTRVVFSSLNFQLNNSFFNYVFYRNNDGSKPAFGDIIRNTKNGAGSSVNKLNFTLLGDPALKLIYPEHSVNTIAINGRSIDAIPDTIQALSKVQLEGMVTDKHGNFMETFSGEVNVVVFDKPLEVRTLGNAGATPFEFKSFSSILFRGKATVENGIFDIEFVVPFDIRYNYGFGKISYYARSDQYGTAFGAYENIVVGGFNVDAPEDNDGPQVNMYLNHAGFRSGDVTNSRPMLYAEIFDESGINTSGAGIGHDIVLIINGNRNEPIVLNSYFQAKPDTYQEGTIVYQLPELEPGKHEISLRVWDTYNNSTTEVLEFTVGRGKDLTIRDFKWYPNPASGNTTGYFSFGLDEPNSRLNINVDVISSDGRTIGKYRVDVVAEGNYVSPVPVALGSLGIRNPGLYYIRFHISTSGGKESQIVEKILVKP

SEQ ID NO: 143 - protein, 942 aa, Alkalitalea saponilacus
MRRISKNLLFVLGFFFAFSSISAQNLAEIPVPLDPMVRTGTLQNGLTYYIRYNEEPKDRASFYIVQNVGALLEEDHQNGLAHFLEHMAFNGTENFEGKGILNTLERHGVAFGRNINAYTSFNETVYNISDVPVNRPGILDTCLLILYDWSNGLLLTDEEIELERGVILEEWRTRRNSNIRMRDQWFPVLFEGSMYAVRDIIGDTTVIKYHDPEVLRQFYHDWYRTDLQAIIMVGQFDVDEMEEKVIELFSEIPAVENALERPFFEIPKREGTAFVVATDREATQTSITIYIPRRNRDMQKKTLEDLRSGYIRSLYNSMTSARIQELLQQGTPPFINGYTQAGGFMRGYDSYVIGVTANPGEAEKAVEAIMVETERVLRYGFTENELARAKSNILTNLESRYNDRGKIRNDVFARQLQNHYLINAVVPGIEFEYEFANQVIPGITVEEVSAIAREWIREDNRTIVVTGPDNIEHIAETSAFSIMDGVKLAEISPYEDRLLAESLIEKELPGSSIEQTVILEDFDAVEWTLSNGVRVVFRHADYEKDNVLLSAYSPGGSSVKGNDFVPSITLFNELITSYGVGDFDAVSLQQMLSGKRVSVRPMVYDFSETISGNAAPRDFETMMQLVYLYFEQPRFDEEAHNALMSRYVSFVANMQNEPRKIMSDSITLLLSDFHPRVRNLDVSLINEVCFEQIRAIYQDRIHDASDFVFFIVGNMDEEVVRLMSKQYLGSLTGTGREETWVDHGVRFPQGQQKKQIEIPLEIPKANVNVFYSREMDYAPENLMFMRVLRGILNLRYIETIREDEGGTYGVSVGWTMNRKPVQTGGIQMRFETDPERVDHLKPILYREIEKIIAEGPTQDDFQKTIENILKDREQARRHNSFWLNSLYNFYREGVNHADEENFEEIARNMTLEDIHQFVIEFFNEADLMDILFLPQAEIVSAN

SEQ ID NO: 144 - protein, 413 aa, Alkalitalea saponilacus
MIEIYKHQLANGLKIVVHPDITTPLVAVNLLYDVGARDEAPDKTGFAHLFEHLMFGGSVNVPSYDEPLQRVGGENNAWTSNDFTNYYVTLPAANIETAFWLESDRMLELNFTDKNLEVQRKVVIEEFKQRYLNQPYGDIPLLTRPMAYKQHPYQWPTIGKDISHIENATMDDVKNFFYRHYAPNNAVLSVSGNVQPDSVFKLAEKWFGDIPRRDVPVRNIPAELPQQEARFLQVKRDVPAHLLNIHFHIGARRDDDFCINDLLSDILSNGPSSRLIQSLIKDKQLFSDVNAYISGDMDPGLFAVTGRLMPGIKMKDAEDAVWNELHSITNTLVDDRELQKVKNKIESNLVFAEISFLNKAMNMAQYELMGDAENINREIEHYRAVTAEQIQATAGSVFRKENSSTLHYLAEKG

SEQ ID NO: 145 - protein, 428 aa, Alkalitalea saponilacus
MHIKPDRSKGPAFETINQIGFLPVAGLSLPNGIEVSMITAGSQDVTKIDWMFPAGAVQAGKPLLASTVGNLLMEGTTSRTSQEISGMLDFYGAYLSTQTFYHNTVVTLICLTKELPDMLPLVEDIIKNPAFDKRETDIYINKRRQEYILDSEKVKTIAARRFPEVVFGANHPYGKTLKLSHFDELTRDELFEFHKNAYTPLGCRIIVSGQPGNEIGDLLVKYFGSSQWLPGTVNLNGVGEIEPLGQKVHLIEKEGALQSALRIGRPLFNNNHPDFIPLQIVNTILGGYFGSRLMTSVREEKGLTYGIGSNIVAYKNGGMWVIGSEVMGEMRQAAVGAIIDEMVRLTKEPVPENELEVVKNYMLGELMRNFDGPFSTSDIFRSLWEYDLDFTFYAKMVEEITKIDQQRIMQLSEKYLNPDDFYVVVAGK

SEQ ID NO: 146 - protein, 264 aa, Alkalitalea saponilacus
MKRNRFFVTLLTVVLLSSCNDGKVNFFTLNQDVEFGQQVVAEILANPQEYNVLPRQGNEEAYAYLEGIRDKILASKDIRYRDRFQWDIYIIDQDVLNAFALPGGPTFYYTGLMKYLDDEASLAGVMGHEIAHVDRRHATNRMTKMYGFSILFSVLRGDNESLLGDIAESLATGVTALAFSRQDEFEADEYAVRYLYPTELDSRGVAYFFEKMDLAKQSRVVTYLSTHPDPGDRISEIHRHHQRLGGKEGNPFTKRYQEFLQLLP

SEQ ID NO: 147 - protein, 472 aa, Alkalitalea saponilacus
MRWIIALPILFSCLCSSFAASNSKVPAPPNFPGASVGISVIDLSSGLEVTGVNQDKLLTPASVLKLSTTAKALDKLSPEYRFSTSFFYSGEIKNGILYGNLVIRGGGDGTLGSFYFDSTQPDNTLQYFAEQLKKNGIHTINGKLIIDQTLFPEPRYPAGRLWEDMANYYGAVPSGLSWRDNTFHLTLRSSASSGEKCQIVSVTPPLDDISFISHVYSATHNRDSAYIFGYPGLSQWEVRGSIPTSRTDFTIRGALPNSGKTFAHELAKHIGYNIDNNIIDIQDNINYEDLHLLFTHLSPPLEEIIQIVNQRSHNLLADHLFLLNGLNAPKHHSLWDLATWNTIKYWKNAGIDMPLRFHDGSGLSPKNLASPRFFTDLLAHVNQTQYQSVFEKSLSVSGQSGSLRRMWSTNNRRGRVLAKSGSMQGVLGYSGYIYTTSGRKLAFCIIVNNYTQSFLEIRNSIEEYINFFIDHY

SEQ ID NO: 148 - protein, 433 aa, Alkalitalea saponilacus
MDRAHKLANELIDFIYDGASPFHVVESMAMQLDQAGFEFLDSTAEWELKKGGKYYITPNGSSLFAFVAGTGNPAETGFRIVSAHSDSPTFRIKPTPEMGVDNYYIKLNTEVYGGPILMSWLDRPLSIAGRVSLKSDSSLWPENRLVNFNRPLVIIPSVAIHLNRSVNDGVAINKQKEMLPLLGILPDNDAKEGLLTRLIAQELGIDSGEILDFDLTLNEYNKGCIMGMHNEFISSPKLDNLAMTHAGFKAFLNSKPSEATQMLCIFDNEEVGSLTKQGAGSPVFRHLFERIMHQFGKSKEDFYRAVYKSFMISADMAHSIHPNYEEKHDPVLHPLMNKGPVIKITANQKYTSDGDSIAVFESICQKAGVPCQKFLNRSDMAGGSTLGNVSTGQLDIRSVDIGNAMLGMHSVRELAGVTDHEYLIRVMQTFYEL

SEQ ID NO: 149 - protein, 417 aa, Alkalitalea saponilacus
MHPLLYIIFAIIIFEALWDFFLGELNRKSWSDKVPKRLEDVYPQDKFQKQKEYRIANYRFGLFSSAVSTILILMVLWYQGFGWLHYTVENFIGHKYLQPLVYFGAIGLGSMILSLPFSIYSTFVIEERFGFNRTTKSTFITDLIKSLLLGALIGGLLLWLVVWFYHTAGSLFWLYAWGGLSLFMIFFSKFYTTLILPLFNKLTPLEEGELKSAIESMSRKAGFSLENVYVMDGSKRSTKANAFFSGFGENKRIVLFDTLINDLDKDEIVAVLAHEIGHYRLKHTIRGTILGILQTGITLFLLGWFINHPGISQALGVASPVFHVALLGFGLLYSPISAMAGLGMTILSRRQEYQADAFAAKYANASALQSALKKISATALNNPTPHPWFVFFNYSHPPLLKRLEALDSFTSVKPTIK

SEQ ID NO: 150 - protein, 451 aa, Alkalitalea saponilacus
MIKKILLILLIITSIPLTGGELVTVVVTNNASSDGSVFVAQFNLQNSIDIEEHIFFKRKQTSPNSVKEIFSSQTGGKIGEIPEKNGTLQILANTNEHQLTIIGHRFSAKEELRNQKGMLDGENLKRIALQRSTSAHDAINTIAALAEKHGYNGNGYRFFIADPSEVWMMEMTGKGAMNRGAVWVARLIPDGRMAVHGIEPSIGSFPISSRNNDVLYSQDVISFAREMGFFDGRNRDFNFKNAYTDPQSNDENSGIVRETAGLFNASIHQRSDSVSLPLFFQPSQKVSLRSVKELTKKLHHGEETDSVNTDKTVSTFIVQLRNWLPRPIGGVVWLWVGGDSIGNFQPFYIGIDEFPPSFREKHDIIGEINRICANRTDSAILDECMRIRHELEEKYLRFAPAVEQTARALFVSNPALAVEYLTDYCFSQSLIAKRRWREYLEELQNMENINH

SEQ ID NO: 151 - protein, 890 aa, Alkalitalea saponilacus
MRPNNYLLKNLLLTMALLAIALSTSAQSRQRPAEANLNNQLMQLSSPAEDLLETDENIDIRFYHLHIDVDIENEKIYGDVYIELTAVNNLNQVVLNLHSDFEITSVGEDATSWTLENNLLTLGLNSSFNVGETVKLRIVYNGNPPLAPGRFINKGFRFDRHSNQTVPAIANYSTPYLSHYWFPCKDGPTDKADRVWVDITIPDESYNGQPLMAVSNGVLLNDNPPVENGKRTFQWRHEHPIVPYYILVAVSNYVLIEDQYENTVNGNSFPLEFYAYPQDIVDANSAMVKMHDIMDAFIHYFGDYPFADEKFGMTQVPLSWAIENQTNPIIGGFGENWADIIVHETSHMWFGASITNQTWQHVWLNEGFATYAEALYKEFSSDFNIEEYHTRMRAMEKRFNDFPNLYLSDDSNYDYIFEEIYYEKGAWLLHMLRGQLGDELFFDCIKSYAQNPNFRFGHATTEDFRDHCQAISGKDLTTFFQQWVYDFAFPIYSYDYLTDDVSGETTFTLFQRQNAIWGDREVFEMEVDIKFNFDDGTSVIERVVNNAVEQQFTFNFGKAIQQIEIDPDEWIIREIRSHKKEILAFNVPEQISSEINQEEQTITITVPFGTDLSQITPTIELSEKASVAPESGTPVDFSEGNVVFTVRAEDRTTKEYTVIIEMAPNSENRILSFAIEGQIEETVINDETFEIFVTMPYGADLSDLSPDIQISEEATVNPQSGSSVDFSEGSVIFTVTAQNEDTQEYSVTVNTSSENDLRIISFTITDQLDETLIDHEESTIHVTMPTGYDLTDLAPVISLAGNTTVDPESEVSVDFSTGPVEYTVKTQDESEQKVYTVTVENLLRDGDLIIEFSVPDQIGETSIDDEENTILVIMPTGADITEITPEITIS

SEQ ID NO: 152 - protein, 1298 aa, Alkalitalea saponilacus
MITSNKLLLILATVALFYVAANVEAQKRQRPSLPDTDLSEKQKARKEFIQQEWEAYMALKSASETLQTDENIDVTFYHLTIDVNTTAQSISGNTYIELKSTVNNLTQVKLNLHTSMTVTAVGENAISWSRSGSNVLNLNLDQSYNIGETVNLRIYYNGTPIIPAGTGKGFRFLTHSSTVPAVTALSTPYLAHYWFPCKDGPYDKADSVKVDIIVPDVSYQGYPLMGVSNGMLYDTIIDGGKRTYRWKHNYPIVPYYVSVSVSNYRVFGEQYNRNGHDFPLTYYVFPNDYNTALSTFSGVPDVFDAFIHYFGDYPFKTEKYGMTQIASGLTYIEKQTNSIMASVAPSAWWLVVHELAHMWFGNSITNRPWNHVWLNEGFATYAEALHEEYYFGKAAYHQYMNNTLTSGWDYTRTLYLSDDSNPTQIFHFFYYDKGAWVLHMLRNHLGDDLFFEILKSYAQDPEFKYLYVNTETFREYIESKSGMDLEVFFDQWVYGTSFPDISFNYSYDPSTGKNGVTISQIQSWWTYDRYIYEMYLPLRFTLSDGSVVEEKVFNNQRIQSFHFDHGLSVTNMQLDPDQWNMIWWSGRNTSLAVPPAPMITSFNIPGQVNNTVINELTRTILITMPAETSLTTLSPAIGLTANTTVSPTSGVPNDFSSPVKYTVTGINHSQRIYTVYVSTVPSDEKLITSFTIPNYISSEIDHDEETILVIMPPGTDITNLVPGITVSVNAEVSPASGIAQDFTSPVPYTVTAENQTQKSYTVTVELDITPDVTNIWNGNISTDWNHPGNWSHGVPQEQMSVHIGAYMTRFPTISSNVTIKNLTVDAGATLMQVSGTLTIQGEFRLKSSSEVNASYIMTGGSIDIEPEKVIIEQVISNPGYNYAISSPVSGSLATRLNSGITGTTYIYNNPTNTYLQLDENEPFEPGTGMVFRNNDHIQFSGVINTGSVIVPLTRTSAGLGWNFIGNPYTAAVDWRSLNKTNVDDLFWIYRNDLGTYGTFNNNTGLAVGLNDPPYLIPSGHAIWVRVTLGQAEGAVTFSPNAMVHNPFSYLKAKKPHDYSFIKLISRYNGHSDEAAIAFVPESTKGASDPYDSDKLFGNNRKTAEIYTLSQGRPLAINALPQEESMTIPLGVFVRRSGVLGMQLSDHDLTDNTVVLLRDKLTGEITDLTSGQRYRTYLRITEEHYMEKVKEEDKPTRIDDRFELIITKSTPTGFKEELNSELQNPSNDDVHVYNSVNGIIVYAETKSSPFYLLYDSTGRRISTETLQPYEENNINLPQRGIYIISIIWEDNVKNRKIIF

SEQ ID NO: 153 - protein, 714 aa, Alkalitalea saponilacus
MTFFTHKVQNLLPLILLLFLTGLEAQQRSDITSKETTSQVTAPLSTQDAAQLLQTDFNIDVQFYHISIDIDIENETIDGSVVVDFKPLINNLNQIKLNLRNVFTVTNITMDGAPVTWSHSNHILNVNLNQTYSIGDEPSVKIYYNGAPERVQSGGVTKGFRFDTHGNNVPAIVNLSTPYLSHYWFPCKDGPTDKADNGIRLDITVPNTTYGDRKLKAVSNGMLINEVVNNGKRTYTWQHNHAIAPYYILVAVSNYQTIERTYNNNGHNFPIKYYTFPANSNQATSIANMFNQAFDAYIHYFGDYPYRDEGYAMTEIVPFWYIEKQTNSVVANWNWTILMPHELAHMWFGNSITNQTWQHIWLNEGFATYAEALYYEYTSGMGAYHNHMRSMGARHIWDRVLFNEDDSRHWEIFDYFYYEKGAWLLHMLRGYIGDDEIFFDLIKAYAQDPQFKHGYVTTDEFRQYVEAFTGLDLYNFFDQWVYDMSFADYEYNFYSDLAQGKAGLTINQSQSEGTSNEREVFEMNLDLRIEFADGSSRKERVYNNQKLQHFYFDIDKEVIDIIIDPDEWVIRFDVVFNSSLPVPPAPIAENRILSFSVEEQIGEAQINHTTGTIQFAVSDNENINALTPQIEVSPGAIVSPASGATQDFSSPIVYTVTGSDNSVKEYTVTVVTLSGDSQITSFTIEDQIGETVIDNGNISITMPFGTDLTSLTPV

SEQ ID NO: 154 - protein, 546 aa, Alkalitalea saponilacus
MKYNNNLKQIILPAVLAFVLILGFFIGRIWTPSTSSTGSNRLFIYPQSNKLEALINLIEQEYVDTINKAELIEKVIPEILKNLDPHTVYIPKEDLQAANEELDGNFGGIGVQFSMQNDTVLVISVISGGPSEKLGIIPGDRIITVNDSVIAGVSMNTDNVVRLLRGEMGTKVNVGIKRQGREELLDFEITRGMIPIYSVDVSYMITDSIGYIKISRFGRNTYQEMLTAMARLKAHNCQSVIIDLRGNSGGYLDVAISIINEFLSKGDLIVYTEGKNNPRQNIYANGAGSCQDVGVTILIDEFSASASEIMAGAIQDNDRGLVVGRRSFGKGLVQQQIPLPDRSAIRLTVARYYTPSGRGIQKPYENGVEDYHRDILARFEHGEFFERDSIVMDESLEFFTRGGRIIFGGGGVMPDVFVPRDTTQLTEYYFRLHDRGIIYQYALNYTDNNRLQLQRFENAESLVAHLSNQDLLSGLVEFARGRGVQFNQAQFRRSSERLEVELHAYIARNVFDNEGFYPVSHKIDEVVRAALYHIRNGYDREVLSLN

SEQ ID NO: 155 - protein, 571 aa, Alkalitalea saponilacus
MNKKRGLTKRGWFITILLSVIISVGFIAANTDRRNFEIVKNLDIFYTLFRELNSFYVDEINPDDLIKTSIDGMLESLDPYTTFIPESEMDDFRFMTTGEYAGIGALITRRGNFVVVSEPYEGFPAQEAGLRAGDRILKIDGDDMKGKQTSDVSDRLKGPAGTEVIVLVERPGKSSPITITITRRSIQINPVPYYGMLDDKTGIIILNNFTQNCSQEVEKALKELKKNENMSRLILDLRGNPGGLMDEAVKIANLFLPRGSEVVSTKGRVSQWDKTYRAPRQPIDTVMPLAVLINRGSASASEIVAGALQDHDRALVIGQRSFGKGLVQTTRSLAYNSSLKVTTARYYIPSGRSIQAVDYANRNEDGSVGFIPDSLMREFSTSGGRTVFDGGGISPDVIVERDRFSSISMALIGQQTVFDYATLFAVKTPSIEKPGVFQISDDIYADFISYVTGLEDFRYESQSQNQFRKLKETAEREGYFDVNKELFSAMEENLRPDVARDLGTFREEVEEFLAMELLRRFYYQRGAIIHNLKTDNEVAKAREILSNPAKYNDMLNGTILTHAGDKRGARN

SEQ ID NO: 156 - protein, 525 aa, Alkalitalea saponilacus
MKFRLLFIFLLPLTLLTAQRNDPAFNNIQIAWQLITNFYVDTVDSDALAREAIESMLRKLDPHSVLIPADEVKAMNEPLDGNFEGVGIEFSIMNDTLVVITPIVGGPSEEVGIRSGDRIVAIDGENVASIGLQNSDVFSMLRGQKGTRVTVSIYRKGTPGLLDFTVTRDRIPIYSLDASYMATPETGYIKLSRFAATTHEEFTKALRELKQQGMQNLILDLRGNGGGYLKAALDIADEFLDANKMLLYTEGNSVPRREHNSSRGGLWRKGELLIMIDEGSASASEIVAGAVQDWDRGVVIGRRSFGKGLVQRPFSLPDGSEIRLTIANYYTPSGRSIQKPFNNGVKEYRSEIGLRHLNGELTNGDSIQFEGEEVYRTLVSGRVVYGGGGIIPDLFVPLDTTMYSDYYRRIVASGTLNRVTMEYMDNNRRRFNDKFPDFHKFNETFVIPDELISKLIEEGENAGISHDSKGMDVSGELIKTQMKALIARDLWGTSEYYRVLNPLISVYHKAIQLIENRDLFVELLN

SEQ ID NO: 157 - protein, 442 aa, Alkalitalea saponilacus
MKQTKKLLLFFLGLFIAMFPVDAQSGRIEFSEFTLGNGLHVVLHQDNATPIVTVAVMYDVGSKHERPDRTGFAHFFEHLMFEGTKHIPRGEYARFVEMAGGTLNANTSADRTYYYQTLPSNQLELGLWLESERMLHASVDSVGIQTQKQVVIEERKQMYDNRPYGTILIETMARAFTKHPYQWTTIGEPEHIMAAEDHEFQEFYEMFYVPNNAVLVIAGDIVKEDTRALIEKYFGDIPTRTEEIYRPNIIEPPLKAEVRDTIFDNVQIPLVLQAYRTPALNTEDYFAIDMLGTLLSTGQSSRFFRELVDNQELALQVGTFPLPYNEPTVTLTYAFANMGIEPHVLEEAMNAEIEKVRNELIPEEEFQKLRNQFENDIIGGNSRIAERAHNLATYHTYFGDASLINKELEKYMAVTREDIQRVARKYFRTDNRVVLYYLPKRQ

SEQ ID NO: 158 - protein, 685 aa, Alkalitalea saponilacus
MKKIILSILTICFTTGLLAQLDRSTPPSAGPAPQINIGEYKKFKLSNGLQVFVVEDNRLPFVAYSLNLEIDPILEGEAVGYVSMAGSLMRSGTTNRTKGEIDEAIDFIGATFNTFSDGMYARSLKKHSEELLEIMSDVVMNPSFQQEELDRSILRMRSALQANKSDAGSIAANVANVLRFGKNDPYGELVSEETLENITVDLLKDYHKTYFRPNVGYLVIVGDISLKEAKKQAKKHFGKWKKGDVPTHQYNDPAKYEQPKVAIANREGAKQSTINVTHTVNLTPGHPDAIKASLMNQILGGGSFNARLFQNLREDKAFTYGAYSRLSNDKRIGHFTASTEVRTSVTDSAVYEILHEMTRMRTELVSEEELDLMKNVLTGSFSRSLEDPQTVARFALNIERYNLPADYYRTYLEKVAAVTPQDIKAMANKYLHPDHVIILAVGEADKIRESLSKFSPTGEVVQYDFYGNVVTGPREVTDVNAVEVIERYLEAIGGHDAVNAVEDVKMHASFTIQGMQLNMITQQKAPNKLLVETLMGGNVVTKQVFDGVNGLIVSPMGEQRLEGEMLEEMKKASALFAEHALLKPDAEIELVGVENVEGMEAFRINVLSNGESTKSLYYCVESGLKLREVSTGMQGTVISVFMDYKEVNGVKFPSAMRQSAGPQTFDITIDSIEVNTGIDDEVFAL

SEQ ID NO: 159 - protein, 713 aa, Alkalitalea saponilacus
MKRKLVICVTLLALTIAGTSCRQKSSPGLTYPVTQKGDVVDTYFGHEVPDPFRWLEDDHAPETKEWVKAQNKVTNAWLQQIPFREDIKNRLTEVWSYTRQFSPWKRGENIFYYRHDGIRNHAVLYVKEKNGEEKVLIDPNLFSEDGTTSLAMASVSKDGKYVAYGISKGGSDWREVFVREVATGKDLDTHLKWIKFSGLSWDENGFYYSRYDEPAPGDELSASNEFQKVFYHKLGTSQDQDLLIHQDNDNPQMNFSAQVDDDNKYLMLYSRISTQGNNLFIRDLNRGGNWIVADTDFETQSSYVGTIGNEILVLTNYDAPRYRLMAIHPNRPNVENWREIIPESGNVLRSVTTSDNYIIAHYMVDVQSRLSLYSKAGRYIRDIKLPGSGSASGLSTFSEEDVLYFTFASFTTPESVYRKDLKSTNPPVAHFVPNVDFKSEEYTVNQVFVEAEDGAEIPLFIVHKKDIELDGSNPALLYGYGGFNVVQSPRFDARIVPWLENGGIYIHAHIRGGGEYGEGWYRAGIKKNKQRVFDDFILAAEFLVESGYTSPEKLAIMGGSNGGLLVGAVANQRPDLFAVALPAVGVMDMLRYQYFTIGWAWAGDYGRSDDSEEMFKYLYAYSPIHNIPKGKLFPATLVTTADHDDRVVPAHSFKYIATLQDRYSGPNPVLIRIETLAGHGAGKPLSMQIEEVADRLAFTLFSMNETWNSEKNK

SEQ ID NO: 160 - protein, 202 aa, Alkalitalea saponilacus
MKLKKCFLSVISAAILFFAGCKTAEERVVVLEKEDVKRVAVLVGEGFHDGEAYMPMGFLANRGIKVTVIGPERGEVKAYNSDFTIKIEKAVSEVSVDDFDALILPGGHAPSVLRDIDEVVAFARDFYKSGKPTAAICHGPQILITAGVMEGKSCTAVGSVEDELVAAGANFLDQSVVVDGNLITSRVPRDLNDFSRAIYDAL

SEQ ID NO: 161 - protein, 586 aa, Alkalitalea saponilacus
MNKFFKYFLAVVLGSMVSAFFFIVGIVMFITILASTASKDVTVKDDSILVLDLNGPVVERTTSDPFEMMLSQLSGQKSPKGLNQILASIKKAKEDDRIRGIYMEAGMISTGYASIEEIRNALIDFRESGKFVHSYAPIYSQRAYYLASAADRVYLNPTGMLEFKGLSSAYTFFKGTLEKLGVEMQVFKHGEFKSAVEPFILESMSDEARLQTETYLNSMWGHITSQIAQSRNLDVESVRATAELFPTFREDTLLISSGLIDGFKYKDEVLSELKKLTGIEEEKDLNAIGVMKYADVYLPGKRKGLEKNKIAVVYAIGEIDGTSGGINSEKLSRTIRQARRDSTIKAIVLRINSPGGSGLGSEIIWREVKLAQEVKPVVVSMGDLAASGGYYIACAADTIIAHPTTLTGSIGVFGLIPNTQELLRKMGITTDRVKTNTFADMPSLDRPFTREEKELMQAYIERFYNVFLQRCADGRDTTTDAINIVGEGRVWSGENALGLDLVDKLGGVSDAVAVAARMAEIETYRVVELPEVLSPIEQIMKGLGGDARARVGRIFFGEEYQIFQTIQDLKTAYPVQARIPYEISVN

SEQ ID NO: 162 - protein, 680 aa, Alkalitalea saponilacus
MNFKPLITAKLIILIMLSAFISSCSNAPQKPALDPANMDMTINPGDDFYRFVNNGWLENNPLPDDYSRYGAFEQLNEENEQKLYDLLMAIRSDKSAAHGSNRQKIRDFYNSAMDTASIEEQGITPLQPILDRIEAIDSKEKLQTVIAELHQTGIRPLFGMGASQDRKNTDWMIASVGQGGLGMSDRDYYLKDDARSKEIREGYKNFIAHMFSLAGYEDTEAKKAVEAIMQIETSLAEVSMDRLTLRNPYATYHIMTLDELSDKSPNFNWASYFNSRNVSIEDLNVAQPEFFKAVSDLMNSVELEKWKTYLKWNVLNSSASFLSSDFDKANFAFYGTVMTGSEVQRERWKRVLGVLNGSLSEAVGQEYVALYFPPEAKERMIDLVEHLRTAFHQRIGNLDWMSAETKEEAYGKLAAMNVKIGYPDKWIDYSDLEIKDQPYILNVLAARAFNIKRNLDEIGQQVDRDKWFMSPQTVNAYYSATMNEIVFPAAILQPPFFYLHADDAMNYGAIGMVIGHEMTHGFDDQGRQFAKDGNLRDWWTEEDSRRFDELSQVLVNQYNNYVMLDSLTINGKLSLGENIADLGGLSIAYQALQNKLEEDGRPEEIDGFTPEQRFFLSYAQVWRNHMREQRLRQQLNEGPHSPGEARVNGIVYNMEEFYKAFNLDDSGERFIAPDDRANIW

SEQ ID NO: 163 - protein, 418 aa, Alkalitalea saponilacus
MTRKDFEVMAPAGSFESLKAAIQGGADSVYFGAGNLNMRSRSSSNFSAGDLKEIASICKENGLKSYLTLNIVLYDEDLEEMRKMVDVAKESGISAVIVSDQAAIHYASQKGIPIHISTQVNISNIETLRFYSKYADVVVLARELNMDQVKKIHEAIVEEDIRGPGGDLVRIEMFAHGALCMAVSGKCYLSLHQYNYSANRGACLQSCRRGYVVTDKESGDELEVDNQYIMSPKDLKTIHFLNKLVDSGVRIFKIEGRARGPEYVKSVSACYNEALEAIAGGYFTSEFIAGWDERLSSVFNRGFWDGYYQGQKLGEWSANYGSMATKRKIYVGKGTNYFPKIGVGEFRLETQSLNVDDEILITGPTTGVLEMKVKELRVDLKPVNEVKKGDLFSMPVDDKIRRSDKLFKIVKASQAKIQ

SEQ ID NO: 164 - protein, 618 aa, Alkalitalea saponilacus
MLQEKGRVTSLELLAPARDLECGLAAINHGADAVYTGAPKFGARAAAGNSLTDIATLTEYAHLFNAKVYVAINTLLYDHELTEAEKLIHQLYKIGVDAIIIQDMGITQMNLPPIAVHASTQTDNRTPEKVKFLEDAGFDQVVLARELTLNEIAEIRNITNVPLEFFIHGALCVSYSGQCYMSQATSGRSANRGECSQPCRLPYSLENLDGKTLIKNQHLLSLKDLSNTNHLHDLIKAGISSFKIEGRLKDATYVKNVTSWYRQQLDRIIETDSNLARSSSGRVTIPFEPSPAKTFSRGFTTYFLNGREKDIWSLHTPKSLGEKLGRVVTISRDYFIAEDGIDLNNGDGICFLNKSKQLRGFRINKTVENKVYADDIKELYTGAMLYRNHDQLFEKQLINSKENRRIAIDLNLSETEDGISLQLIDEDGLSSEIRKNIIKEPAKNPDLALKTIGDQLSKWGNTIYNPNSIKLQLLQPIFIPAAEINAVRRELNDVHKTKRLNSYRRQEKLFPQTSHPYPNAVKDFSLNVSNHLAQKFYNIHGVKKTEPAFEIKSPTGARLMTTRHCIRYATNSCPKENPKATPENLILKSGKNSYELKFDCKKCEMMIFDLDSNQIKNT

SEQ ID NO: 165 - protein, 257 aa, Alkalitalea saponilacus
MRGSISPYSVLSVRREPSEKSELETQLLFGEVFYVDEIMNGWVKIKTEFDGYEGWIDERMYYPVRDKEIELWLSAPGVIIPTPMFKLIREPEKSAQLISAGSRIVFNGEDRNSFVIGHKEFYCQSTVPDRTPDLEEIAKGFLNTSYLWGGRNIFGIDCSGLSQVVFKIMGKRLPRNASQQIEHGAMVSFVEEARAGDLAFFDNPEGEITHVGICLGQGRILHASGEVRLDHLDHQGIFNRELQKYTHHLRVIKRMME

SEQ ID NO: 166 - protein, 592 aa, Alkalitalea saponilacus
MYTSDKLLLIRSKMEIQGIQACIIPYGDQHLSEYPAEHWKTRDWISNFTGSAGTLVITAHEAGLWTDSRYFLQAENQLDTSCVQLFKEGMPDVPEYAEWLTHVLEPGDKVGINGVLFSVSQVRKLVKTLRDHRIQSDLKFTLAEECWDTRPPIPEDSVFEHDDKFCGQTRAAKLEAIRKYMRKQKISHYIVSMLDEVAWVLNLRGTDVPYNPVFHSFLIIEHDQVRFFIDPHKLTAGIARKLDADNIKVSLYDDFYQHVQDITSEARFLIDPDRTNYTIFATMSQAAQKIEERSIVSILKARKTNKEIENFRTTLINDGVAMVQFLKWLEDHVGSGSITELSAAKQLKSFRAKLPGFSGESFSTISGYKGHGAIVHYSVNRESDITLQPEGLFLIDSGGQYPGGTTDITRTVALGDFPEQAAVDYTLVLQGHIALATAIFPNGTRGVHLDPLARKAMWKFGINYGHGTGHGIGYFLNVHEGPQSIRPQDNGVELEPGMITSNEPGIYRTGEYGIRIENLILCKEKIETEFGLFMEFETLSLCPIDTKMVKKELLSSDETEWLNSYHKMVYDKLAPMLDEEHKTWLKNKTTAI

SEQ ID NO: 167 - protein, 550 aa, Alkalitalea saponilacus
MQRKNKFQFIKYLPGVILMALMACATPEYTIEPFGENIETDINILASDEFEGRAPASPGGIKARDFIKSRFQEIGLKPANGDSYLQAVPLVEVTGSDFTTLNIKGNGAELSFNYLDDMVVGSYRLEESLQLDKSELVFVGYGVVAPEYGWNDYEGLDVEGKTVVILVNDPGFATGDETMFTGNAMTYYGRWTYKFEEAARQGAAGALIIHQTEPASYGWEVVRNSWSGTQYGVVTNGNRDRLPVEGWIHLDAATKIFDAAGINILETIASAAHRDFVAQPLGLTASVSFNNTFNHSECHNVIGYIEGTKYPEETVVYMAHWDHLGMVVTEQGVDIYNGAVDNATGVAGIMAIAERFMKEGAPERSVAFLAVTAEESGLLGSRFYAENPLFPIATTVAGINMDALNVYGPTNDVVSIGFGLSELDDYLDRQAGAQNRVVKPNPFPERGYYYRSDHFNMARQGVPMIYANGGNDYIGRDEEYTRMVQQDAASRYHAPTDVVHDLWNYDGIHQDLWLFYNIGKDLANTDHFPNWAPDNEFRAARDAKAHLRRN

SEQ ID NO: 168 - protein, 483 aa, Alkalitalea saponilacus
MYPFENLKPAEIWTYFHEICQIPRPSKNEEKMINYLIDFAEKHGLDLKKDKIGNLVISKPATAGFESLPSVVLQSHIDMVCEKNNETVHNFMTDSINPYIDREWVKAKGTTLGADDGIGIAAQLAILASKEIEHGHIECLFTVDEETGLTGAFELEPDMFSGKILINLDSEDEGEIFIGCAGGIGTIGYFNPEFEATSKDAFAFKVSVSGLKGGHSGDDIDKGLGNAIKILNRYIYDATRQFGFQLATIEGGNLHNAIAREASATGVVPWKYKEEVRVLINCFIADLQEEIGKTEPHIKLHLESISLPEKILTKDFHNRLVNTIYAMPHGVITMSSSVPGLVETSTNLASINFEGEQLVINTSQRSALESGINNIANMVDSVFKLGEATTKQTDGYPGWNPNPDSSILKTAVETYKMLFKTEPQVKAIHAGLECGLFLQKYPGLDMISIGPTIKGAHSPDERLNIETVQKFWDHLLAILKHVA

SEQ ID NO: 169 - protein, 689 aa, Alkalitalea saponilacus
MKKLVLLTLAIIFCFSSCRQEAHEKSYDTLHFELSGDRMTPEALWSFGRLGNISVAPDQNTITYTITYPHIEENRFYSDIYTIPVNGGEPTRITNTSTIESQVNWRPDGEKINYISNESGSSQLWEINADGSGRQQVSDVDGGISGYLFSPDMSHIAYIRRVKLDESINDRHPDLPHANARVDDDLMYRHWDTWHDQHYRHIFIAPYKSGQMVRNGKDIMQGERFDSPMKPFGGMEQIAWTPCGTKLAYTCKKLAGRDYAFSTNSDIYLYDLNNETTTNLTEGMPGYDKNPKFSSDGRLMLWESMERDGYESDKNRLMVMDMETGEVADFSIGFDHNVSGPVWDETGEFVWFVSSIGGTEQIYLMDLADGGIHQITEGQHNFRGVQQVGEQLIASRESMSSPADLFKIDLRDGTTSNLTNINTHIMDQVTMGTVEERWVTTTDNKEMLVWVIYPPNFDPEKKYPAILYCQGGPQGALSQFWSYRWNFQMMAANDYIVVAPNRRGMPGHGTEWNEQISGDWGGQNLLDYLSAIDALAEEPYVDENRLGAVGASYGGYSVFWLAGNHDGRFSAFISHCGVFNLDMMYTNTEEMFFVDWDLDGPYWEQPDNRYDYSPHLFVENWDTPMLVIHGAKDFRVPYSQGMGAFNAARALDLPARFLFFPEENHWVLSPQNGILWQREFAGWLNEWLK

SEQ ID NO: 170 - protein, 751 aa, Alkalitalea saponilacus
MIDSDNKYFSVVLFLKTYIFRALMTLKLKTNLLLKMRKIFTGFIILAIIAIGNVKADEGMWVLPLLEKLNMETMQEMGLQLSAEEIYSVNESSLKDAIVIFGRGCTGEMISNKGLLLTNHHCGYGQIQELSTLENNYLDNGFWAANLEEELYAPGLTATFMKWMRDVTDDVFSVVEEGMDEQSRQTAIRERINELTEAEQDESGYQIQIRDFFAGNQYFMVAYEVFNDVRMVGVPPSSIGKYGYDTDNWMWPRHTGDFALFRVYADADGNPAEFSPDNVPYRPDHHLPISIKGYEKDDFAMTLGYPGSTQRYLSSWGIEERMNIFNQTLIDVRGVKQDIWAEAMAKSDRVRLQYATKFSRSSNYWKNSIGMNRGLEELNVLVQKRELENEFAQWVNQDESRKERYGAVLSLLEQAYENRADHYKANNYMRETLLRGTELFMFASGARELENALKDGNEEEIQSAIENLRNMAEEFYRDYHAPLDQRVMAAMLREYAENIPEEFHPKFFKEIPRRHQGDYEAMASYFFSRSFFVNQDDLNAFLDRPRLRRLLNDPAYKAGISTFETYRELLRLNQIAERQLGEANRLFIAGLKEMKPDKVFYPDANFTMRLSYGTVGDYEPRDAVIYKHYTTLEGVMEKEDPDNFEFYVPEKLKQLHRDRDYGRYAAADGRMYVNFTTNNDITGGNSGSPVINGNGELIGLAFDGNWEAMSGDIAFEPDLQKCINVDIRYVLFIIDKFAGAGHLIEEMTIVE

SEQ ID NO: 171 - protein, 718 aa, Alkalitalea saponilacus
MIKYLSLTFLLFHLILNHSHAREGMWIPVLIEQFNLTEMQEKGFELTADDIYNINEKSMHDAVVIFGAGCTGSMISPEGLLITNHHCGHRVIQSHSSVEQDYLTDGFWAMSREDELVNPNLRVTFLRRMEDVTTDVLQNVTNEMTMRQRKDSIDSNIERIIAKAIDGTHYVGRVESFFNGNQFFLMVNEVFTDVRLVGAPPSSIGKFGGDTDNWMWPRHTGDVAFFRVYACENNLPAEYSSENVPYKPKYFFPISLQGVEEGDFTMVMGYPGRTEQYVPSQHLKMLTKDIYPPLIGVRTHKLNIMDSYMEQDAAVRIAYASKHSSVSNAWKRWQGEIRGLGILNAVEKKQDYEKSLRNWILSNELISDEHAIILDLYDSLYTDFSYYRLGRDYILEMIGRTGMETVRFSGVFDRLALIGDDNGIPDEVKENLRASISEHFRDFYKPLDREMTISLLNMFFSEMYPKYNPDVFELIFEKFDGDFEAFVDDLFKNSVFTNEEKTKEWLESVTYDTRLDYRKDPAYVLFRSLRDFYYFNLTPGFNRAGQKLDSLNRVYINLMKEYEPERLFYPDANFTMRVSYGTVRGYEPRDGVYYQHLTTIDGVFEKYDPSFSDYFVPEHLKYLYENRKFGNYAVDGTLPLCFVATNHTTGGNSGSPVLNNRGELIGVNFDRAWEGVMSDLMFNPDQCRNISVDIRYALFLIEKYGKADYLLDEMKIIQ

SEQ ID NO: 172 - protein, 729 aa, Alkalitalea saponilacus
MRILILALLASFILNINAQKKALSLDDFVSAQTFAAERVQGLRPMKDGSSYSVLEANGTQIVRYSYATGEKTGVIADIPNLKDTPIKSILDYEFSDDETKILVYTNRQNIYRHSFIADYYVIDIARREIEPLSENGAQQAATFSPNGHAVAFVRNNNIFIKNLRFGTEAAITSDGEKNHIINGVPDWVYEEEFSFNRAFEWSPDGRELAFMRFDESHVREFSFPLYMGSSPNQSEFELYPGEYRYKYPKAGERNAKVSVHVFNLRNRTTKEMEVGGDNIYIPRIRWTTQPDQLAIVTLNRRQNQLDLYIANPSSGVARTIFTDRNERYVDYSVLDNIHFLEDGRHFVYVGELDGFNHIHLFGMDGRKIRQITKGEWDVTNYLGFDNRNRLFYFQAAAVSPLRREIYSIRMDGTRLTRLSENEGTNMAWFSSDFSFFINEFSNTTTPPVYQIFNRNNRLIRTIEDNRALKSRVAEYAKPTKEFFSFKNSQNVELNGYIIRPLDFSERNQYPLLLTQYSGPNSQRVLDRWEPGWEYFLATQGYIVVCVDGRGTGARGEDFRKQLYMQLGRFESEDQIETAKYMAKRPYVDADRIGIWGWSYGGYITALSMSRSEIFRTGIAVAPVTDWKFYDTVYTERYMRTPRENPSGYANFSPLNLADSLHGRLFLIHGSADDNVHYQNIMEYSNRLVQANKQFDMFIYPNRAHSLIGGNTRNHLYHMKFEFLERNLKN

SEQ ID NO: 173 - protein, 492 aa, Alkalitalea saponilacus
MKTRKLISTFAIAFLGALAGVFIYSQFFSAEPRIIEVPVKTNHPGTNSMFTSLPAGSSSAQYPDLTYAAEKSVHAVVHVQTKGRSSGSGAPSSGHPLFDFFFGPRGFGQPQPQQPVMGSGSGVIISQDGYIVTNNHVIDRADEIEITLNDNRSYKAILVGADPTTDIALLKIEETDLPYLVYGNSDALNIGEWVLAVGNPFNLTSTVTAGIVSAKSRSIQILGQMSIEAFIQTDAAVNPGNSGGALVNTRGELIGINTAIASRTGSFTGYSFAVPVSIVEKVVDDLLEFGAVQRGLLGVSIRGMNNELARELGMDRVRGVYVVEPTEGGGAKAAGIKSRDVILSVNGDAVNSVPQLQERVSRFRPGDNVQLEVLRDGKRKPFTVTLRNIHGNTDLVQNVDKMSLLGASFEPLSDDERQRLRIRNGIKVTEVGSGKFRDAGIREGYVIIQANRVPVNSEDDLRKVVDVASDALFLSGVYQNGRTSFYAINLQE

SEQ ID NO: 174 - protein, 1818 aa, Alkalitalea saponilacus
MRPFNSKCIFSFILAGILCIIITKAETPDIQKARNEAAAFFASELKSSHEVVLYPRYQSPLGVSTPVFAFQKEDEGYVVIAKFGDNYVVAGYSEDGLLDAENTPEAFWLLLQSYEQMDSIAPPALKTLKSSGVVVSPLLASRGVNLGQTYHTNAGGCPSGCAATAMAQIMAYHRHPDQPTGAHCYVHPNQGEHCVDFSEIQFDWNNMNNTNLQYYIGVSMEMNFCGSPYGSFPERSDFFNVMEDYFGYFLHTQGMGSDYWKYELDNGRPFYASMQGERSGHAVVIDGYDSDDYFHIHFGWAGLSNGFFLLNNENLIAAGSDRYRSRFSRTVFISPNHYVTNEQDSLALVAIHNSLNGQTGWDLSKPVVKWHGVNVMNERVMRVQIGSFGSNISGTIPPQIGQLTELRSLILNADINDIPEEIGLLSELTYLRLNGNINGTLPASITNLNKLQGLSIQRGQGNLTWQIPSDIDRMSSLTELYLPDIAVGTLPESFGQLSQLRTAYLYQGALTGQIPSSIGNLGNLENIQLARNQLTGTIPTSIGNLTNLVYLDLSENELSGSLPEGLGQLQRLYRLNLQNNDFSGTLPEQLNWYDLVDLQLHNNQLEGEIPSSIGNSKNLQGLRLHNNNFSEFPDEIGELIALTHIDVSENQLTSLPESLMNIPGLLRFKAANNHIAELPDNFGAWENLIELNLSNNRIETFPVEICFLTNLETVDLSHNKIKRLPSAITMLTPKNHLLLAHNEISGSISRSLLNVPLFALTLSRNRLTFDDLPAPEKLRHGIGDQKSALLSVNEIKAKMGDTLYIDIRDLGNFSNPDNEYFWLIYPDKISARFKNELDNQESDPVLVLPVNEETLSRQYYCKIFNFNVPEYDRDHMGSISTLPALRFLNTDTIGITLYTEQELVEKAYPDRYVTESKKLHNHLVYDNNVTLLAPAGLRGEVTWQGSLDGQKWHTISEEMEQENIKVNVVDFNEQELVISAQSPAWFRSAITEESCDPIYTDSVRVKPLGNLLFDEMVNVAEESLTISVDSIEVTLPVGLTDKDFRLTITKLDNPPPTPDMHRLSSVYDVTVSFGTVFDIPLEIKLKNIDITDVDAMNLPDFRPVYYDDQAQEWVEYLEGGISLEDDAVVFYTPHLTKLGWWEVRHGSYTHRFTKNRAEVIYKWDTGTGEINSFMGYEMTARQSPSKPWHQSNTDPDTGGTPLMIQDVAEYLNQVIDSFAVRGLNLWRSRFIVYVSNTGSGSFGHISAGGYARGYFTLNSQLLIETDDLKRTIAHEYMHYMQQFYMAVMTANTFWAEANAPLAGRLVWGVSDLENAEPEVNLQQSYKPVGGDKSIFDLLGQSWDAATFLPVLEKFTANQADANLSSTFLHYMHQYREGTKLNPVKMLTDLHTFGSLSSIIWRNYLNDQIVAQLGSTVGQEYDDYVRYMLEGSNPKLTILNKGKGNPLSHIINNTKDEEMGTFAQNMIYHFNKDENDPQVDDISFAVPYLASKMIVMSNSTPDRAVVVNYTRKHDLNPDGKVYYGKYDFESEKMVFEEISDSTKFSMLLEPNSQFSAKRYQNMGFLLFVNQRCPSVIGISNNFNTSFELEAMPVINIYNIADARITDRSIHQYSDGRSRSFIIDGNINIPNAPGRNHTTTNYNSRKRMLNDSAYVVYSGFTERLVVDNGQNSPTSITTWNKEQVITYNFVKGTLEIQQSILTTYRWGGYSLPQPNSDVYMPAYTHTIRNETKRLKLKNVTSFEEGQYPGYYGDVLEFKTSNTNETMQAVEEIYHTFTETRYDSEGDVVSSDSATYTGTDFSSPDITVEVKVHNKRVFFAN

SEQ ID NO: 175 - protein, 482 aa, Alkalitalea saponilacus
MSFTIRATLEVPQEISKIFLIQNTEQLKDFMFSETEIEYIEKKYQENEKDKSPLVIIKRLSQILAVVKPTTDEPLEIIKERMRRRGAEILSGLKAEKNEKAAIIDLISNPPLTLALAEGLALNAYSFNKYKTGEKNSLNYEFLIVSPQVKGCDIAKLTRVIEAVYLARDLVNEPVGYLNAEKLGELVLEYAEKFGFKAEVFNKKKIESLKMGGLLAVNKGSIDPPTFSVLEWKPENAVNSKPYVIAGKGVMFDTGGVNLKTPPGSLDTMKCDMGGAASVIGTMAAVAANELPVHVIGLIPATDNRLGGHAIVPGDILKMHNGLTVEVINTDAEGRLILADALSFSKKYDPELVIDLATLTGNAAIAIGIHGIVAMGTAPQNVQNELNNAGDEVCERLVWFPFWEDYDKSIKSDIADIKNLGEREGGAISAGKFLGKFVDAPWVHLDIAGPAYVMAATDYRPTGGTGVGVRLLYQFFNSKSSK

SEQ ID NO: 176 - protein, 349 aa, Alkalitalea saponilacus
MKSKILPTILILLFVTAQVYACTTFFLNGEQKLFGRNFDFPSGVGHIYINPANIEKTSFIFPPEKPFTWVSKYGSISFNQNGREMPYGGINEAGLVIEQMWHQEAKYPEPDQRKALTELQWIQYHLDNSATVQDVINSDEKLRISITSVATLHFLVADASGDLAAIEFFDGKMVVHSGDELKYPVLSNCSYDVSLNYIATTNPNLEHTPWVENSSGRFKTAAGMIGAKDLKQKDKTAFAFEILDAVAQGESTRWSIVYDISNFKIHLKTNENKEVRTINFNEFDFSCTNTPLFIDIDHANPSVKNFKPFNIEDNFNLIDKVCNEVEFLGQMPTEYRQAVAAFPATFNCK

SEQ ID NO: 177 - protein, 259 aa, Alkalitalea saponilacus
MVYLKTDEEIELLRESNLLVAKTLGELAKVIKPGVTTLQLDKIAETFIRDHKGVPGFLNYQGFPNTLCTSVNDQVVHGIPNDKPLNDGDIVSIDCGVLLNGFYGDCAYTFEVGQVDEKIRRLLQTTKESLYKGIEQAFEGNRLGDIGHAVQTLCESRGYSVVREMVGHGIGRKLHEPPEVPNYGRKGSGIKLRKGMVIAVEPMINLGKRDIKMWNDNWTISTIDKSISAHYEHTIAIGKNEADILSSFKFVEEVLTLQS

SEQ ID NO: 178 - protein, 304 aa, Alkalitalea saponilacus
MIIPPYIQKGDTIGLISPAGKIAHQVVTIAGNYLEHAGFPYVQGACLSGAWNQFSGTDEQRVSDINEMIHNPEVKMIWCSRGGYGTMRLLNRIDWAHLKKNPKWLVGFSDITAFHSALQNVHGMVSIHGPMLKNLVKGNFEFSGVKTLWDMVQGEMPDYVADYQKLNRTGDASGVLIGGNLTLLSALKGSVYDFHPKGKILFIEEVGEHFYHLDRMMQGLKISGKLSALSGLVVGQMTDMSDNATPFGATANEIVMDAVKDYDFPVMFGFPAGHDVRNEPLLMGAKVQLSVSDNQSRLKFLNSF

SEQ ID NO: 179 - protein, 55 aa, Alkalitalea saponilacus
MRKQRICQQLNECPHSPGEARVNDIVYNMEEFYKAFNLDDSGDRFIAPDDRARIW

SEQ ID NO: 180 - protein, 577 aa, Alkalitalea saponilacus
MARCTGLFLIIISALYISPTLSRAQYNYPRWDFHMPLDIDLVVSGSFGELRGSHFHSGVDFTTHGKTGLPIYSIDDGYVFRIAVSPVGFGKAIYVNHPNGFSSVYAHAEWFSKSIEEIVTNIQYEKESFAIDESFAPGEIPVKRGQIIAYSGNSGSSGGPHLHFEIRETDTQKPINVHFFDFPVKDDVPPHIEAVVIYPLNEQSRVNGKSEPLYLPVVFHSGRFHLRGNPRVEASGQIGVGIETLDYFTGSWRKCSVYSIQLIVDEQPWFKSRLDGFLFSQTRYLNSHIDFKRRRTHRQVIQKSFLDENNQLDIYQTGASRGVVAMTSGESRQFHYRVKDAAGNLSQLIFNIHGTNPPRIPEVSAAPKMETLHPASAWSDSFGDFGVSFPANSFYSRVKADFNVIPNPGVGIGQHFSVLNENVPIHQFFEITIPIPHQYLNHQRLTAARVGNNGSLIYAGGTRRGNQMVVRTRDAGTYCLTTDETPPTLRLLNIPAGRNYSNRDAIRVDIRDNFSGIASYRATINGEWALFEYDPKNNLLIGFFDKFRINKGQRHTLEIVATDNVGNETRLSTDFIY

SEQ ID NO: 181 - protein, 332 aa, Alkalitalea saponilacus
MKNSVLCFMAIPLLFIACGQGSGNQQRSVATTIAKPDLITPEFNADSAYYFIEKQVSFGPRVPNTPEHIACAEYLAETLERFGAEVIVQEAEVRAFDNTRLNIRNIIGQFQPEKSERLLLFAHWDTRPFADHDPDPAMRNTPILGANDGGSGVGVLLEIARHLQENPTHPGIDIIFFDAEDYGIPDHFHVPYKPDTWCLGSQYWGQNPHVRNYYARFGILLDMVGAKDAQFYREQHSLRFAPRLVDHIWNIAHELGYGAWFNFGIGGLITDDHVYVYKHLNIPSVNIIQHDPTSPTSFGSYWHTHADNMDIIDKATLKAVGQTVMEVIYREK

SEQ ID NO: 182 - protein, 487 aa, Alkalitalea saponilacus
MVRTHHFLITLLFLIFVSGNLYSQELRERLETHVTILAADSLEGRGLGTRGKDIARDYIRNQFAEIGLTSFKEDYFHHFEFRSTSGVIANIYGTNVVGFLKGHDSKLKDEYIVIGAHYDHLGYEMRGDERVIFPGADDNASGVSLMLEMARYFATNPESHGRSLIFVAFDAEESGLIGSRWFIEDERFASKDIKTMFSLDMVGMYRSNEGLNLKGIGSIAGGEELAGYLAGNHNLILRKQGSRIEERTDTWYFGLAGIPSVHVHTGPHSPYHQPGDLAHLLQYEEMAKVKNFTVDLVKILSFQESIEPSGSFLAQSGNVRFDFGAVAMLGRSRHLYPDEFFTADDVFGFGAGFFLRIHMGQKIVVQPEVLYDYNGSKSPEGSFRRHSVMLPLNIQYNLMSMHGGIFRMYPFAGGYYQHHFNGKNGGETIDFSTYYKDHEWGFQYGLGIDMLKFHLGFVYHQALTGVADDDLLKIRSSSNRFRIGYRF

SEQ ID NO: 183 - protein, 276 aa, Alkalitalea saponilacus
MSVIMETKNRHILLVMAIMIAISGIYWSCATVPITGRRQLSLVPESELMAMSYTQYNQFLEEHKISQNQEQVDMVKRVGERIASAVEKYFEQKGWSDQFANFQWEFNLIEDDTPNAWCMPGGKVVFYTGILPITQNEEGLAVVMGHEIAHAVAKHGSERMSQQIGIQFGAVALSALLSEKPEETQNLYLAAYGVTSQVGLMLPYSRKHEHEADRLGLIFMAMAGYNPSVAVDFWQRMAQLSQGGSPPAFLSTHPSDQARVNYIREVLPEALEYYNP

SEQ ID NO: 184 - protein, 470 aa, Alkalitalea saponilacus
MKATKYIKIIFLFATGIFLILSSCKKDDEINPGNIEEIPSGILNINQFISYYMNLAYFWNKEMPDIDYKTEPDPEKYFYKLLKEPDDRWSFITDNITELENYLQGIAKSKGYSIAPYYFKEGSNQVVAFVQFVYRDSPAEQAGLKRGDMFYKINGQTITDINYQQLLSLDDVTLTMGQIIDGDIVKLDPEVNISAVENFSSHPILSTSIIEASGLKIGYLAYGSFINNFDTAIVNTFSRFHEAGVDELILDLRYNGGGHVGSAVTLASLIGSADLADETFIFERWNSNLSSFNDAVKFEEQGFNLGLNRLFVLTTDRTASASEMVIYGLEPYIDIIQVGENTYGKYYGSVIISDNNQNPHMRRHNWAIQPIVFRAENIKNNINYQQGLPPTFTIDDDMYAVHLFDEGAQLGEKEEFFIANVLSIIETGSPILSDAELKRSSLRSSKAVKLKDILSTYHGLMISERTSGDF

SEQ ID NO: 185 - protein, 558 aa, Alkalitalea saponilacus
MKTPILFFKLMVLMTIFYSCKDDDKAQILSTVEVNIKIDENYNFIPLENTTIRITNIQSGETDSTKLLDATKVLFTDLIPGDYQIQAYRHLTDDEKESLYGDKSTQIYITSTQNIKAGAIKDIRIYLTLKPNVEFLPAQTLTVNNFIYTYMDYAYFWHKEMPEINYRTQRDPEAYFYSLLKDPDDKWSFITDDIEALIAYFDGVSKSKGYSIQPYYLRQGSNQVIIYVEYVYRNSPASEAGLQRGDMIHKINGETVTDQNYQRLLNNDNMVLTLGYLDDSGNIVSLSPEVEINAVENLQHHPIIASSIHEVEGSTIGYIAYSSFTASYDTALVNTFSDFKAAGVNELVLDLRYNGGGRVTSAVLLAGLIAPKSSVGEVFIEEVWNENLKNYNAKLRIPNQSMNLDLSRVYILTTSGTASASEMVIYGLAPHMEVIQIGTQTHGKYYGSIMIQDIDENTNQRRHSWALQPIVMRAQNVTNDINYQQGLPPNHTLRDNIYNAQLGDIEEHFLSNAISLITSGSLVELAPELKKASIDYIKIENFKENNIPYHGTMITELP

SEQ ID NO: 186 - protein, 428 aa, Alkalitalea saponilacus
MRRHNLNRYLALVFLISCSCLTKGLGNEEFDFETTLRFDFILAGDHSNQRAYPVSFSQHPGWSGTVNQLISPFDFGEYRYLLIHPESGDTLFQRGFSTLFEEWRTVEEAKYSRRAFQQTVLMPMPLMKMTLVIDGRERDGLFLQLLKETIEPGSLSIKISQPTEFEKRILHGDLGVPKADFLIMAEGFEIDEMEVFFQKAVELTEAILNVEPFKSHRDLMSVSALGVPSKQSGVNDPHQNTWRNSAMGVSFNSLGIDRYLVTESFWKVHDYAAQVPHDHLIILVNGNKYGGGGIYNHFSVVTSHNRLSAEVLLHEIGHGFAGLGDEYFDSDVSYTDYINQEIEPWQPNLTTLINFGSKWEYLLSSDTPVPTPIRPKYRNVTGVFEGGGYVAKGVFRPAINCRMRSVDASAFCEVCHKVILQKLLFYSQ

SEQ ID NO: 187 - protein, 235 aa, Alkalitalea saponilacus
MERLNSIKILPQPDDTTCGPTSLHAVYRFFGLKVELSEVIETVTSFEEGGTLAVMLGIDALKRGFDATIYTYNLKVFDPSWAETDNEQLCELLGEQLQYKTGKKFSQATKAYQNFLNLGGKISFEDLNKKILKRYFEKDVPILTGLSATYLYNTKREYTNRKNRSVFDDLKGEPMGHFVVLCGMSGNTVYVADPYKENPISGKNYYEVDTNRLLNSVLLGIVTYDANMLVIVPKD

SEQ ID NO: 188 - protein, 700 aa, Alkalitalea saponilacus
MKKLFGFILTLVFMASFATTDENPFFSDYETPFGVPPFHLIENSHFIPAFEEGVRQQEAEIAAIINNPALPDFDNTVAALDYSGELLNRVASVFYNYNSSNTSDEIQALAQEVAPMMSSHRDNISLNPALFARIQTVYNQKDELGLTEEQAMLLEETYQSFVRNGAALPAEQQERFREINQELSVLTLQFGQNVLADVNGFKLWVDDEADLAGLPGSVVDAAAEAAAADGQEGKWLFTLHNPSVMPFLTYADNRDLREKMNRAYVLRGNNDNDNNNQEIINRLTELRLERSNMLGFDTYADFALQNRMAGNVETVETFLKDLWTAALPIARDEAVELQKMITSEGGDYELAYWDWRYYAEKVRKAKYDLDEGEISQYFEINNVRDGIFMIVNKLWGLEFVERADVPVYHPDATAWEVLEADGSHLGILYMDMHPRASKRGGAWMSSYRRQQVSQDGEFVHPIITIVCNFTAPSGNQPALLTFDEMTTFFHEFGHAIHGLMSDVIYPGLAGTSVPRDFVELPSQVLENWAKHPEVLKMFAKHYETGETIPDELIDRIMASANFNQGFATVEFLASALLDMDYHTKTVFEPFDVNEFESGVQNRYDMMDEIYFRHGSTHFQHIFSGGYSAGYYSYIWAGVLDADAFEAFVETGDLFHQETARKFREEILERGGTRDAMEMYKSFRGKEPGIEPLLRQRGLVR

SEQ ID NO: 189 - protein, 678 aa, Alkalitalea saponilacus
MNNILNQHFNTPYQTPPFNEIQPDFFLPAVKEAIKQGINEVREIIENSQDPDFSNTIEALERSGKQLSRISSILFNLNAAETSEAIQKAARDVSPLLSEYANDIWLNEALFEKVKTIYNNKGTLQLSQEQQTLLDKTYKGFIRKGALLDDKQKKRYRQITNELSQLSIQFGENLLAETNDYKLHITNEEELSGLPEAVIEAAAHLAKNEGKEGWMFSLHITSFMPFMKYADNRKLREQLFRAYSSRCNHNNKHDNKEIILKQTALRLEKAELLGYKSHAQYVLEERMAQTPEKVNNFLEEFYSKSFDFAKKDIEEVKAFAKKAGFNEEFQRWDFAYYSEKLKTARFQLDDEMTRPYFQLEKVKQGIFNLTKKLWGLSYKKSENIPVYHPDVEAWEVYDESGEQLSILYLDFHPRKSKQGGAWMTSFRDQHVKNGINILPQISVVCNFTEPTPTRPSLLTYNELTTFLHEFGHALHGMLSKVTYESLSGTSVYHDFVELPSQIMENWAREKDWLQEIGIHYKTGEPIPEELINNILASGNFQSGYQIIRQLSFGFNDMAWHTITEPVQSNPVEFEREAMKPTELFPLIEGTCMSTAFGHIFDGGYASGYYGYKWAEVLDADAYTMFKLHGIFDKNTAQKFRDTILSKGGTIHPMELYKAFRGQEPSIEPLLKRSGITKH

SEQ ID NO: 190 - protein, 673 aa, Alkalitalea saponilacus
MKVLSMMAAMMFGLLIHSIAEKSPITAENLWEFARVGSPTVSPDGKQTVFPVSTYCIEENNSKTHLYLMNNENGNYRQLTFNGSENSPAWSPDGQYIAFVSRRNNNPAQLFILPLYGGEPRKITDLPVGVFAPKWFPNGKKLAFGANIHPDYDGDWDQLKEIQKQSRENKVTAKVTENVMYRFWDRWITDGFYPRLFTVDLNSETVTDLMPGTNNFFNMMGGVNYDIAPDGKTIVVSMNSTEPPYERLNYDLYLVPTNGSGELTNITADNPADDMNPVFSPDGKKILYGAKEIYHFYADKTVMVLYDVATGNKQRLTDHIDLSCENWFFSENGRTIYFHAQDNSMTSIFSIPANGGQHTELFGSGTNSGAALAGNRHLIFNHHNLSAAPELYRLNLRNRQTEKMTGFNDDLVATINWGSIENVTYKGAEDRDVQMFINYPPDYDPNKKYPLVLMIHGGPHSIFGDSFHFRWNSQLFAAPGYIVAMPNFHGSTSFGQDFAISIHGEHAPKPFEDIMKATDYLIERGIVDETRMAATGGSYGGYMVSWIAGHTDRFAALVNHAGVYDLHLQFASDYSGNRAYQYSGSPWENFDQLNANNPAQFAHNFKTPMLVIHGELDYRVPVAHGFLIYGIYKSMGLDARLVYYPDENHWILNPQNSIFWYEELHNWLERYLK